European Patent Specification EP 4 381 096 B1, published May 28, 2025. Title: METHOD FOR DETECTING AN ANALYTE IN A PATHOGEN-COMPRISING SAMPL. Applicant: Resolve BioSciences GmbH. Application EP PCT/EP2022/071935, filed August 4, 2022. The sequence listing filed with the application follows.

SEQUENCE LISTING (1400 sequences)

SEQ ID NO: 1 - DNA, 45 bp, synthetic construct
  misc_feature 1..45: note = Target Specific Oligonucleotide
  source 1..45: mol_type = other DNA
actactagagaccggtagaaatgagtaacgattaccgacttatcc

SEQ ID NO: 2 - DNA, 42 bp, synthetic construct
  misc_feature 1..42: note = Target Specific Oligonucleotide
  source 1..42: mol_type = other DNA
tggcggggaacgaagtatatagtaacgattaccgacttatcc

SEQ ID NO: 3 - DNA, 40 bp, synthetic construct
  misc_feature 1..40: note = Target Specific Oligonucleotide
  source 1..40: mol_type = other DNA
tggcgtcaatggttgcggtgtaacgattaccgacttatcc

SEQ ID NO: 4 - DNA, 41 bp, synthetic construct
  misc_feature 1..41: note = Target Specific Oligonucleotide
  source 1..41: mol_type = other DNA
tcggtcactcgaataacccggtaacgattaccgacttatcc

SEQ ID NO: 5 - DNA, 41 bp, synthetic construct
  misc_feature 1..41: note = Target Specific Oligonucleotide
  source 1..41: mol_type = other DNA
ctccaaatcgaggtgcaccagtaacgattaccgacttatcc

SEQ ID NO: 6 - DNA, 40 bp, synthetic construct
  misc_feature 1..40: note = Target Specific Oligonucleotide
  source 1..40: mol_type = other DNA
ggccagttcccgagttggtgtaacgattaccgacttatcc

SEQ ID NO: 7 - DNA, 42 bp, synthetic construct
  misc_feature 1..42: note = Target Specific Oligonucleotide
  source 1..42: mol_type = other DNA
agacttcaagcgacatgctctgtaacgattaccgacttatcc

SEQ ID NO: 8 - DNA, 42 bp, synthetic construct
  misc_feature 1..42: note = Target Specific Oligonucleotide
  source 1..42: mol_type = other DNA
ggagcaccaccgtagatacaagtaacgattaccgacttatcc

SEQ ID NO: 9 - DNA, 44 bp, synthetic construct
  misc_feature 1..44: note = Target Specific Oligonucleotide
  source 1..44: mol_type = other DNA
ctctccaaatcacgtatttgtgggtaacgattaccgacttatcc

SEQ ID NO: 10 - DNA, 45 bp, synthetic construct
  misc_feature 1..45: note = Target Specific Oligonucleotide
  source 1..45: mol_type = other DNA
agagtttgcctatcaggtcttattgtaacgattaccgacttatcc

SEQ ID NO: 11 - DNA, 40 bp, synthetic construct
  misc_feature 1..40: note = Target Specific Oligonucleotide
  source 1..40: mol_type = other DNA
ggccaagtcgcactccacagtaacgattaccgacttatcc

SEQ ID NO: 12 - DNA, 43 bp, synthetic construct
  misc_feature 1..43: note = Target Specific Oligonucleotide
  source 1..43: mol_type = other DNA
tccttttctacgtcatgacacagtaacgattaccgacttatcc

SEQ ID NO: 13 - DNA, 46 bp, synthetic construct
  misc_feature 1..46: note = Target Specific Oligonucleotide
  source 1..46: mol_type = other DNA
ttccattagacgaataagtttttcagtaacgattaccgacttatcc

SEQ ID NO: 14 - DNA, 44 bp, synthetic construct
  misc_feature 1..44: note = Target Specific Oligonucleotide
  source 1..44: mol_type = other DNA
tttctggtaagctcatcacatctgtaacgattaccgacttatcc

SEQ ID NO: 15 - DNA, 46 bp, synthetic construct
  misc_feature 1..46: note = Target Specific Oligonucleotide
  source 1..46: mol_type = other DNA
gagttagggtagtcataattgatgagtaacgattaccgacttatcc

SEQ ID NO: 16 - DNA, 47 bp, synthetic construct
  misc_feature 1..47: note = Target Specific Oligonucleotide
  source 1..47: mol_type = other DNA
ttcttccaattcgatgaatataatccgtaacgattaccgacttatcc

SEQ ID NO: 17 - DNA, 48 bp, synthetic construct
  misc_feature 1..48: note = Target Specific Oligonucleotide
  source 1..48: mol_type = other DNA
tgttattaggtgtaaagaaagtgtatggtaacgattaccgacttatcc

SEQ ID NO: 18 - DNA, 42 bp, synthetic construct
  misc_feature 1..42: note = Target Specific Oligonucleotide
  source 1..42: mol_type = other DNA
gagataaggtcgctcacttgcgtaacgattaccgacttatcc

SEQ ID NO: 19 - DNA, 42 bp, synthetic construct
  misc_feature 1..42: note = Target Specific Oligonucleotide
  source 1..42: mol_type = other DNA
acctctgtcttcgaccaactggtaacgattaccgacttatcc

SEQ ID NO: 20 - DNA, 41 bp, synthetic construct
  misc_feature 1..41: note = Target Specific Oligonucleotide
  source 1..41: mol_type = other DNA
acccctggaacgacctgaacgtaacgattaccgacttatcc

SEQ ID NO: 21 - DNA, 41 bp, synthetic construct
  misc_feature 1..41: note = Target Specific Oligonucleotide
  source 1..41: mol_type = other DNA
agtatctgtcccgacggtcagtaacgattaccgacttatcc

SEQ ID NO: 22 - DNA, 40 bp, synthetic construct
  misc_feature 1..40: note = Target Specific Oligonucleotide
  source 1..40: mol_type = other DNA
accccttttgcccgcagaggtaacgattaccgacttatcc

SEQ ID NO: 23 - DNA, 44 bp, synthetic construct
  misc_feature 1..44: note = Target Specific Oligonucleotide
  source 1..44: mol_type = other DNA
tttaagcaggctagagtaacctcgtaacgattaccgacttatcc

SEQ ID NO: 24 - DNA, 45 bp, synthetic construct
  misc_feature 1..45: note = Target Specific Oligonucleotide
  source 1..45: mol_type = other DNA
gcattggataaccaatcataggtggtaacgattaccgacttatcc

SEQ ID NO: 25 - DNA, 41 bp, synthetic construct
  misc_feature 1..41: note = Target Specific Oligonucleotide
  source 1..41: mol_type = other DNA
tcccctagtccgagttgctcgtaaccctaattatgggaatc

SEQ ID NO: 26 - DNA, 43 bp, synthetic construct
  misc_feature 1..43: note = Target Specific Oligonucleotide
  source 1..43: mol_type = other DNA
ccaatttgcacttggatgtgtagtaaccctaattatgggaatc

SEQ ID NO: 27 - DNA, 43 bp, synthetic construct
  misc_feature 1..43: note = Target Specific Oligonucleotide
  source 1..43: mol_type = other DNA
ttttgccagtagaacaagcatggtaaccctaattatgggaatc

SEQ ID NO: 28 - DNA, 40 bp, synthetic construct
  misc_feature 1..40: note = Target Specific Oligonucleotide
  source 1..40: mol_type = other DNA
ggaggcaaggttccgcaacgtaaccctaattatgggaatc

SEQ ID NO: 29 - DNA, 44 bp, synthetic construct
  misc_feature 1..44: note = Target Specific Oligonucleotide
  source 1..44: mol_type = other DNA
agaattccacgtaaatcacatgcgtaaccctaattatgggaatc

SEQ ID NO: 30 - DNA, 44 bp, synthetic construct
  misc_feature 1..44: note = Target Specific Oligonucleotide
  source 1..44: mol_type = other DNA
tatgcatgtacagggaagtatccgtaaccctaattatgggaatc

SEQ ID NO: 31 - DNA, 43 bp, synthetic construct
  misc_feature 1..43: note = Target Specific Oligonucleotide
  source 1..43: mol_type = other DNA
gtgtgcatgccttagaaaaagcgtaaccctaattatgggaatc

SEQ ID NO: 32 - DNA, 43 bp, synthetic construct
  misc_feature 1..43: note = Target Specific Oligonucleotide
  source 1..43: mol_type = other DNA
agcttttgtgcccttatcatgagtaaccctaattatgggaatc

SEQ ID NO: 33 - DNA, 46 bp, synthetic construct
  misc_feature 1..46: note = Target Specific Oligonucleotide
  source 1..46: mol_type = other DNA
cttcattagtatcttgtcacttggggtaaccctaattatgggaatc

SEQ ID NO: 34 - DNA, 45 bp, synthetic construct
  misc_feature 1..45: note = Target Specific Oligonucleotide
  source 1..45: mol_type = other DNA
agatgatgaccctaccaaatttgggtaaccctaattatgggaatc

SEQ ID NO: 35 - DNA, 44 bp, synthetic construct
  misc_feature 1..44: note = Target Specific Oligonucleotide
  source 1..44: mol_type = other DNA
aggcaagagatagatatgtgggcgtaaccctaattatgggaatc

SEQ ID NO: 36 - DNA, 44 bp, synthetic construct
  misc_feature 1..44: note = Target Specific Oligonucleotide
  source 1..44: mol_type = other DNA
cagctgccactataatcatgtttgtaaccctaattatgggaatc

SEQ ID NO: 37 - DNA, 45 bp, synthetic construct
  misc_feature 1..45: note = Target Specific Oligonucleotide
  source 1..45: mol_type = other DNA
ggaacatgctaatttaaggtgagtgtaaccctaattatgggaatc

SEQ ID NO: 38 - DNA, 46 bp, synthetic construct
  misc_feature 1..46: note = Target Specific Oligonucleotide
  source 1..46: mol_type = other DNA
aggactttgctatatcaagtagttcgtaaccctaattatgggaatc

SEQ ID NO: 39 - DNA, 46 bp, synthetic construct
  misc_feature 1..46: note = Target Specific Oligonucleotide
  source 1..46: mol_type = other DNA
aaaggagatagtaacaatggttttcgtaaccctaattatgggaatc

SEQ ID NO: 40 - DNA, 43 bp, synthetic construct
  misc_feature 1..43: note = Target Specific Oligonucleotide
  source 1..43: mol_type = other DNA
aaatcagtggttcaccctgttcgtaaccctaattatgggaatc

SEQ ID NO: 41 - DNA, 48 bp, synthetic construct
  misc_feature 1..48: note = Target Specific Oligonucleotide
  source 1..48: mol_type = other DNA
cttgtcataagataattaggcaaattagtaaccctaattatgggaatc

SEQ ID NO: 42 - DNA, 47 bp, synthetic construct
  misc_feature 1..47: note = Target Specific Oligonucleotide
  source 1..47: mol_type = other DNA
tcattaagttaatgctaaggatctttgtaaccctaattatgggaatc

SEQ ID NO: 43 - DNA, 43 bp, synthetic construct
  misc_feature 1..43: note = Target Specific Oligonucleotide
  source 1..43: mol_type = other DNA
tgtcactggtacaagtggacttgtaaccctaattatgggaatc

SEQ ID NO: 44 - DNA, 45 bp, synthetic construct
  misc_feature 1..45: note = Target Specific Oligonucleotide
  source 1..45: mol_type = other DNA
ttggtcactatacaagtgacttctgtaaccctaattatgggaatc

SEQ ID NO: 45 - DNA, 43 bp, synthetic construct
  misc_feature 1..43: note = Target Specific Oligonucleotide
  source 1..43: mol_type = other DNA
aggaaaatgggcgtaaaggagggtaaccctaattatgggaatc

SEQ ID NO: 46 - DNA, 46 bp, synthetic construct
  misc_feature 1..46: note = Target Specific Oligonucleotide
  source 1..46: mol_type = other DNA
ttcatctacaatagggacaacaaacgtaaccctaattatgggaatc

SEQ ID NO: 47 - DNA, 44 bp, synthetic construct
  misc_feature 1..44: note = Target Specific Oligonucleotide
  source 1..44: mol_type = other DNA
gataagtctacgtggaaaagcatgtaaccctaattatgggaatc

SEQ ID NO: 48 - DNA, 45 bp, synthetic construct
  misc_feature 1..45: note = Target Specific Oligonucleotide
  source 1..45: mol_type = other DNA
caggactacagttaagcatttactgtaaccctaattatgggaatc

SEQ ID NO: 49 - DNA, 43 bp, synthetic construct
  misc_feature 1..43: note = Target Specific Oligonucleotide
  source 1..43: mol_type = other DNA
gtctaggaaattgccgtggttggtaaccctaattatgggaatc

SEQ ID NO: 50 - DNA, 42 bp, synthetic construct
  misc_feature 1..42: note = Target Specific Oligonucleotide
  source 1..42: mol_type = other DNA
aatcatcgtctcgaaagcggtgtaaccctaattatgggaatc

SEQ ID NO: 51 - DNA, 43 bp, synthetic construct
  misc_feature 1..43: note = Target Specific Oligonucleotide
  source 1..43: mol_type = other DNA
cttgaccaaattcgaaggtccagtaaccctaattatgggaatc

SEQ ID NO: 52 - DNA, 43 bp, synthetic construct
  misc_feature 1..43: note = Target Specific Oligonucleotide
  source 1..43: mol_type = other DNA
gatgactctgttcgcatcctcggtaaccctaattatgggaatc

SEQ ID NO: 53 - DNA, 42 bp, synthetic construct
  misc_feature 1..42: note = Target Specific Oligonucleotide
  source 1..42: mol_type = other DNA
gatgctagtgtcaaacctgccgtaaccctaattatgggaatc

SEQ ID NO: 54 - DNA, 44 bp, synthetic construct
  misc_feature 1..44: note = Target Specific Oligonucleotide
  source 1..44: mol_type = other DNA
tgatacagggctcgtacttatccgtaaccctaattatgggaatc

SEQ ID NO: 55 - DNA, 43 bp, synthetic construct
  misc_feature 1..43: note = Target Specific Oligonucleotide
  source 1..43: mol_type = other DNA
aggagtcacacgagttgaaaaggtaaccctaattatgggaatc

SEQ ID NO: 56 - DNA, 44 bp, synthetic construct
  misc_feature 1..44: note = Target Specific Oligonucleotide
  source 1..44: mol_type = other DNA
ctcattacaccgaggtatgaagggtaaccctaattatgggaatc

SEQ ID NO: 57 - DNA, 40 bp, synthetic construct
  misc_feature 1..40: note = Target Specific Oligonucleotide
  source 1..40: mol_type = other DNA
ctctgtcacggctcgggtggtaaccctaattatgggaatc

SEQ ID NO: 58 - DNA, 43 bp, synthetic construct
  misc_feature 1..43: note = Target Specific Oligonucleotide
  source 1..43: mol_type = other DNA
ctaccatatgtacccgacctcagtaaccctaattatgggaatc

SEQ ID NO: 59 - DNA, 44 bp, synthetic construct
  misc_feature 1..44: note = Target Specific Oligonucleotide
  source 1..44: mol_type = other DNA
aaccttaggtcgggtatagagaggtaaccctaattatgggaatc

SEQ ID NO: 60 - DNA, 44 bp, synthetic construct
  misc_feature 1..44: note = Target Specific Oligonucleotide
  source 1..44: mol_type = other DNA
gaagcacttagacactgtaaggcgtaaccctaattatgggaatc

SEQ ID NO: 61 - DNA, 42 bp, synthetic construct
  misc_feature 1..42: note = Target Specific Oligonucleotide
  source 1..42: mol_type = other DNA
aataatcaccggcagtaacgggtaaccctaattatgggaatc

SEQ ID NO: 62 - DNA, 43 bp, synthetic construct
  misc_feature 1..43: note = Target Specific Oligonucleotide
  source 1..43: mol_type = other DNA
aggaagaaacctatggcagacagtaaccctaattatgggaatc

SEQ ID NO: 63 - DNA, 46 bp, synthetic construct
  misc_feature 1..46: note = Target Specific Oligonucleotide
  source 1..46: mol_type = other DNA
catgtgttattacgatgttctttgtgtaaccctaattatgggaatc

SEQ ID NO: 64 - DNA, 45 bp, synthetic construct
  misc_feature 1..45: note = Target Specific Oligonucleotide
  source 1..45: mol_type = other DNA
actactgtttggtacttgtatctggtaaccctaattatgggaatc

SEQ ID NO: 65 - DNA, 42 bp, synthetic construct
  misc_feature 1..42: note = Target Specific Oligonucleotide
  source 1..42: mol_type = other DNA
aaatcagtggcggacagtagcgtaaccctaattatgggaatc

SEQ ID NO: 66 - DNA, 41 bp, synthetic construct
  misc_feature 1..41: note = Target Specific Oligonucleotide
  source 1..41: mol_type = other DNA
caggcaatgccgactggattgtaaccctaattatgggaatc

SEQ ID NO: 67 - DNA, 48 bp, synthetic construct
  misc_feature 1..48: note = Target Specific Oligonucleotide
  source 1..48: mol_type = other DNA
tcttatctaagaccaactataggtatggtaaccctaattatgggaatc

SEQ ID NO: 68 - DNA, 43 bp, synthetic construct
  misc_feature 1..43: note = Target Specific Oligonucleotide
  source 1..43: mol_type = other DNA
gggaactgtctattgagcactcgtaaccctaattatgggaatc

SEQ ID NO: 69 - DNA, 47 bp, synthetic construct
  misc_feature 1..47: note = Target Specific Oligonucleotide
  source 1..47: mol_type = other DNA
attacaatctttagtactcatggaaagtaaccctaattatgggaatc

SEQ ID NO: 70 - DNA, 46 bp, synthetic construct
  misc_feature 1..46: note = Target Specific Oligonucleotide
  source 1..46: mol_type = other DNA
aaggtattctcatgcctagaatattgtaaccctaattatgggaatc

SEQ ID NO: 71 - DNA, 43 bp, synthetic construct
  misc_feature 1..43: note = Target Specific Oligonucleotide
  source 1..43: mol_type = other DNA
tggacagacacgttgtcatttggtaaccctaattatgggaatc

SEQ ID NO: 72 - DNA, 48 bp, synthetic construct
  misc_feature 1..48: note = Target Specific Oligonucleotide
  source 1..48: mol_type = other DNA
ctctcattacaatgctatacatttaacgtaaccctaattatgggaatc

SEQ ID NO: 73 - DNA, 41 bp, synthetic construct
  misc_feature 1..41: note = Target Specific Oligonucleotide
  source 1..41: mol_type = other DNA
tgcagctcgcaacggaacaagtaacggattttacaacttta

SEQ ID NO: 74 - DNA, 43 bp, synthetic construct
  misc_feature 1..43: note = Target Specific Oligonucleotide
  source 1..43: mol_type = other DNA
gagtccatccggacattgacctgtaacggattttacaacttta

SEQ ID NO: 75 - DNA, 41 bp, synthetic construct
  misc_feature 1..41: note = Target Specific Oligonucleotide
  source 1..41: mol_type = other DNA
cttgaacggcctcgacgagggtaacggattttacaacttta

SEQ ID NO: 76 - DNA, 43 bp, synthetic construct
  misc_feature 1..43: note = Target Specific Oligonucleotide
  source 1..43: mol_type = other DNA
cctcctcggttatattggccccgtaacggattttacaacttta

SEQ ID NO: 77 - DNA, 44 bp, synthetic construct
  misc_feature 1..44: note = Target Specific Oligonucleotide
  source 1..44: mol_type = other DNA
accgagacttcgaaaatgaacgagtaacggattttacaacttta

SEQ ID NO: 78 - DNA, 43 bp, synthetic construct
  misc_feature 1..43: note = Target Specific Oligonucleotide
  source 1..43: mol_type = other DNA
cctctggctcgaaactgaaagggtaacggattttacaacttta

SEQ ID NO: 79 - DNA, 44 bp, synthetic construct
  misc_feature 1..44: note = Target Specific Oligonucleotide
  source 1..44: mol_type = other DNA
tgctatggactagatctcggcaagtaacggattttacaacttta

SEQ ID NO: 80 - DNA, 42 bp, synthetic construct
  misc_feature 1..42: note = Target Specific Oligonucleotide
  source 1..42: mol_type = other DNA
gccttgaccggtcagaagacggtaacggattttacaacttta

SEQ ID NO: 81 - DNA, 42 bp, synthetic construct
  misc_feature 1..42: note = Target Specific Oligonucleotide
  source 1..42: mol_type = other DNA
taccacagagatcgcagctgcgtaacggattttacaacttta

SEQ ID NO: 82 - DNA, 40 bp, synthetic construct
  misc_feature 1..40: note = Target Specific Oligonucleotide
  source 1..40: mol_type = other DNA
accagcccgaacctcgcccgtaacggattttacaacttta

SEQ ID NO: 83 - DNA, 44 bp, synthetic construct
  misc_feature 1..44: note = Target Specific Oligonucleotide
  source 1..44: mol_type = other DNA
actgtatgcttgccggtaattctgtaacggattttacaacttta

SEQ ID NO: 84 - DNA, 41 bp, synthetic construct
  misc_feature 1..41: note = Target Specific Oligonucleotide
  source 1..41: mol_type = other DNA
gaacatgaaccggccccgacgtaacggattttacaacttta

SEQ ID NO: 85 - DNA, 42 bp, synthetic construct
  misc_feature 1..42: note = Target Specific Oligonucleotide
  source 1..42: mol_type = other DNA
caggaatcccgtcaagggtgggtaacggattttacaacttta

SEQ ID NO: 86 - DNA, 47 bp, synthetic construct
  misc_feature 1..47: note = Target Specific Oligonucleotide
  source 1..47: mol_type = other DNA
tctcgatttacctcgtttaagatctcgtaacggattttacaacttta

SEQ ID NO: 87 - DNA, 43 bp, synthetic construct
  misc_feature 1..43: note = Target Specific Oligonucleotide
  source 1..43: mol_type = other DNA
agaaccatggtcgaactgacctgtaacggattttacaacttta

SEQ ID NO: 88 - DNA, 41 bp, synthetic construct
  misc_feature 1..41: note = Target Specific Oligonucleotide
  source 1..41: mol_type = other DNA
tctgaggggctacgctgagagtaacggattttacaacttta

SEQ ID NO: 89 - DNA, 41 bp, synthetic construct
  misc_feature 1..41: note = Target Specific Oligonucleotide
  source 1..41: mol_type = other DNA
aagcctctgttacgcccacggtaacggattttacaacttta

SEQ ID NO: 90 - DNA, 46 bp, synthetic construct
  misc_feature 1..46: note = Target Specific Oligonucleotide
  source 1..46: mol_type = other DNA
aatgattcaactcgtactggatcccgtaacggattttacaacttta

SEQ ID NO: 91 - DNA, 44 bp, synthetic construct
  misc_feature 1..44: note = Target Specific Oligonucleotide
  source 1..44: mol_type = other DNA
cctcggaaatcccgattctgatagtaacggattttacaacttta

SEQ ID NO: 92 - DNA, 41 bp, synthetic construct
  misc_feature 1..41: note = Target Specific Oligonucleotide
  source 1..41: mol_type = other DNA
ggcccctactcggttgtggggtaacggattttacaacttta

SEQ ID NO: 93 - DNA, 45 bp, synthetic construct
  misc_feature 1..45: note = Target Specific Oligonucleotide
  source 1..45: mol_type = other DNA
ggaaaatggaacgaaactcctgttgtaacggattttacaacttta

SEQ ID NO: 94 - DNA, 40 bp, synthetic construct
  misc_feature 1..40: note = Target Specific Oligonucleotide
  source 1..40: mol_type = other DNA
ctgggtcgtgcgaggtcctgtaacggattttacaacttta

SEQ ID NO: 95 - DNA, 40 bp, synthetic construct
  misc_feature 1..40: note = Target Specific Oligonucleotide
  source 1..40: mol_type = other DNA
cacggggctaggacggggtgtaacggattttacaacttta

SEQ ID NO: 96 - DNA, 39 bp, synthetic construct
  misc_feature 1..39: note = Target Specific Oligonucleotide
  source 1..39: mol_type = other DNA
ccgatggcgtactcgtcgggtaacccttattcggtacta

SEQ ID NO: 97 - DNA, 42 bp, synthetic construct
  misc_feature 1..42: note = Target Specific Oligonucleotide
  source 1..42: mol_type = other DNA
gatcagatcagaatccgaggtggtaacccttattcggtacta

SEQ ID NO: 98 - DNA, 40 bp, synthetic construct
  misc_feature 1..40: note = Target Specific Oligonucleotide
  source 1..40: mol_type = other DNA
ggttgtactcgcgacagttggtaacccttattcggtacta

SEQ ID NO: 99 - DNA, 40 bp, synthetic construct
  misc_feature 1..40: note = Target Specific Oligonucleotide
  source 1..40: mol_type = other DNA
gacctgctcattcgaggtgagtaacccttattcggtacta

SEQ ID NO: 100 - DNA, 39 bp, synthetic construct
  misc_feature 1..39: note = Target Specific Oligonucleotide
  source 1..39: mol_type = other DNA
tcacgtagtagcggcttcggtaacccttattcggtacta

SEQ ID NO: 101 - DNA, 42 bp, synthetic construct
  misc_feature 1..42: note = Target Specific Oligonucleotide
  source 1..42: mol_type = other DNA
ccaaagatgggcctacttgtcagtaacccttattcggtacta

SEQ ID NO: 102 - DNA, 39 bp, synthetic construct
  misc_feature 1..39: note = Target Specific Oligonucleotide
  source 1..39: mol_type = other DNA
gacagagctgcacgcttgggtaacccttattcggtacta

SEQ ID NO: 103 - DNA, 39 bp, synthetic construct
  misc_feature 1..39: note = Target Specific Oligonucleotide
  source 1..39: mol_type = other DNA
ctgggcctgtttgcgctcagtaacccttattcggtacta

SEQ ID NO: 104 - DNA, 38 bp, synthetic construct
  misc_feature 1..38: note = Target Specific Oligonucleotide
  source 1..38: mol_type = other DNA
tccttaggcatgcgcggcgtaacccttattcggtacta

SEQ ID NO: 105 - DNA, 39 bp, synthetic construct
  misc_feature 1..39: note = Target Specific Oligonucleotide
  source 1..39: mol_type = other DNA
cagcggcagtactcgctgtgtaacccttattcggtacta

SEQ ID NO: 106 - DNA, 38 bp, synthetic construct
  misc_feature 1..38: note = Target Specific Oligonucleotide
  source 1..38: mol_type = other DNA
atgccaccgatgacccgcgtaacccttattcggtacta

SEQ ID NO: 107 - DNA, 38 bp, synthetic construct
  misc_feature 1..38: note = Target Specific Oligonucleotide
  source 1..38: mol_type = other DNA
atcagcgtcgctccctcggtaacccttattcggtacta

SEQ ID NO: 108 - DNA, 41 bp, synthetic construct
  misc_feature 1..41: note = Target Specific Oligonucleotide
  source 1..41: mol_type = other DNA
ctttgagagctcgaacatcgtgtaacccttattcggtacta

SEQ ID NO: 109 - DNA, 42 bp, synthetic construct
  misc_feature 1..42: note = Target Specific Oligonucleotide
  source 1..42: mol_type = other DNA
ttccagtagttaaggcagagcagtaacccttattcggtacta

SEQ ID NO: 110 - DNA, 39 bp, synthetic construct
  misc_feature 1..39: note = Target Specific Oligonucleotide
  source 1..39: mol_type = other DNA
gagctgcaggatcgggtccgtaacccttattcggtacta

SEQ ID NO: 111 - DNA, 41 bp, synthetic construct
  misc_feature 1..41: note = Target Specific Oligonucleotide
  source 1..41: mol_type = other DNA
acatgagtggtttcgtagcgggtaacccttattcggtacta

SEQ ID NO: 112 - DNA, 40 bp, synthetic construct
  misc_feature 1..40: note = Target Specific Oligonucleotide
  source 1..40: mol_type = other DNA
tgccgatgacatggaactcggtaacccttattcggtacta

SEQ ID NO: 113 - DNA, 43 bp, synthetic construct
  misc_feature 1..43: note = Target Specific Oligonucleotide
  source 1..43: mol_type = other DNA
tggtgtaattgaccttgtaggtagtaacccttattcggtacta

SEQ ID NO: 114 - DNA, 39 bp, synthetic construct
  misc_feature 1..39: note = Target Specific Oligonucleotide
  source 1..39: mol_type = other DNA
cattggccgaaagcaggctgtaacccttattcggtacta

SEQ ID NO: 115 - DNA, 40 bp, synthetic construct
  misc_feature 1..40: note = Target Specific Oligonucleotide
  source 1..40: mol_type = other DNA
gagacctctgccgaaactgggtaacccttattcggtacta

SEQ ID NO: 116 - DNA, 41 bp, synthetic construct
  misc_feature 1..41: note = Target Specific Oligonucleotide
  source 1..41: mol_type = other DNA
agtcttgtgcttcgggtcaaagtaacccttattcggtacta

SEQ ID NO: 117 - DNA, 41 bp, synthetic construct
  misc_feature 1..41: note = Target Specific Oligonucleotide
  source 1..41: mol_type = other DNA
cctcttctcgcctggcatagggtaacccttattcggtacta

SEQ ID NO: 118 - DNA, 41 bp, synthetic construct
  misc_feature 1..41: note = Target Specific Oligonucleotide
  source 1..41: mol_type = other DNA
gtaacggtgaaaatggaccgggtaacccttattcggtacta

SEQ ID NO: 119 - DNA, 42 bp, synthetic construct
  misc_feature 1..42: note = Target Specific Oligonucleotide
  source 1..42: mol_type = other DNA
tccctctaagggattaatgccagtaacccttattcggtacta

SEQ ID NO: 120 - DNA, 43 bp, synthetic construct
  misc_feature 1..43: note = Target Specific Oligonucleotide
  source 1..43: mol_type = other DNA
agttcaagtatcccgcgactagtaacaattagagtgaaatacc

SEQ ID NO: 121 - DNA, 43 bp, synthetic construct
  misc_feature 1..43: note = Target Specific Oligonucleotide
  source 1..43: mol_type = other DNA
gaacgcaggctgtttactgttgtaacaattagagtgaaatacc

SEQ ID NO: 122 - DNA, 44 bp, synthetic construct
  misc_feature 1..44: note = Target Specific Oligonucleotide
  source 1..44: mol_type = other DNA
ggtccaggtaaactaatggctggtaacaattagagtgaaatacc

SEQ ID NO: 123 - DNA, 44 bp, synthetic construct
  misc_feature 1..44: note = Target Specific Oligonucleotide
  source 1..44: mol_type = other DNA
ctctgttgagtttacctcgcaagtaacaattagagtgaaatacc

SEQ ID NO: 124 - DNA, 44 bp, synthetic construct
  misc_feature 1..44: note = Target Specific Oligonucleotide
  source 1..44: mol_type = other DNA
tacttcaactaaccagtccacggtaacaattagagtgaaatacc

SEQ ID NO: 125 - DNA, 44 bp, synthetic construct
  misc_feature 1..44: note = Target Specific Oligonucleotide
  source 1..44: mol_type = other DNA
ccatgagacaaggcttaagactgtaacaattagagtgaaatacc

SEQ ID NO: 126 - DNA, 43 bp, synthetic construct
  misc_feature 1..43: note = Target Specific Oligonucleotide
  source 1..43: mol_type = other DNA
cggccaaagaatagtcgtagcgtaacaattagagtgaaatacc

SEQ ID NO: 127 - DNA, 45 bp, synthetic construct
  misc_feature 1..45: note = Target Specific Oligonucleotide
  source 1..45: mol_type = other DNA
ccatttccctaaggtatgtgtgagtaacaattagagtgaaatacc

SEQ ID NO: 128 - DNA, 46 bp, synthetic construct
  misc_feature 1..46: note = Target Specific Oligonucleotide
  source 1..46: mol_type = other DNA
ctctcatactgttagtgatgtctggtaacaattagagtgaaatacc

SEQ ID NO: 129 - DNA, 42 bp, synthetic construct
  misc_feature 1..42: note = Target Specific Oligonucleotide
  source 1..42: mol_type = other DNA
cagctttgtcccgtgactgtgtaacaattagagtgaaatacc

SEQ ID NO: 130 - DNA, 41 bp, synthetic construct
  misc_feature 1..41: note = Target Specific Oligonucleotide
  source 1..41: mol_type = other DNA
tgctgcaatgctagcagcggtaacaattagagtgaaatacc

SEQ ID NO: 131 - DNA, 46 bp, synthetic construct
  misc_feature 1..46: note = Target Specific Oligonucleotide
  source 1..46: mol_type = other DNA
aagacaggaacctatcaatgtagtgtaacaattagagtgaaatacc

SEQ ID NO: 132 - DNA, 46 bp, synthetic construct
  misc_feature 1..46: note = Target Specific Oligonucleotide
  source 1..46: mol_type = other DNA
tagattagattatgcccaagtcaggtaacaattagagtgaaatacc

SEQ ID NO: 133 - DNA, 46 bp, synthetic construct
  misc_feature 1..46: note = Target Specific Oligonucleotide
  source 1..46: mol_type = other DNA
catgtaacccactttaggtttacagtaacaattagagtgaaatacc

SEQ ID NO: 134 - DNA, 47 bp, synthetic construct
  misc_feature 1..47: note = Target Specific Oligonucleotide
  source 1..47: mol_type = other DNA
ccagtctttcgtattaatgattcaggtaacaattagagtgaaatacc

SEQ ID NO: 135 - DNA, 42 bp, synthetic construct
  misc_feature 1..42: note = Target Specific Oligonucleotide
  source 1..42: mol_type = other DNA
tgcaacccgtctcgtcttcggtaacaattagagtgaaatacc

SEQ ID NO: 136 - DNA, 47 bp, synthetic construct
  misc_feature 1..47: note = Target Specific Oligonucleotide
  source 1..47: mol_type = other DNA
gtgtaggtatcatctgtaatgtacagtaacaattagagtgaaatacc

SEQ ID NO: 137 - DNA, 41 bp, synthetic construct
  misc_feature 1..41: note = Target Specific Oligonucleotide
  source 1..41: mol_type = other DNA
tcccggacttcagtaccgcgtaacaattagagtgaaatacc

SEQ ID NO: 138 - DNA, 41 bp, synthetic construct
  misc_feature 1..41: note = Target Specific Oligonucleotide
  source 1..41: mol_type = other DNA
cgaggaggttgcgaaaggcgtaacaattagagtgaaatacc

SEQ ID NO: 139 - DNA, 49 bp, synthetic construct
  misc_feature 1..49: note = Target Specific Oligonucleotide
  source 1..49: mol_type = other DNA
tatacatatactcaacacttatagagggtaacaattagagtgaaatacc

SEQ ID NO: 140 - DNA, 49 bp, synthetic construct
  misc_feature 1..49: note = Target Specific Oligonucleotide
  source 1..49: mol_type = other DNA
gtaatagataccataatttgtacttgggtaacaattagagtgaaatacc

SEQ ID NO: 141 - DNA, 40 bp, synthetic construct
  misc_feature 1..40: note = Target Specific Oligonucleotide
  source 1..40: mol_type = other DNA
tgctgctgcgctagacccgtaacaattagagtgaaatacc

SEQ ID NO: 142 - DNA, 40 bp, synthetic construct
  misc_feature 1..40: note = Target Specific Oligonucleotide
  source 1..40: mol_type = other DNA
gcgtggcgagccaaagacgtaacaattagagtgaaatacc

SEQ ID NO: 143 - DNA, 40 bp, synthetic construct
  misc_feature 1..40: note = Target Specific Oligonucleotide
  source 1..40: mol_type = other DNA
tccgcggttgttggacgggtaacaattagagtgaaatacc

SEQ ID NO: 144 - DNA, 41 bp, synthetic construct
  misc_feature 1..41: note = Target Specific Oligonucleotide
  source 1..41: mol_type = other DNA
ctgtcacatacgcaaactggtgtaacatcgttatagctaga

SEQ ID NO: 145 - DNA, 41 bp, synthetic construct
  misc_feature 1..41: note = Target Specific Oligonucleotide
  source 1..41: mol_type = other DNA
tcgccatataccggtcaaagagtaacatcgttatagctaga

SEQ ID NO: 146 - DNA, 42 bp, synthetic construct
  misc_feature 1..42: note = Target Specific Oligonucleotide
  source 1..42: mol_type = other DNA
tggatggtgcaataatccgagggtaacatcgttatagctaga

SEQ ID NO: 147 - DNA, 43 bp, synthetic construct
  misc_feature 1..43: note = Target Specific Oligonucleotide
  source 1..43: mol_type = other DNA
agtgctgatcccttaagtatgtcgtaacatcgttatagctaga

SEQ ID NO: 148 - DNA, 43 bp, synthetic construct
  misc_feature 1..43: note = Target Specific Oligonucleotide
  source 1..43: mol_type = other DNA
acctccattaaccaatccagaaggtaacatcgttatagctaga

SEQ ID NO: 149 - DNA, 43 bp, synthetic construct
  misc_feature 1..43: note = Target Specific Oligonucleotide
  source 1..43: mol_type = other DNA
tggtgtacttgacccacttatttgtaacatcgttatagctaga

SEQ ID NO: 150 - DNA, 41 bp, synthetic construct
  misc_feature 1..41: note = Target Specific Oligonucleotide
  source 1..41: mol_type = other DNA
cagaagagaacgtggagcagggtaacatcgttatagctaga

SEQ ID NO: 151 - DNA, 44 bp, synthetic construct
  misc_feature 1..44: note = Target Specific Oligonucleotide
  source 1..44: mol_type = other DNA
tccctgtgaagtttatagacttcagtaacatcgttatagctaga

SEQ ID NO: 152 - DNA, 40 bp, synthetic construct
  misc_feature 1..40: note = Target Specific Oligonucleotide
  source 1..40: mol_type = other DNA
tgtaaaagcaaacgcacgccgtaacatcgttatagctaga

SEQ ID NO: 153 - DNA, 44 bp, synthetic construct
  misc_feature 1..44: note = Target Specific Oligonucleotide
  source 1..44: mol_type = other DNA
attcagatgacgagaaatgatacagtaacatcgttatagctaga

SEQ ID NO: 154 - DNA, 39 bp, synthetic construct
  misc_feature 1..39: note = Target Specific Oligonucleotide
  source 1..39: mol_type = other DNA
tggtcacgccatttccggcgtaacatcgttatagctaga

SEQ ID NO: 155 - DNA, 45 bp, synthetic construct
  misc_feature 1..45: note = Target Specific Oligonucleotide
  source 1..45: mol_type = other DNA
agcaagtataccataaggaaattcagtaacatcgttatagctaga

SEQ ID NO: 156 - DNA, 40 bp, synthetic construct
  misc_feature 1..40: note = Target Specific Oligonucleotide
  source 1..40: mol_type = other DNA
ctcgccgtcctgtcgattttgtaacatcgttatagctaga

SEQ ID NO: 157 - DNA, 38 bp, synthetic construct
  misc_feature 1..38: note = Target Specific Oligonucleotide
  source 1..38: mol_type = other DNA
agcgagccgagaactccggtaacatcgttatagctaga

SEQ ID NO: 158 - DNA, 43 bp, synthetic construct
  misc_feature 1..43: note = Target Specific Oligonucleotide
  source 1..43: mol_type = other DNA
tattttgttcagacaacatggctgtaacatcgttatagctaga

SEQ ID NO: 159 - DNA, 40 bp, synthetic construct
  misc_feature 1..40: note = Target Specific Oligonucleotide
  source 1..40: mol_type = other DNA
ccacttggtacaacggagccgtaacatcgttatagctaga

SEQ ID NO: 160 - DNA, 40 bp, synthetic construct
  misc_feature 1..40: note = Target Specific Oligonucleotide
  source 1..40: mol_type = other DNA
cagaacacctgcgaggagaggtaacatcgttatagctaga

SEQ ID NO: 161 - DNA, 39 bp, synthetic construct
  misc_feature 1..39: note = Target Specific Oligonucleotide
  source 1..39: mol_type = other DNA
ttcatcagcgacgcccctggtaacatcgttatagctaga

SEQ ID NO: 162 - DNA, 41 bp, synthetic construct
  misc_feature 1..41: note = Target Specific Oligonucleotide
  source 1..41: mol_type = other DNA
cctgcaaaaaaacggtcacgtgtaacatcgttatagctaga

SEQ ID NO: 163 - DNA, 41 bp, synthetic construct
  misc_feature 1..41: note = Target Specific Oligonucleotide
  source 1..41: mol_type = other DNA
tgtgggagtcccttaggtcaagtaacatcgttatagctaga

SEQ ID NO: 164 - DNA, 38 bp, synthetic construct
  misc_feature 1..38: note = Target Specific Oligonucleotide
  source 1..38: mol_type = other DNA
gcatcgggagcacgcactgtaacatcgttatagctaga

SEQ ID NO: 165 - DNA, 39 bp, synthetic construct
  misc_feature 1..39: note = Target Specific Oligonucleotide
  source 1..39: mol_type = other DNA
ggctctgcacaacgcttgcgtaacatcgttatagctaga

SEQ ID NO: 166 - DNA, 41 bp, synthetic construct
  misc_feature 1..41: note = Target Specific Oligonucleotide
  source 1..41: mol_type = other DNA
agccaggacacaatagtcagggtaacatcgttatagctaga

SEQ ID NO: 167 - DNA, 41 bp, synthetic construct; identical to SEQ ID NO: 166
  misc_feature 1..41: note = Target Specific Oligonucleotide
  source 1..41: mol_type = other DNA

SEQ ID NO: 168 - DNA, 42 bp, synthetic construct
  misc_feature 1..42: note = Target Specific Oligonucleotide
  source 1..42: mol_type = other DNA
ttgcacatcctacggtcttctgtaacttactacggagttaac

SEQ ID NO: 169 - DNA, 43 bp, synthetic construct
  misc_feature 1..43: note = Target Specific Oligonucleotide
  source 1..43: mol_type = other DNA
gtagctcattcgcaaatcttgggtaacttactacggagttaac

SEQ ID NO: 170 - DNA, 41 bp, synthetic construct
  misc_feature 1..41: note = Target Specific Oligonucleotide
  source 1..41: mol_type = other DNA
cctttaagcgcgtcgtgtccgtaacttactacggagttaac

SEQ ID NO: 171 - DNA, 39 bp, synthetic construct
  misc_feature 1..39: note = Target Specific Oligonucleotide
  source 1..39: mol_type = other DNA
cctcgacgcatgatgccggtaacttactacggagttaac

SEQ ID NO: 172 - DNA, 40 bp, synthetic construct
  misc_feature 1..40: note = Target Specific Oligonucleotide
  source 1..40: mol_type = other DNA
gccccatggctcgtgtagggtaacttactacggagttaac

SEQ ID NO: 173 - DNA, 42 bp, synthetic construct
  misc_feature 1..42: note = Target Specific Oligonucleotide
  source 1..42: mol_type = other DNA
ccaattgtgttccggcaagttgtaacttactacggagttaac

SEQ ID NO: 174 - DNA, 43 bp, synthetic construct
  misc_feature 1..43: note = Target Specific Oligonucleotide
  source 1..43: mol_type = other DNA
gataggatttggtcggaaacctgtaacttactacggagttaac

SEQ ID NO: 175 - DNA, 41 bp, synthetic construct
  misc_feature 1..41: note = Target Specific Oligonucleotide
  source 1..41: mol_type = other DNA
tagttgccaacggtgttgtagtaacttactacggagttaac

SEQ ID NO: 176 - DNA, 42 bp, synthetic construct
  misc_feature 1..42: note = Target Specific Oligonucleotide
  source 1..42: mol_type = other DNA
cttggcctatgcggaagtaacgtaacttactacggagttaac

SEQ ID NO: 177 - DNA, 41 bp, synthetic construct
  misc_feature 1..41: note = Target Specific Oligonucleotide
  source 1..41: mol_type = other DNA
ctcgcagcgataggaaccatgtaacttactacggagttaac

SEQ ID NO: 178 - DNA, 44 bp, synthetic construct
  misc_feature 1..44: note = Target Specific Oligonucleotide
  source 1..44: mol_type = other DNA
tttgcattcgtccatatcaactggtaacttactacggagttaac

SEQ ID NO: 179 - DNA, 43 bp, synthetic construct
  misc_feature 1..43: note = Target Specific Oligonucleotide
  source 1..43: mol_type = other DNA
tcaatatcaacgggtaaaccgggtaacttactacggagttaac

SEQ ID NO: 180 - DNA, 45 bp, synthetic construct
  misc_feature 1..45: note = Target Specific Oligonucleotide
  source 1..45: mol_type = other DNA
ttgttactgacgtgggaaatattggtaacttactacggagttaac

SEQ ID NO: 181 - DNA, 40 bp, synthetic construct
  misc_feature 1..40: note = Target Specific Oligonucleotide
  source 1..40: mol_type = other DNA
tctccgctgatacccgggtgtaacttactacggagttaac

SEQ ID NO: 182 - DNA, 42 bp, synthetic construct
  misc_feature 1..42: note = Target Specific Oligonucleotide
  source 1..42: mol_type = other DNA
ggccagtcaccgaaatttcatgtaacttactacggagttaac

SEQ ID NO: 183 - DNA, 43 bp, synthetic construct
  misc_feature 1..43: note = Target Specific Oligonucleotide
  source 1..43: mol_type = other DNA
agttcgtagcctatctcacactgtaacttactacggagttaac

SEQ ID NO: 184 - DNA, 42 bp, synthetic construct
  misc_feature 1..42: note = Target Specific Oligonucleotide
  source 1..42: mol_type = other DNA
cacattcccgtacgtttgctggtaacttactacggagttaac

SEQ ID NO: 185 - DNA, 45 bp, synthetic construct
  misc_feature 1..45: note = Target Specific Oligonucleotide
  source 1..45: mol_type = other DNA
agtgagtccctatgtatcctttctgtaacttactacggagttaac

SEQ ID NO: 186 - DNA, 44 bp, synthetic construct
  misc_feature 1..44: note = Target Specific Oligonucleotide
  source 1..44: mol_type = other DNA
aagcattataacgtgatccacaggtaacttactacggagttaac

SEQ ID NO: 187 - DNA, 38 bp, synthetic construct
  misc_feature 1..38: note = Target Specific Oligonucleotide
  source 1..38: mol_type = other DNA
tgcgccctgaagcgcacgtaacttactacggagttaac

SEQ ID NO: 188 - DNA, 47 bp, synthetic construct
  misc_feature 1..47: note = Target Specific Oligonucleotide
  source 1..47: mol_type = other DNA
taaaaaatagcacgattacagtatacgtaacttactacggagttaac

SEQ ID NO: 189 - DNA, 44 bp, synthetic construct
  misc_feature 1..44: note = Target Specific Oligonucleotide
  source 1..44: mol_type = other DNA
catatcgacggattgagcctaacgtaacttactacggagttaac

SEQ ID NO: 190 - DNA, 42 bp, synthetic construct
  misc_feature 1..42: note = Target Specific Oligonucleotide
  source 1..42: mol_type = other DNA
cggtttctcgcgagagaaatagtaacttactacggagttaac

SEQ ID NO: 191 - DNA, 43 bp, synthetic construct
  misc_feature 1..43: note = Target Specific Oligonucleotide
  source 1..43: mol_type = other DNA
cttcccatctcgtgtaacatgagtaacttactacggagttaac

SEQ ID NO: 192 - DNA, 41 bp, synthetic construct
  misc_feature 1..41: note = Target Specific Oligonucleotide
  source 1..41: mol_type = other DNA
gcatttcacatcggactgtaccgtaacttcgaaacggaaac

SEQ ID NO: 193 - DNA, 38 bp, synthetic construct
  misc_feature 1..38: note = Target Specific Oligonucleotide
  source 1..38: mol_type = other DNA
tggaattctcggcggaccagtaacttcgaaacggaaac

SEQ ID NO: 194 - DNA, 41 bp, synthetic construct
  misc_feature 1..41: note = Target Specific Oligonucleotide
  source 1..41: mol_type = other DNA
gaagtggaaatacgacctttgcgtaacttcgaaacggaaac

SEQ ID NO: 195 - DNA, 39 bp, synthetic construct
  misc_feature 1..39: note = Target Specific Oligonucleotide
  source 1..39: mol_type = other DNA
gctggtcccttgcgtaacatgtaacttcgaaacggaaac

SEQ ID NO: 196 - DNA, 43 bp, synthetic construct
  misc_feature 1..43: note = Target Specific Oligonucleotide
  source 1..43: mol_type = other DNA
ttttcatctattcgagatgctcccgtaacttcgaaacggaaac

SEQ ID NO: 197 - DNA, 40 bp, synthetic construct
  misc_feature 1..40: note = Target Specific Oligonucleotide
  source 1..40: mol_type = other DNA
tattcatcccgtggggtagtagtaacttcgaaacggaaac

SEQ ID NO: 198 - DNA, 42 bp, synthetic construct
  misc_feature 1..42: note = Target Specific Oligonucleotide
  source 1..42: mol_type = other DNA
taaaaataggcccggatttgtctgtaacttcgaaacggaaac

SEQ ID NO: 199 - DNA, 42 bp, synthetic construct
  misc_feature 1..42: note = Target Specific Oligonucleotide
  source 1..42: mol_type = other DNA
tccaaccttgacgacaagatagggtaacttcgaaacggaaac

SEQ ID NO: 200 - DNA, 40 bp, synthetic construct
  misc_feature 1..40: note = Target Specific Oligonucleotide
  source 1..40: mol_type = other DNA
aggcaacagtcgaaccattctgtaacttcgaaacggaaac

SEQ ID NO: 201 - DNA, 40 bp, synthetic construct
  misc_feature 1..40: note = Target Specific Oligonucleotide
  source 1..40: mol_type = other DNA
gcttcatttgcgactgctcttgtaacttcgaaacggaaac

SEQ ID NO: 202 - DNA, 41 bp, synthetic construct
  misc_feature 1..41: note = Target Specific Oligonucleotide
  source 1..41: mol_type = other DNA
catcaggacgcttgtattggtggtaacttcgaaacggaaac

SEQ ID NO: 203 - DNA, 41 bp, synthetic construct
  misc_feature 1..41: note = Target Specific Oligonucleotide
  source 1..41: mol_type = other DNA
atcttcaatccgagaatccagcgtaacttcgaaacggaaac

SEQ ID NO: 204 - DNA, 42 bp, synthetic construct
  misc_feature 1..42: note = Target Specific Oligonucleotide
  source 1..42: mol_type = other DNA
ctgtagtgtggtagtaaggaagagtaacttcgaaacggaaac

SEQ ID NO: 205 - DNA, 42 bp, synthetic construct
  misc_feature 1..42: note = Target Specific Oligonucleotide
  source 1..42: mol_type = other DNA
gaacaccttacttacaacacctggtaacttcgaaacggaaac

SEQ ID NO: 206 - DNA, 43 bp, synthetic construct
  misc_feature 1..43: note = Target Specific Oligonucleotide
  source 1..43: mol_type = other DNA
gtacattgtacaccgttacaatgggtaacttcgaaacggaaac

SEQ ID NO: 207 - DNA, 42 bp, synthetic construct
  misc_feature 1..42: note = Target Specific Oligonucleotide
  source 1..42: mol_type = other DNA
tttcaagtcgtctatgttagctggtaacttcgaaacggaaac

SEQ ID NO: 208 - DNA, 44 bp, synthetic construct
  misc_feature 1..44: note = Target Specific Oligonucleotide
  source 1..44: mol_type = other DNA
caaagcaactatatgaagcttcattgtaacttcgaaacggaaac

SEQ ID NO: 209 - DNA, 42 bp, synthetic construct
  misc_feature 1..42: note = Target Specific Oligonucleotide
  source 1..42: mol_type = other DNA
catacttctatcgagagctcagggtaacttcgaaacggaaac

SEQ ID NO: 210 - DNA, 43 bp, synthetic construct
  misc_feature 1..43: note = Target Specific Oligonucleotide
  source 1..43: mol_type = other DNA
acgaagaaatcgagtaggtctagggtaacttcgaaacggaaac

SEQ ID NO: 211 - DNA, 41 bp, synthetic construct
  misc_feature 1..41: note = Target Specific Oligonucleotide
  source 1..41: mol_type = other DNA
gaatcattgagtcgacccttcagtaacttcgaaacggaaac

SEQ ID NO: 212 - DNA, 41 bp, synthetic construct
  misc_feature 1..41: note = Target Specific Oligonucleotide
  source 1..41: mol_type = other DNA
tgatgtgcttaagtagtgcagcgtaacttcgaaacggaaac

SEQ ID NO: 213 - DNA, 41 bp, synthetic construct
  misc_feature 1..41: note = Target Specific Oligonucleotide
  source 1..41: mol_type = other DNA
tccacggcatgatacatacaacgtaacttcgaaacggaaac

SEQ ID NO: 214 - DNA, 40 bp, synthetic construct
  misc_feature 1..40: note = Target Specific Oligonucleotide
  source 1..40: mol_type = other DNA
tctcagagcatcccgaatccagtaacttcgaaacggaaac

SEQ ID NO: 215 - DNA, 42 bp, synthetic construct
  misc_feature 1..42: note = Target Specific Oligonucleotide
  source 1..42: mol_type = other DNA
gtggaacgaagagtaggtagtttgtaacttcgaaacggaaac

SEQ ID NO: 216 - DNA, 39 bp, synthetic construct
  misc_feature 1..39: note = Target Specific Oligonucleotide
  source 1..39: mol_type = other DNA
gatcaatactggacggagtcaggtaacctcgtcggatca

SEQ ID NO: 217 - DNA, 38 bp, synthetic construct
  misc_feature 1..38: note = Target Specific Oligonucleotide
  source 1..38: mol_type = other DNA
gagcttgttactcgtgccttggtaacctcgtcggatca

SEQ ID NO: 218 - DNA, 37 bp, synthetic construct
  misc_feature 1..37: note = Target Specific Oligonucleotide
  source 1..37: mol_type = other DNA
cttcttacacttgcggacgcgtaacctcgtcggatca

SEQ ID NO: 219 - DNA, 41 bp, synthetic construct
  misc_feature 1..41: note = Target Specific Oligonucleotide
  source 1..41: mol_type = other DNA
caatacctattccgttacacacttgtaacctcgtcggatca

SEQ ID NO: 220 - DNA, 39 bp, synthetic construct
  misc_feature 1..39: note = Target Specific Oligonucleotide
  source 1..39: mol_type = other DNA
gctccttcagtccggttttattgtaacctcgtcggatca

SEQ ID NO: 221 - DNA, 36 bp, synthetic construct
  misc_feature 1..36: note = Target Specific Oligonucleotide
  source 1..36: mol_type = other DNA
gacgcacgagccgtgatctgtaacctcgtcggatca

SEQ ID NO: 222 - DNA, 41 bp, synthetic construct
  misc_feature 1..41: note = Target Specific Oligonucleotide
  source 1..41: mol_type = other DNA
gactgctaaggcataggaattttcgtaacctcgtcggatca

SEQ ID NO: 223 - DNA, 39 bp, synthetic construct
  misc_feature 1..39: note = Target Specific Oligonucleotide
  source 1..39: mol_type = other DNA
caccacataattacggggacacgtaacctcgtcggatca

SEQ ID NO: 224 - DNA, 34 bp, synthetic construct
  misc_feature 1..34: note = Target Specific Oligonucleotide
  source 1..34: mol_type = other DNA
cggcaaggcccttcgcagtaacctcgtcggatca

SEQ ID NO: 225 - DNA, 37 bp, synthetic construct
  misc_feature 1..37: note = Target Specific Oligonucleotide
  source 1..37: mol_type = other DNA
tccatctggtacgtggtggggtaacctcgtcggatca

SEQ ID NO: 226 - DNA, 38 bp, synthetic construct
  misc_feature 1..38: note = Target Specific Oligonucleotide
  source 1..38: mol_type = other DNA
gtcctgccgcgtatgatttctgtaacctcgtcggatca

SEQ ID NO: 227 - DNA, 37 bp, synthetic construct
  misc_feature 1..37: note = Target Specific Oligonucleotide
  source 1..37: mol_type = other DNA
tgttcaggctgacgactgcagtaacctcgtcggatca

SEQ ID NO: 228 - DNA, 36 bp, synthetic construct
  misc_feature 1..36: note = Target Specific Oligonucleotide
  source 1..36: mol_type = other DNA
gcatggaggtccgtcctgtgtaacctcgtcggatca

SEQ ID NO: 229 - DNA, 38 bp, synthetic construct
  misc_feature 1..38: note = Target Specific Oligonucleotide
  source 1..38: mol_type = other DNA
ttgagggagcgtaatcccaaggtaacctcgtcggatca

SEQ ID NO: 230 - DNA, 36 bp, synthetic construct
  misc_feature 1..36: note = Target Specific Oligonucleotide
  source 1..36: mol_type = other DNA
ccggcgtctgcgtacttccgtaacctcgtcggatca

SEQ ID NO: 231 - DNA, 39 bp, synthetic construct
  misc_feature 1..39: note = Target Specific Oligonucleotide
  source 1..39: mol_type = other DNA
cgactatctgcgtctatcatccgtaacctcgtcggatca

SEQ ID NO: 232 - DNA, 40 bp, synthetic construct
  misc_feature 1..40: note = Target Specific Oligonucleotide
  source 1..40: mol_type = other DNA
gagaattcgatgatcaactcacggtaacctcgtcggatca

SEQ ID NO: 233 - DNA, 35 bp, synthetic construct
  misc_feature 1..35: note = Target Specific Oligonucleotide
  source 1..35: mol_type = other DNA
tggcctgtcgtccggtctgtaacctcgtcggatca

SEQ ID NO: 234 - DNA, 38 bp, synthetic construct
  misc_feature 1..38: note = Target Specific Oligonucleotide
  source 1..38: mol_type = other DNA
cagggattccgtcatatggctgtaacctcgtcggatca

SEQ ID NO: 235 - DNA, 40 bp, synthetic construct
  misc_feature 1..40: note = Target Specific Oligonucleotide
  source 1..40: mol_type = other DNA
agacatcgatggtacatatgggtgtaacctcgtcggatca

SEQ ID NO: 236 - DNA, 37 bp, synthetic construct
  misc_feature 1..37: note = Target Specific Oligonucleotide
  source 1..37: mol_type = other DNA
tctgagctgtatcgctgcaagtaacctcgtcggatca

SEQ ID NO: 237 - DNA, 37 bp, synthetic construct
  misc_feature 1..37: note = Target Specific Oligonucleotide
  source 1..37: mol_type = other DNA
tcttaggcccattcgttggagtaacctcgtcggatca

SEQ ID NO: 238 - DNA, 37 bp, synthetic construct
  misc_feature 1..37: note = Target Specific Oligonucleotide
  source 1..37: mol_type = other DNA
ttatacaccgtgccgaacgcgtaacctcgtcggatca

SEQ ID NO: 239 - DNA, 37 bp, synthetic construct
  misc_feature 1..37: note = Target Specific Oligonucleotide
  source 1..37: mol_type = other DNA
atgccctttgcgatctgcacgtaacctcgtcggatca

SEQ ID NO: 240 - DNA, 42 bp, synthetic construct
  misc_feature 1..42: note = Target Specific Oligonucleotide
  source 1..42: mol_type = other DNA
ggcagaattccgaagttcagcgtaacataatcgtagtttcgg

SEQ ID NO: 241 - DNA, 42 bp, synthetic construct
  misc_feature 1..42: note = Target Specific Oligonucleotide
  source 1..42: mol_type = other DNA
gtttccttcacgacaggtgtggtaacataatcgtagtttcgg

SEQ ID NO: 242 - DNA, 44 bp, synthetic construct
  misc_feature 1..44: note = Target Specific Oligonucleotide
  source 1..44: mol_type = other DNA
ctggtagaaatgcgactaaagacgtaacataatcgtagtttcgg

SEQ ID NO: 243 - DNA, 44 bp, synthetic construct
  misc_feature 1..44: note = Target Specific Oligonucleotide
  source 1..44: mol_type = other DNA
tgaccagcatcgtttcatctaatgtaacataatcgtagtttcgg

SEQ ID NO: 244 - DNA, 42 bp, synthetic construct
  misc_feature 1..42: note = Target Specific Oligonucleotide
  source 1..42: mol_type = other DNA
ttcgaagttcaaccgagtgacgtaacataatcgtagtttcgg

SEQ ID NO: 245 - DNA, 42 bp, synthetic construct
  misc_feature 1..42: note = Target Specific Oligonucleotide
  source 1..42: mol_type = other DNA
ccaccaatccaatgcggaattgtaacataatcgtagtttcgg

SEQ ID NO: 246 - DNA, 42 bp, synthetic construct
  misc_feature 1..42: note = Target Specific Oligonucleotide
  source 1..42: mol_type = other DNA
agactcggtgccattcgtattgtaacataatcgtagtttcgg

SEQ ID NO: 247 - DNA, 42 bp, synthetic construct
  misc_feature 1..42: note = Target Specific Oligonucleotide
  source 1..42: mol_type = other DNA
ataactgctaactgcgcaaccgtaacataatcgtagtttcgg

SEQ ID NO: 248 - DNA, 43 bp, synthetic construct
  misc_feature 1..43: note = Target Specific Oligonucleotide
  source 1..43: mol_type = other DNA
gtagtgaggccgcttataaccagtaacataatcgtagtttcgg

SEQ ID NO: 249 - DNA, 43 bp, synthetic construct
  misc_feature 1..43: note = Target Specific Oligonucleotide
  source 1..43: mol_type = other DNA
ggtgatgattcgatggagtgaagtaacataatcgtagtttcgg

SEQ ID NO: 250 - DNA, 42 bp, synthetic construct
  misc_feature 1..42: note = Target Specific Oligonucleotide
  source 1..42: mol_type = other DNA
ctgctgctttacgtttggtgcgtaacataatcgtagtttcgg

SEQ ID NO: 251 - DNA, 43 bp, synthetic construct
  misc_feature 1..43: note = Target Specific Oligonucleotide
  source 1..43: mol_type = other DNA
tcatcaaccacgtctttggatagtaacataatcgtagtttcgg

SEQ ID NO: 252 - DNA, 44 bp, synthetic construct
  misc_feature 1..44: note = Target Specific Oligonucleotide
  source 1..44: mol_type = other DNA
aggcagatcttaaagtgttggttgtaacataatcgtagtttcgg

SEQ ID NO: 253 - DNA, 43 bp, synthetic construct
  misc_feature 1..43: note = Target Specific Oligonucleotide
  source 1..43: mol_type = other DNA
tgagggcttatacgaaagcaaggtaacataatcgtagtttcgg

SEQ ID NO: 254 - DNA, 44 bp, synthetic construct
  misc_feature 1..44: note = Target Specific Oligonucleotide
  source 1..44: mol_type = other DNA
gctcagtactgactttggtatgtgtaacataatcgtagtttcgg

SEQ ID NO: 255 - DNA, 45 bp, synthetic construct
  misc_feature 1..45: note = Target Specific Oligonucleotide
  source 1..45: mol_type = other DNA
cagtcaatcattagatccacatctgtaacataatcgtagtttcgg

SEQ ID NO: 256 - DNA, 40 bp, synthetic construct
  misc_feature 1..40: note = Target Specific Oligonucleotide
  source 1..40: mol_type = other DNA
ggaagctgctcgtcgaagcgtaacataatcgtagtttcgg

SEQ ID NO: 257 - DNA, 47 bp, synthetic construct
  misc_feature 1..47: note = Target Specific Oligonucleotide
  source 1..47: mol_type = other DNA
gagaagatacttatagcttcttgtctgtaacataatcgtagtttcgg

SEQ ID NO: 258 - DNA, 45 bp, synthetic construct
  misc_feature 1..45: note = Target Specific Oligonucleotide
  source 1..45: mol_type = other DNA
tcaatgctatctaactgatgaagagtaacataatcgtagtttcgg

SEQ ID NO: 259 - DNA, 46 bp, synthetic construct
  misc_feature 1..46: note = Target Specific Oligonucleotide
  source 1..46: mol_type = other DNA
atcttcccaattgatgtaagtacttgtaacataatcgtagtttcgg

SEQ ID NO: 260 - DNA, 40 bp, synthetic construct
  misc_feature 1..40: note = Target Specific Oligonucleotide
  source 1..40: mol_type = other DNA
catcacagtccgagacgccgtaacataatcgtagtttcgg

SEQ ID NO: 261 - DNA, 40 bp, synthetic construct
  misc_feature 1..40: note = Target Specific Oligonucleotide
  source 1..40: mol_type = other DNA
cattccaccggcctgtgcggtaacataatcgtagtttcgg

SEQ ID NO: 262 - DNA, 44 bp, synthetic construct
  misc_feature 1..44: note = Target Specific Oligonucleotide
  source 1..44: mol_type = other DNA
ggacagcactactctagagtaaggtaacataatcgtagtttcgg

SEQ ID NO: 263 - DNA, 43 bp, synthetic construct
  misc_feature 1..43: note = Target Specific Oligonucleotide
  source 1..43: mol_type = other DNA
tgccaagtaacttagcacacccgtaacataatcgtagtttcgg

SEQ ID NO: 264 - DNA, 38 bp, synthetic construct
  misc_feature 1..38: note = Target Specific Oligonucleotide
  source 1..38: mol_type = other DNA
gtgccacctttcaccgtgagtaaccggtagaattacgg

SEQ ID NO: 265 - DNA, 38 bp, synthetic construct
  misc_feature 1..38: note = Target Specific Oligonucleotide
  source 1..38: mol_type = other DNA
ccgcaggtacgacttgcctgtaaccggtagaattacgg

SEQ ID NO: 266 - DNA, 40 bp, synthetic construct
  misc_feature 1..40: note = Target Specific Oligonucleotide
  source 1..40: mol_type = other DNA
tgggcttcaatcagatggtcagtaaccggtagaattacgg

SEQ ID NO: 267 - DNA, 41 bp, synthetic construct
  misc_feature 1..41: note = Target Specific Oligonucleotide
  source 1..41: mol_type = other DNA
agaacaccagggtacgcatagtgtaaccggtagaattacgg

SEQ ID NO: 268 - DNA, 38 bp, synthetic construct
  misc_feature 1..38: note = Target Specific Oligonucleotide
  source 1..38: mol_type = other DNA
tctccgagagtgtcagcgggtaaccggtagaattacgg

SEQ ID NO: 269 - DNA, 38 bp, synthetic construct
  misc_feature 1..38: note = Target Specific Oligonucleotide
  source 1..38: mol_type = other DNA
gtcttcccggccggtcttggtaaccggtagaattacgg

SEQ ID NO: 270 - DNA, 39 bp, synthetic construct
  misc_feature 1..39: note = Target Specific Oligonucleotide
  source 1..39: mol_type = other DNA
catgttgcagattgtcgccagtaaccggtagaattacgg

SEQ ID NO: 271 - DNA, 39 bp, synthetic construct
  misc_feature 1..39: note = Target Specific Oligonucleotide
  source 1..39: mol_type = other DNA
ggttcagtcgtttgcgaacagtaaccggtagaattacgg

SEQ ID NO: 272 - DNA, 41 bp, synthetic construct
  misc_feature 1..41: note = Target Specific Oligonucleotide
  source 1..41: mol_type = other DNA
agctaccaattagacccactcggtaaccggtagaattacgg

SEQ ID NO: 273 - DNA, 40 bp, synthetic construct
  misc_feature 1..40: note = Target Specific Oligonucleotide
  source 1..40: mol_type = other DNA
cgtagttctcgtctccgatcagtaaccggtagaattacgg

SEQ ID NO: 274 - DNA, 39 bp, synthetic construct
  misc_feature 1..39: note = Target Specific Oligonucleotide
  source 1..39: mol_type = other DNA
ggagctgaacttgacgccaggtaaccggtagaattacgg

SEQ ID NO: 275 - DNA, 40 bp, synthetic construct
  misc_feature 1..40: note = Target Specific Oligonucleotide
  source 1..40: mol_type = other DNA
taatggatgtactcgttgggcgtaaccggtagaattacgg

SEQ ID NO: 276 - DNA, 38 bp, synthetic construct
  misc_feature 1..38: note = Target Specific Oligonucleotide
  source 1..38: mol_type = other DNA
tctgtgcatagccgtcccggtaaccggtagaattacgg

SEQ ID NO: 277 - DNA, 38 bp, synthetic construct
  misc_feature 1..38: note = Target Specific Oligonucleotide
  source 1..38: mol_type = other DNA
tggctggacggatcggatcgtaaccggtagaattacgg

SEQ ID NO: 278 - DNA, 37 bp, synthetic construct
  misc_feature 1..37: note = Target Specific Oligonucleotide
  source 1..37: mol_type = other DNA
ggtttgcgtcgttgcggcgtaaccggtagaattacgg

SEQ ID NO: 279 - DNA, 39 bp, synthetic construct
  misc_feature 1..39: note = Target Specific Oligonucleotide
  source 1..39: mol_type = other DNA
tctctggggacgtgacaaaggtaaccggtagaattacgg

SEQ ID NO: 280 - DNA, 42 bp, synthetic construct
  misc_feature 1..42: note = Target Specific Oligonucleotide
  source 1..42: mol_type = other DNA
gaattcatcagctagattggcaagtaaccggtagaattacgg

SEQ ID NO: 281 - DNA, 38 bp, synthetic construct
  misc_feature 1..38: note = Target Specific Oligonucleotide
  source 1..38: mol_type = other DNA
tcactccgtgggctaagcggtaaccggtagaattacgg

SEQ ID NO: 282 - DNA, 40 bp, synthetic construct
  misc_feature 1..40: note = Target Specific Oligonucleotide
  source 1..40: mol_type = other DNA
tgtaagggaacacggaagtgggtaaccggtagaattacgg

SEQ ID NO: 283 - DNA, 38 bp, synthetic construct
  misc_feature 1..38: note = Target Specific Oligonucleotide
  source 1..38: mol_type = other DNA
ctcaatggtggcgcggatcgtaaccggtagaattacgg

SEQ ID NO: 284 - DNA, 40 bp, synthetic construct
  misc_feature 1..40: note = Target Specific Oligonucleotide
  source 1..40: mol_type = other DNA
aaccactcaatctgcgtctcggtaaccggtagaattacgg

SEQ ID NO: 285 - DNA, 39 bp, synthetic construct
  misc_feature 1..39: note = Target Specific Oligonucleotide
  source 1..39: mol_type = other DNA
gctgtagggcgccattttgtgtaaccggtagaattacgg

SEQ ID NO: 286 - DNA, 38 bp, synthetic construct
  misc_feature 1..38: note = Target Specific Oligonucleotide
  source 1..38: mol_type = other DNA
tgagtgacggcattgcgcagtaaccggtagaattacgg

SEQ ID NO: 287 - DNA, 39 bp, synthetic construct
  misc_feature 1..39: note = Target Specific Oligonucleotide
  source 1..39: mol_type = other DNA
caaagtggctcatcgccaccgtaaccggtagaattacgg

SEQ ID NO: 288 - DNA, 45 bp, synthetic construct
  misc_feature 1..45: note = Target Specific Oligonucleotide
  source 1..45: mol_type = other DNA
tctatatgctaaatgtattgccatggtaacgcttctcataacact

SEQ ID NO: 289 - DNA, 43 bp, synthetic construct
  misc_feature 1..43: note = Target Specific Oligonucleotide
  source 1..43: mol_type = other DNA
ctatgaaacttcgtggtcactccgtaacgcttctcataacact

SEQ ID NO: 290 - DNA, 43 bp, synthetic construct
  misc_feature 1..43: note = Target Specific Oligonucleotide
  source 1..43: mol_type = other DNA
aactaactcatctgcagtaccatgtaacgcttctcataacact

SEQ ID NO: 291 - DNA, 43 bp, synthetic construct
  misc_feature 1..43: note = Target Specific Oligonucleotide
  source 1..43: mol_type = other DNA
aaaacctgcttgatccacattctgtaacgcttctcataacact

SEQ ID NO: 292 - DNA, 45 bp, synthetic construct
  misc_feature 1..45: note = Target Specific Oligonucleotide
  source 1..45: mol_type = other DNA
acattaacaaatcactcttgattcagtaacgcttctcataacact

SEQ ID NO: 293 - DNA, 43 bp, synthetic construct
  misc_feature 1..43: note = Target Specific Oligonucleotide
  source 1..43: mol_type = other DNA
ttttgcttagctcatggtaaacagtaacgcttctcataacact

SEQ ID NO: 294 - DNA, 45 bp, synthetic construct
  misc_feature 1..45: note = Target Specific Oligonucleotide
  source 1..45: mol_type = other DNA
gaggagctgttggataaataattttgtaacgcttctcataacact

SEQ ID NO: 295 - DNA, 43 bp, synthetic construct
  misc_feature 1..43: note = Target Specific Oligonucleotide
  source 1..43: mol_type = other DNA
aagcaggcaggtattgtatgattgtaacgcttctcataacact

SEQ ID NO: 296 - DNA, 45 bp, synthetic construct
  misc_feature 1..45: note = Target Specific Oligonucleotide
  source 1..45: mol_type = other DNA
gcaacttatatatcagtggtgaatggtaacgcttctcataacact

SEQ ID NO: 297 - DNA, 45 bp, synthetic construct
  misc_feature 1..45: note = Target Specific Oligonucleotide
  source 1..45: mol_type = other DNA
agattatgtatgcatgagaaccaacgtaacgcttctcataacact

SEQ ID NO: 298 - DNA, 45 bp, synthetic construct
  misc_feature 1..45: note = Target Specific Oligonucleotide
  source 1..45: mol_type = other DNA
gatcatgactctccttatggttaatgtaacgcttctcataacact

SEQ ID NO: 299 - DNA, 43 bp, synthetic construct
  misc_feature 1..43: note = Target Specific Oligonucleotide
  source 1..43: mol_type = other DNA
tgtgaaaccggtttataaacctagtaacgcttctcataacact

SEQ ID NO: 300 - DNA, 46 bp, synthetic construct
  misc_feature 1..46: note = Target Specific Oligonucleotide
  source 1..46: mol_type = other DNA
aataagattagctactgtctacagtggtaacgcttctcataacact

SEQ ID NO: 301 - DNA, 45 bp, synthetic construct
  misc_feature 1..45: note = Target Specific Oligonucleotide
  source 1..45: mol_type = other DNA
taaacaaatagtgatacatccacacgtaacgcttctcataacact

SEQ ID NO: 302 - DNA, 45 bp, synthetic construct
  misc_feature 1..45: note = Target Specific Oligonucleotide
  source 1..45: mol_type = other DNA
ttcagtcatctaacaatgtattcctgtaacgcttctcataacact

SEQ ID NO: 303 - DNA, 43 bp, synthetic construct
  misc_feature 1..43: note = Target Specific Oligonucleotide
  source 1..43: mol_type = other DNA
agctgtgggaaagtctttaactcgtaacgcttctcataacact

SEQ ID NO: 304 - DNA, 46 bp, synthetic construct
  misc_feature 1..46: note = Target Specific Oligonucleotide
  source 1..46: mol_type = other DNA
atagatgaactattgatgtacacaacgtaacgcttctcataacact

SEQ ID NO: 305 - DNA, 45 bp, synthetic construct
  misc_feature 1..45: note = Target Specific Oligonucleotide
  source 1..45: mol_type = other DNA
tacagatgaaattgagacctaaaacgtaacgcttctcataacact

SEQ ID NO: 306 - DNA, 45 bp, synthetic construct
  misc_feature 1..45: note = Target Specific Oligonucleotide
  source 1..45: mol_type = other DNA
agcaatttgggttaacagaaatagagtaacgcttctcataacact

SEQ ID NO: 307 - DNA, 46 bp, synthetic construct
  misc_feature 1..46: note = Target Specific Oligonucleotide
  source 1..46: mol_type = other DNA
aatccaatgggataagtactattagtgtaacgcttctcataacact

SEQ ID NO: 308 - DNA, 45 bp, synthetic construct
  misc_feature 1..45: note = Target Specific Oligonucleotide
  source 1..45: mol_type = other DNA
aatgttattccgtggaaaattacatgtaacgcttctcataacact

SEQ ID NO: 309 - DNA, 47 bp, synthetic construct
  misc_feature 1..47: note = Target Specific Oligonucleotide
  source 1..47: mol_type = other DNA
ttacagaattgtgtctgaaaaattatggtaacgcttctcataacact

SEQ ID NO: 310 - DNA, 40 bp, synthetic construct
  misc_feature 1..40: note = Target Specific Oligonucleotide
  source 1..40: mol_type = other DNA
atcagagaggcgctatgcctgtaacgcttctcataacact

SEQ ID NO: 311 - DNA, 38 bp, synthetic construct
  misc_feature 1..38: note = Target Specific Oligonucleotide
  source 1..38: mol_type = other DNA
cggcgacacgatacagcggtaacgcttctcataacact

SEQ ID NO: 312 - DNA, 40 bp, synthetic construct
  misc_feature 1..40: note = Target Specific Oligonucleotide
  source 1..40: mol_type = other DNA
cacttcaaatgcgcaacaagcgtaacgtcgctgaaaaatc

SEQ ID NO: 313 - DNA, 39 bp, synthetic construct
  misc_feature 1..39: note = Target Specific Oligonucleotide
  source 1..39: mol_type = other DNA
gtaagcactgcgcaagacaagtaacgtcgctgaaaaatc

SEQ ID NO: 314 - DNA, 41 bp, synthetic construct
  misc_feature 1..41: note = Target Specific Oligonucleotide
  source 1..41: mol_type = other DNA
gtgatgagctcgacaggatattgtaacgtcgctgaaaaatc

SEQ ID NO: 315 - DNA, 37 bp, synthetic construct
  misc_feature 1..37: note = Target Specific Oligonucleotide
  source 1..37: mol_type = other DNA
atggcgtcgtcggcacacgtaacgtcgctgaaaaatc

SEQ ID NO: 316 - DNA, 40 bp, synthetic construct
  misc_feature 1..40: note = Target Specific Oligonucleotide
  source 1..40: mol_type = other DNA
tttacaacagcgtggcaagtggtaacgtcgctgaaaaatc

SEQ ID NO: 317 - DNA, 40 bp, synthetic construct
  misc_feature 1..40: note = Target Specific Oligonucleotide
  source 1..40: mol_type = other DNA
aggcatgaagtgagacaatgcgtaacgtcgctgaaaaatc

SEQ ID NO: 318 - DNA, 41 bp, synthetic construct
  misc_feature 1..41: note = Target Specific Oligonucleotide
  source 1..41: mol_type = other DNA
cctggctagtggtatatgtcacgtaacgtcgctgaaaaatc

SEQ ID NO: 319 - DNA, 39 bp, synthetic construct
  misc_feature 1..39: note = Target Specific Oligonucleotide
  source 1..39: mol_type = other DNA
gctgatgatgttcaagcgcagtaacgtcgctgaaaaatc

SEQ ID NO: 320 - DNA, 41 bp, synthetic construct
  misc_feature 1..41: note = Target Specific Oligonucleotide
  source 1..41: mol_type = other DNA
ctgccagttagttaggcaagttgtaacgtcgctgaaaaatc

SEQ ID NO: 321 - DNA, 38 bp, synthetic construct
  misc_feature 1..38: note = Target Specific Oligonucleotide
  source 1..38: mol_type = other DNA
gcagctccgggctacaagtgtaacgtcgctgaaaaatc

SEQ ID NO: 322 - DNA, 40 bp, synthetic construct
  misc_feature 1..40: note = Target Specific Oligonucleotide
  source 1..40: mol_type = other DNA
tggcagctgtctaactggagcgtaacgtcgctgaaaaatc

SEQ ID NO: 323 - DNA, 38 bp, synthetic construct
  misc_feature 1..38: note = Target Specific Oligonucleotide
  source 1..38: mol_type = other DNA
acgcgtgtgcgagtagatggtaacgtcgctgaaaaatc

SEQ ID NO: 324 - DNA, 38 bp, synthetic construct
  misc_feature 1..38: note = Target Specific Oligonucleotide
  source 1..38: mol_type = other DNA
agctccacgaaggatgccagtaacgtcgctgaaaaatc

SEQ ID NO: 325 - DNA, 39 bp, synthetic construct
  misc_feature 1..39: note = Target Specific Oligonucleotide
  source 1..39: mol_type = other DNA
tgaggacggcatcgagatccgtaacgtcgctgaaaaatc

SEQ ID NO: 326 - DNA, 39 bp, synthetic construct
  misc_feature 1..39: note = Target Specific Oligonucleotide
  source 1..39: mol_type = other DNA
gtcttgagacccggtcttgggtaacgtcgctgaaaaatc

SEQ ID NO: 327 - DNA, 38 bp, synthetic construct
  misc_feature 1..38: note = Target Specific Oligonucleotide
  source 1..38: mol_type = other DNA
agtggtctggatcggtgcggtaacgtcgctgaaaaatc

SEQ ID NO: 328 - DNA, 39 bp, synthetic construct
  misc_feature 1..39: note = Target Specific Oligonucleotide
  source 1..39: mol_type = other DNA
tccattctgggtcgagtggagtaacgtcgctgaaaaatc

SEQ ID NO: 329 - DNA, 39 bp, synthetic construct
  misc_feature 1..39: note = Target Specific Oligonucleotide
  source 1..39: mol_type = other DNA
ggaccccaaggtgttccaaggtaacgtcgctgaaaaatc

SEQ ID NO: 330 - DNA, 38 bp, synthetic construct
  misc_feature 1..38: note = Target Specific Oligonucleotide
  source 1..38: mol_type = other DNA
agcagcttggctactccccgtaacgtcgctgaaaaatc

SEQ ID NO: 331 - DNA, 42 bp, synthetic construct
  misc_feature 1..42: note = Target Specific Oligonucleotide
  source 1..42: mol_type = other DNA
tttgggtatgggtactgtgtagagtaacgtcgctgaaaaatc

SEQ ID NO: 332 - DNA, 39 bp, synthetic construct
  misc_feature 1..39: note = Target Specific Oligonucleotide
  source 1..39: mol_type = other DNA
gccgcagggatagatccagggtaacgtcgctgaaaaatc

SEQ ID NO: 333 - DNA, 42 bp, synthetic construct
  misc_feature 1..42: note = Target Specific Oligonucleotide
  source 1..42: mol_type = other DNA
tgaagacagtcctatggacttccgtaacgtcgctgaaaaatc

SEQ ID NO: 334 - DNA, 37 bp, synthetic construct
  misc_feature 1..37: note = Target Specific Oligonucleotide
  source 1..37: mol_type = other DNA
aagctgaagcgcgggtcagtaacgtcgctgaaaaatc

SEQ ID NO: 335 - DNA, 37 bp, synthetic construct
  misc_feature 1..37: note = Target Specific Oligonucleotide
  source 1..37: mol_type = other DNA
ccacgcagcccttcgagagtaacgtcgctgaaaaatc

SEQ ID NO: 336 - DNA, 45 bp, synthetic construct
  misc_feature 1..45: note = Target Specific Oligonucleotide
  source 1..45: mol_type = other DNA
tagtaggtgtcgacaactagagcgtaactcttcaagattaatacc

SEQ ID NO: 337 - DNA, 44 bp, synthetic construct
  misc_feature 1..44: note = Target Specific Oligonucleotide
  source 1..44: mol_type = other DNA
gatggtcctgatcgagaaaccagtaactcttcaagattaatacc

SEQ ID NO: 338 - DNA, 44 bp, synthetic construct
  misc_feature 1..44: note = Target Specific Oligonucleotide
  source 1..44: mol_type = other DNA
aagaggacttcgctgaattgacgtaactcttcaagattaatacc

SEQ ID NO: 339 - DNA, 44 bp, synthetic construct
  misc_feature 1..44: note = Target Specific Oligonucleotide
  source 1..44: mol_type = other DNA
gaacctccgactgtatgtcagcgtaactcttcaagattaatacc

SEQ ID NO: 340 - DNA, 45 bp, synthetic construct
  misc_feature 1..45: note = Target Specific Oligonucleotide
  source 1..45: mol_type = other DNA
tctgaattagagcgatgttgacagtaactcttcaagattaatacc

SEQ ID NO: 341 - DNA, 41 bp, synthetic construct
  misc_feature 1..41: note = Target Specific Oligonucleotide
  source 1..41: mol_type = other DNA
gcattcctccgatcgcacagtaactcttcaagattaatacc

SEQ ID NO: 342 - DNA, 46 bp, synthetic construct
  misc_feature 1..46: note = Target Specific Oligonucleotide
  source 1..46: mol_type = other DNA
ctctatatttagctcgctgttcaagtaactcttcaagattaatacc

SEQ ID NO: 343 - DNA, 41 bp, synthetic construct
  misc_feature 1..41: note = Target Specific Oligonucleotide
  source 1..41: mol_type = other DNA
tattcatcacggcgcgcttgtaactcttcaagattaatacc

SEQ ID NO: 344 - DNA, 43 bp, synthetic construct
  misc_feature 1..43: note = Target Specific Oligonucleotide
  source 1..43: mol_type = other DNA
cattggggaccgtgcataaaagtaactcttcaagattaatacc

SEQ ID NO: 345 - DNA, 43 bp, synthetic construct
  misc_feature 1..43: note = Target Specific Oligonucleotide
  source 1..43: mol_type = other DNA
caaggggtgcactatttgggagtaactcttcaagattaatacc

SEQ ID NO: 346 - DNA, 43 bp, synthetic construct
  misc_feature 1..43: note = Target Specific Oligonucleotide
  source 1..43: mol_type = other DNA
ggaccgtatttcggcgaaatagtaactcttcaagattaatacc

SEQ ID NO: 347 - DNA, 43 bp, synthetic construct
  misc_feature 1..43: note = Target Specific Oligonucleotide
  source 1..43: mol_type = other DNA
atactgcacttgtcggcatgagtaactcttcaagattaatacc

SEQ ID NO: 348 - DNA, 43 bp, synthetic construct
  misc_feature 1..43: note = Target Specific Oligonucleotide
  source 1..43: mol_type = other DNA
atggcagatcgatccattggtgtaactcttcaagattaatacc

SEQ ID NO: 349 - DNA, 43 bp, synthetic construct
  misc_feature 1..43: note = Target Specific Oligonucleotide
  source 1..43: mol_type = other DNA
tccctttggaccgtcaagaaggtaactcttcaagattaatacc

SEQ ID NO: 350 - DNA, 42 bp, synthetic construct
  misc_feature 1..42: note = Target Specific Oligonucleotide
  source 1..42: mol_type = other DNA
aggcttgctgacatacgcaggtaactcttcaagattaatacc

SEQ ID NO: 351 - DNA, 42 bp, synthetic construct
  misc_feature 1..42: note = Target Specific Oligonucleotide
  source 1..42: mol_type = other DNA
cttgctttgtgcgaacacccgtaactcttcaagattaatacc

SEQ ID NO: 352 - DNA, 45 bp, synthetic construct
  misc_feature 1..45: note = Target Specific Oligonucleotide
  source 1..45: mol_type = other DNA
ctgatatcgaatgcaatggatgagtaactcttcaagattaatacc

SEQ ID NO: 353 - DNA, 43 bp, synthetic construct
  misc_feature 1..43: note = Target Specific Oligonucleotide
  source 1..43: mol_type = other DNA
taggactggtccgtcaaaaacgtaactcttcaagattaatacc

SEQ ID NO: 354 - DNA, 44 bp, synthetic construct
  misc_feature 1..44: note = Target Specific Oligonucleotide
  source 1..44: mol_type = other DNA
tgaccattctcgggacactaacgtaactcttcaagattaatacc

SEQ ID NO: 355 - DNA, 44 bp, synthetic construct
  misc_feature 1..44: note = Target Specific Oligonucleotide
  source 1..44: mol_type = other DNA
atgattgggtccgtaaaaatgcgtaactcttcaagattaatacc

SEQ ID NO: 356 - DNA, 45 bp, synthetic construct
  misc_feature 1..45: note = Target Specific Oligonucleotide
  source 1..45: mol_type = other DNA
gtttcatgtatggtaggaccaccgtaactcttcaagattaatacc

SEQ ID NO: 357 - DNA, 43 bp, synthetic construct
  misc_feature 1..43: note = Target Specific Oligonucleotide
  source 1..43: mol_type = other DNA
ctcttgcatcgtagcgaactagtaactcttcaagattaatacc

SEQ ID NO: 358 - DNA, 43 bp, synthetic construct
  misc_feature 1..43: note = Target Specific Oligonucleotide
  source 1..43: mol_type = other DNA
atgatgattccctcggtcagagtaactcttcaagattaatacc

SEQ ID NO: 359 - DNA, 46 bp, synthetic construct
  misc_feature 1..46: note = Target Specific Oligonucleotide
  source 1..46: mol_type = other DNA
agtagagaagatcgctgatatccggtaactcttcaagattaatacc

SEQ ID NO: 360 - DNA, 42 bp, synthetic construct
  misc_feature 1..42: note = Target Specific Oligonucleotide
  source 1..42: mol_type = other DNA
aacccttgacatcgccagtttgtaacgtaccgtttgtatatg

SEQ ID NO: 361 - DNA, 45 bp, synthetic construct
  misc_feature 1..45: note = Target Specific Oligonucleotide
  source 1..45: mol_type = other DNA
gaaggttaaacgagatttccaaaggtaacgtaccgtttgtatatg

SEQ ID NO: 362 - DNA, 41 bp, synthetic construct
  misc_feature 1..41: note = Target Specific Oligonucleotide
  source 1..41: mol_type = other DNA
gccactcgacatttctgccggtaacgtaccgtttgtatatg

SEQ ID NO: 363 - DNA, 42 bp, synthetic construct
  misc_feature 1..42: note = Target Specific Oligonucleotide
  source 1..42: mol_type = other DNA
tcatactgtccgcaacatccggtaacgtaccgtttgtatatg

SEQ ID NO: 364 - DNA, 41 bp, synthetic construct; identical to SEQ ID NO: 362
  misc_feature 1..41: note = Target Specific Oligonucleotide
  source 1..41: mol_type = other DNA

SEQ ID NO: 365 - DNA, 42 bp, synthetic construct; identical to SEQ ID NO: 363
  misc_feature 1..42: note = Target Specific Oligonucleotide
  source 1..42: mol_type = other DNA

SEQ ID NO: 366 - DNA, 43 bp, synthetic construct
  misc_feature 1..43: note = Target Specific Oligonucleotide
  source 1..43: mol_type = other DNA
tgaattttgcccgaacttcactgtaacgtaccgtttgtatatg

SEQ ID NO: 367 - DNA, 38 bp, synthetic construct
  misc_feature 1..38: note = Target Specific Oligonucleotide
  source 1..38: mol_type = other DNA
acacactcggagcgcgcgtaacgtaccgtttgtatatg

SEQ ID NO: 368 - DNA, 43 bp, synthetic construct
  misc_feature 1..43: note = Target Specific Oligonucleotide
  source 1..43: mol_type = other DNA
caaacctatatgcccgttgactgtaacgtaccgtttgtatatg

SEQ ID NO: 369 - DNA, 44 bp, synthetic construct
  misc_feature 1..44: note = Target Specific Oligonucleotide
  source 1..44: mol_type = other DNA
caggaacctttaccatgttcatggtaacgtaccgtttgtatatg

SEQ ID NO: 370 - DNA, 46 bp, synthetic construct
  misc_feature 1..46: note = Target Specific Oligonucleotide
  source 1..46: mol_type = other DNA
gaaaatctctacggatgaatttcttgtaacgtaccgtttgtatatg

SEQ ID NO: 371 - DNA, 43 bp, synthetic construct
  misc_feature 1..43: note = Target Specific Oligonucleotide
  source 1..43: mol_type = other DNA
gctgctaagatagccttgtgaggtaacgtaccgtttgtatatg

SEQ ID NO: 372 - DNA, 42 bp, synthetic construct
  misc_feature 1..42: note = Target Specific Oligonucleotide
  source 1..42: mol_type = other DNA
tggcactaaaaaccggagaacgtaacgtaccgtttgtatatg

SEQ ID NO: 373 - DNA, 39 bp, synthetic construct
  misc_feature 1..39: note = Target Specific Oligonucleotide
  source 1..39: mol_type = other DNA
tgcgggaccgccgatacagtaacgtaccgtttgtatatg

SEQ ID NO: 374 - DNA, 45 bp, synthetic construct
  misc_feature 1..45: note = Target Specific Oligonucleotide
  source 1..45: mol_type = other DNA
ggaaattaaacggagtcttacaacgtaacgtaccgtttgtatatg

SEQ ID NO: 375 - DNA, 40 bp, synthetic construct
  misc_feature 1..40: note = Target Specific Oligonucleotide
  source 1..40: mol_type = other DNA
agccagagagcggtatgccgtaacgtaccgtttgtatatg

SEQ ID NO: 376 - DNA, 41 bp, synthetic construct
  misc_feature 1..41: note = Target Specific Oligonucleotide
  source 1..41: mol_type = other DNA
ccaccaagtggggatgtgacgtaacgtaccgtttgtatatg

SEQ ID NO: 377 - DNA, 42 bp, synthetic construct
  misc_feature 1..42: note = Target Specific Oligonucleotide
  source 1..42: mol_type = other DNA
cacacatgacctttaagcgctgtaacgtaccgtttgtatatg

SEQ ID NO: 378 - DNA, 41 bp, synthetic construct
  misc_feature 1..41: note = Target Specific Oligonucleotide
  source 1..41: mol_type = other DNA
tccacagattgcgctgtctagtaacgtaccgtttgtatatg

SEQ ID NO: 379 - DNA, 41 bp, synthetic construct
  misc_feature 1..41: note = Target Specific Oligonucleotide
  source 1..41: mol_type = other DNA
ctccacggacaggttactgcgtaacgtaccgtttgtatatg

SEQ ID NO: 380 - DNA, 39 bp, synthetic construct
  misc_feature 1..39: note = Target Specific Oligonucleotide
  source 1..39: mol_type = other DNA
gcgtcatggcgtcagcacgtaacgtaccgtttgtatatg

SEQ ID NO: 381 - DNA, 39 bp, synthetic construct
  misc_feature 1..39: note = Target Specific Oligonucleotide
  source 1..39: mol_type = other DNA
tcctggccggcaacacacgtaacgtaccgtttgtatatg

SEQ ID NO: 382 - DNA, 42 bp, synthetic construct
  misc_feature 1..42: note = Target Specific Oligonucleotide
  source 1..42: mol_type = other DNA
agccattttgtcgaggtttgggtaacgtaccgtttgtatatg

SEQ ID NO: 383 - DNA, 44 bp, synthetic construct
  misc_feature 1..44: note = Target Specific Oligonucleotide
  source 1..44: mol_type = other DNA
catccgaagcatgatagttgatggtaacgtaccgtttgtatatg

SEQ ID NO: 384 - DNA, 43 bp, synthetic construct
  misc_feature 1..43: note = Target Specific Oligonucleotide
  source 1..43: mol_type = other DNA
tagtgtgttgcgtatcaagtatctagacgatgcgaattaacac

SEQ ID NO: 385 - DNA, 45 bp, synthetic construct
  misc_feature 1..45: note = Target Specific Oligonucleotide
  source 1..45: mol_type = other DNA
ttattgtgaactctagacatgagagtagacgatgcgaattaacac

SEQ ID NO: 386 - DNA, 46 bp, synthetic construct
  misc_feature 1..46: note = Target Specific Oligonucleotide
  source 1..46: mol_type = other DNA
acagtgaatactaagactgtaaaaactagacgatgcgaattaacac

SEQ ID NO: 387 - DNA, 41 bp, synthetic construct
  misc_feature 1..41: note = Target Specific Oligonucleotide
  source 1..41: mol_type = other DNA
acacaaggcacgtagaaacagtagacgatgcgaattaacac

SEQ ID NO: 388 - DNA, 41 bp, synthetic construct
  misc_feature 1..41: note = Target Specific Oligonucleotide
  source 1..41: mol_type = other DNA
caatggacagcggttgtgaaatagacgatgcgaattaacac

SEQ ID NO: 389 - DNA, 42 bp, synthetic construct
  misc_feature 1..42: note = Target Specific Oligonucleotide
  source 1..42: mol_type = other DNA
caccatcacctatcgacagagttagacgatgcgaattaacac

SEQ ID NO: 390 - DNA, 42 bp, synthetic construct
  misc_feature 1..42: note = Target Specific Oligonucleotide
  source 1..42: mol_type = other DNA
cattgcattacgttccacatggtagacgatgcgaattaacac

SEQ ID NO: 391 - DNA, 41 bp, synthetic construct
  misc_feature 1..41: note = Target Specific Oligonucleotide
  source 1..41: mol_type = other DNA
acacagagtgtccgatacccatagacgatgcgaattaacac

SEQ ID NO: 392 - DNA, 43 bp, synthetic construct
  misc_feature 1..43: note = Target Specific Oligonucleotide
  source 1..43: mol_type = other DNA
ggtgattacattgagtgctaggatagacgatgcgaattaacac

SEQ ID NO: 393 - DNA, 41 bp, synthetic construct
  misc_feature 1..41: note = Target Specific Oligonucleotide
  source 1..41: mol_type = other DNA
tccacataagcgttcaaggtatagacgatgcgaattaacac

SEQ ID NO: 394 - DNA, 44 bp, synthetic construct
  misc_feature 1..44: note = Target Specific Oligonucleotide
  source 1..44: mol_type = other DNA
cagaataatcgctattcctagctgtagacgatgcgaattaacac

SEQ ID NO: 395 - DNA, 40 bp, synthetic construct
  misc_feature 1..40: note = Target Specific Oligonucleotide
  source 1..40: mol_type = other DNA
ttacactcatacgtcgccggtagacgatgcgaattaacac

SEQ ID NO: 396 - DNA, 43 bp, synthetic construct
  misc_feature 1..43: note = Target Specific Oligonucleotide
  source 1..43: mol_type = other DNA
tggccataaaggctacttacaattagacgatgcgaattaacac

SEQ ID NO: 397 - DNA, 45 bp, synthetic construct
  misc_feature 1..45: note = Target Specific Oligonucleotide
  source 1..45: mol_type = other DNA
tttcaagttattcgatctgctaacctagacgatgcgaattaacac

SEQ ID NO: 398 - DNA, 45 bp, synthetic construct
  misc_feature 1..45: note = Target Specific Oligonucleotide
  source 1..45: mol_type = other DNA
agttagtcaaggactttactaaggttagacgatgcgaattaacac

SEQ ID NO: 399 - DNA, 42 bp, synthetic construct
  misc_feature 1..42: note = Target Specific Oligonucleotide
  source 1..42: mol_type = other DNA
ttacctcaaatacgggctaccatagacgatgcgaattaacac

SEQ ID NO: 400 - DNA, 47 bp, synthetic construct
  misc_feature 1..47: note = Target Specific Oligonucleotide
  source 1..47: mol_type = other DNA
gagttatattactctaactaaagccagtagacgatgcgaattaacac

SEQ ID NO: 401 - DNA, 43 bp, synthetic construct
  misc_feature 1..43: note = Target Specific Oligonucleotide
  source 1..43: mol_type = other DNA
ttgtcaacacgcataaaatctgctagacgatgcgaattaacac

SEQ ID NO: 402 - DNA, 43 bp, synthetic construct
  misc_feature 1..43: note = Target Specific Oligonucleotide
  source 1..43: mol_type = other DNA
tcatatacaatcggggatctgagtagacgatgcgaattaacac

SEQ ID NO: 403 - DNA, 43 bp, synthetic construct
  misc_feature 1..43: note = Target Specific Oligonucleotide
  source 1..43: mol_type = other DNA
cccacaaaaatacccgtaagttatagacgatgcgaattaacac

SEQ ID NO: 404 - DNA, 47 bp, synthetic construct
  misc_feature 1..47: note = Target Specific Oligonucleotide
  source 1..47: mol_type = other DNA
cactaaattattacgaattttgcaaagtagacgatgcgaattaacac

SEQ ID NO: 405 - DNA, 45 bp, synthetic construct
  misc_feature 1..45: note = Target Specific Oligonucleotide
  source 1..45: mol_type = other DNA
tcaaataaaaaccgtcaaaagtttatagacgatgcgaattaacac

SEQ ID NO: 406 - DNA, 42 bp, synthetic construct
  misc_feature 1..42: note = Target Specific Oligonucleotide
  source 1..42: mol_type = other DNA
agtgcaatggtatcacgtactgtagacgatgcgaattaacac

SEQ ID NO: 407 - DNA, 43 bp, synthetic construct
  misc_feature 1..43: note = Target Specific Oligonucleotide
  source 1..43: mol_type = other DNA
atgtgtcttgcaattggattccctagacgatgcgaattaacac

SEQ ID NO: 408 - DNA, 38 bp, synthetic construct
  misc_feature 1..38: note = Target Specific Oligonucleotide
  source 1..38: mol_type = other DNA
ggtgtgcgcgtcgtacactagacccgttataagtgttg

SEQ ID NO: 409 - DNA, 40 bp, synthetic construct
  misc_feature 1..40: note = Target Specific Oligonucleotide
  source 1..40: mol_type = other DNA
gtgtttagggtcgcggttgatagacccgttataagtgttg

SEQ ID NO: 410 - DNA, 42 bp, synthetic construct
  misc_feature 1..42: note = Target Specific Oligonucleotide
  source 1..42: mol_type = other DNA
gagaatggcgaagtaaatgccctagacccgttataagtgttg

SEQ ID NO: 411 - DNA, 42 bp, synthetic construct
  misc_feature 1..42: note = Target Specific Oligonucleotide
  source 1..42: mol_type = other DNA
gtagatggaatagacacggctgtagacccgttataagtgttg

SEQ ID NO: 412 - DNA, 43 bp, synthetic construct
  misc_feature 1..43: note = Target Specific Oligonucleotide
  source 1..43: mol_type = other DNA
gctcttaatgcatggtacaactgtagacccgttataagtgttg

SEQ ID NO: 413 - DNA, 43 bp, synthetic construct
  misc_feature 1..43: note = Target Specific Oligonucleotide
  source 1..43: mol_type = other DNA
aaaccagtatttcgtcacagtgatagacccgttataagtgttg

SEQ ID NO: 414 - DNA, 42 bp, synthetic construct
  misc_feature 1..42: note = Target Specific Oligonucleotide
  source 1..42: mol_type = other DNA
gatgggaacggtgtagagatgttagacccgttataagtgttg

SEQ ID NO: 415 - DNA, 42 bp, synthetic construct
  misc_feature 1..42: note = Target Specific Oligonucleotide
  source 1..42: mol_type = other DNA
ttccaaatgccgtcaaaactgttagacccgttataagtgttg

SEQ ID NO: 416 - DNA, 39 bp, synthetic construct
  misc_feature 1..39: note = Target Specific Oligonucleotide
  source 1..39: mol_type = other DNA
tgggtcacagacggtgtggtagacccgttataagtgttg

SEQ ID NO: 417 - DNA, 46 bp, synthetic construct
  misc_feature 1..46: note = Target Specific Oligonucleotide
  source 1..46: mol_type = other DNA
aatcaggtatacttctatccttgaaatagacccgttataagtgttg

SEQ ID NO: 418 - DNA, 43 bp, synthetic construct
  misc_feature 1..43: note = Target Specific Oligonucleotide
  source 1..43: mol_type = other DNA
tgctgtattagcaacttggaacttagacccgttataagtgttg

SEQ ID NO: 419 - DNA, 42 bp, synthetic construct
  misc_feature 1..42: note = Target Specific Oligonucleotide
  source 1..42: mol_type = other DNA
gccaataaagcgatggttgatctagacccgttataagtgttg

SEQ ID NO: 420 - DNA, 43 bp, synthetic construct
  misc_feature 1..43: note = Target Specific Oligonucleotide
  source 1..43: mol_type = other DNA
gtaaggatcactggatcctactgtagacccgttataagtgttg

SEQ ID NO: 421 - DNA, 43 bp, synthetic construct
  misc_feature 1..43: note = Target Specific Oligonucleotide
  source 1..43: mol_type = other DNA
gacctcattcagttgatgagaggtagacccgttataagtgttg

SEQ ID NO: 422 - DNA, 41 bp, synthetic construct
  misc_feature 1..41: note = Target Specific Oligonucleotide
  source 1..41: mol_type = other DNA
gcataacagacggttgcaagttagacccgttataagtgttg

SEQ ID NO: 423 - DNA, 41 bp, synthetic construct
  misc_feature 1..41: note = Target Specific Oligonucleotide
  source 1..41: mol_type = other DNA
acctaaagcgagttgctgagttagacccgttataagtgttg

SEQ ID NO: 424 - DNA, 41 bp, synthetic construct
  misc_feature 1..41: note = Target Specific Oligonucleotide
  source 1..41: mol_type = other DNA
gagtcagaaacacgcatggaatagacccgttataagtgttg

SEQ ID NO: 425 - DNA, 42 bp, synthetic construct
  misc_feature 1..42: note = Target Specific Oligonucleotide
  source 1..42: mol_type = other DNA
agcaactctgataggctcacactagacccgttataagtgttg

SEQ ID NO: 426 - DNA, 44 bp, synthetic construct
  misc_feature 1..44: note = Target Specific Oligonucleotide
  source 1..44: mol_type = other DNA
ccatacccactacggataaagatgtagacccgttataagtgttg

SEQ ID NO: 427 - DNA, 42 bp, synthetic construct
  misc_feature 1..42: note = Target Specific Oligonucleotide
  source 1..42: mol_type = other DNA
gctttctgtacgactcaggttttagacccgttataagtgttg

SEQ ID NO: 428 - DNA, 42 bp, synthetic construct
  misc_feature 1..42: note = Target Specific Oligonucleotide
  source 1..42: mol_type = other DNA
caatgttgagccactaaaccactagacccgttataagtgttg

SEQ ID NO: 429 - DNA, 42 bp, synthetic construct
  misc_feature 1..42: note = Target Specific Oligonucleotide
  source 1..42: mol_type = other DNA
atgcttggattaggtccaaagctagacccgttataagtgttg

SEQ ID NO: 430 - DNA, 41 bp, synthetic construct
  misc_feature 1..41: note = Target Specific Oligonucleotide
  source 1..41: mol_type = other DNA
cccggtgatggattagtttggtagacccgttataagtgttg

SEQ ID NO: 431 - DNA, 41 bp, synthetic construct
  misc_feature 1..41: note = Target Specific Oligonucleotide
  source 1..41: mol_type = other DNA
ccatggccataccctggaatttagacccgttataagtgttg

SEQ ID NO: 432 - DNA, 41 bp, synthetic construct
  misc_feature 1..41: note = Target Specific Oligonucleotide
  source 1..41: mol_type = other DNA
attatactgtccagcgtaggtggtagacaaccgtcgttaag

SEQ ID NO: 433 - DNA, 41 bp, synthetic construct
  misc_feature 1..41: note = Target Specific Oligonucleotide
  source 1..41: mol_type = other DNA
tcctggtaaggataggtaccatgtagacaaccgtcgttaag

SEQ ID NO: 434 - DNA, 41 bp, synthetic construct
  misc_feature 1..41: note = Target Specific Oligonucleotide
  source 1..41: mol_type = other DNA
cactgaaataggacggaatctgctagacaaccgtcgttaag

SEQ ID NO: 435 - DNA, 39 bp, synthetic construct
  misc_feature 1..39: note = Target Specific Oligonucleotide
  source 1..39: mol_type = other DNA
aaagtttattggcgcttgccgtagacaaccgtcgttaag

SEQ ID NO: 436 - DNA, 39 bp, synthetic construct
  misc_feature 1..39: note = Target Specific Oligonucleotide
  source 1..39: mol_type = other DNA
gcaatgccattagcgatacgatagacaaccgtcgttaag

SEQ ID NO: 437 - DNA, 38 bp, synthetic construct
  misc_feature 1..38: note = Target Specific Oligonucleotide
  source 1..38: mol_type = other DNA
tgattgaacaccacgcgacatagacaaccgtcgttaag

SEQ ID NO: 438 - DNA, 40 bp, synthetic construct
  misc_feature 1..40: note = Target Specific Oligonucleotide
  source 1..40: mol_type = other DNA
agtcttcgaagcactattgccatagacaaccgtcgttaag

SEQ ID NO: 439 - DNA, 39 bp, synthetic construct
  misc_feature 1..39: note = Target Specific Oligonucleotide
  source 1..39: mol_type = other DNA
tcaatggttgatcggcctctctagacaaccgtcgttaag

SEQ ID NO: 440 - DNA, 41 bp, synthetic construct
  misc_feature 1..41: note = Target Specific Oligonucleotide
  source 1..41: mol_type = other DNA
tggcatgatgtctaataggagtctagacaaccgtcgttaag

SEQ ID NO: 441 - DNA, 38 bp, synthetic construct
  misc_feature 1..38: note = Target Specific Oligonucleotide
  source 1..38: mol_type = other DNA
ctgcggtttagccttgacgttagacaaccgtcgttaag

SEQ ID NO: 442 - DNA, 38 bp, synthetic construct
  misc_feature 1..38: note = Target Specific Oligonucleotide
  source 1..38: mol_type = other DNA
cccagaggacgccatcattttagacaaccgtcgttaag

SEQ ID NO: 443 - DNA, 40 bp, synthetic construct
  misc_feature 1..40: note = Target Specific Oligonucleotide
  source 1..40: mol_type = other DNA
tttcttgaaagacgacagcagttagacaaccgtcgttaag

SEQ ID NO: 444 - DNA, 41 bp, synthetic construct
  misc_feature 1..41: note = Target Specific Oligonucleotide
  source 1..41: mol_type = other DNA
attaaatgttcggaaggatgacctagacaaccgtcgttaag

SEQ ID NO: 445 - DNA, 38 bp, synthetic construct
  misc_feature 1..38: note = Target Specific Oligonucleotide
  source 1..38: mol_type = other DNA
tcttttgtcagcacggttgctagacaaccgtcgttaag

SEQ ID NO: 446 - DNA, 38 bp, synthetic construct
  misc_feature 1..38: note = Target Specific Oligonucleotide
  source 1..38: mol_type = other DNA
ctggatcagctcgaccaggatagacaaccgtcgttaag

SEQ ID NO: 447 - DNA, 38 bp, synthetic construct
  misc_feature 1..38: note = Target Specific Oligonucleotide
  source 1..38: mol_type = other DNA
accatggtccgacttctgcctagacaaccgtcgttaag

SEQ ID NO: 448 - DNA, 40 bp, synthetic construct
  misc_feature 1..40: note = Target Specific Oligonucleotide
  source 1..40: mol_type = other DNA
ctggatattcggttatctgggctagacaaccgtcgttaag

SEQ ID NO: 449 - DNA, 41 bp, synthetic construct
  misc_feature 1..41: note = Target Specific Oligonucleotide
  source 1..41: mol_type = other DNA
atcccctttacgatactcttcagtagacaaccgtcgttaag

SEQ ID NO: 450 - DNA, 38 bp, synthetic construct
  misc_feature 1..38: note = Target Specific Oligonucleotide
  source 1..38: mol_type = other DNA
tccagagcgggaacagtatgtagacaaccgtcgttaag

SEQ ID NO: 451 - DNA, 38 bp, synthetic construct
  misc_feature 1..38: note = Target Specific Oligonucleotide
  source 1..38: mol_type = other DNA
gttgcctgcataagatgggctagacaaccgtcgttaag

SEQ ID NO: 452 - DNA, 38 bp, synthetic construct
  misc_feature 1..38: note = Target Specific Oligonucleotide
  source 1..38: mol_type = other DNA
ccttttgtgccgatgacccgtagacaaccgtcgttaag

SEQ ID NO: 453 - DNA, 37 bp, synthetic construct
  misc_feature 1..37: note = Target Specific Oligonucleotide
  source 1..37: mol_type = other DNA
gcttccgtggactgggacgtagacaaccgtcgttaag

SEQ ID NO: 454 - DNA, 41 bp, synthetic construct
  misc_feature 1..41: note = Target Specific Oligonucleotide
  source 1..41: mol_type = other DNA
ccatagaaggacgaggtatttcctagacaaccgtcgttaag

SEQ ID NO: 455 - DNA, 39 bp, synthetic construct
  misc_feature 1..39: note = Target Specific Oligonucleotide
  source 1..39: mol_type = other DNA
agaatgagtcgctgctcgatatagacaaccgtcgttaag

SEQ ID NO: 456 - DNA, 41 bp, synthetic construct
  misc_feature 1..41: note = Target Specific Oligonucleotide
  source 1..41: mol_type = other DNA
gcttcgacaaacgcaaagcgtagactcaatgatgataaaga

SEQ ID NO: 457 - DNA, 44 bp, synthetic construct
  misc_feature 1..44: note = Target Specific Oligonucleotide
  source 1..44: mol_type = other DNA
gctagttcacagaaagaccattttagactcaatgatgataaaga

SEQ ID NO: 458 - DNA, 41 bp, synthetic construct
  misc_feature 1..41: note = Target Specific Oligonucleotide
  source 1..41: mol_type = other DNA
cagctcatcgaaagcgaccctagactcaatgatgataaaga

SEQ ID NO: 459 - DNA, 40 bp, synthetic construct
  misc_feature 1..40: note = Target Specific Oligonucleotide
  source 1..40: mol_type = other DNA
cggctgctacaaacctcggtagactcaatgatgataaaga

SEQ ID NO: 460 - DNA, 42 bp, synthetic construct
  misc_feature 1..42: note = Target Specific Oligonucleotide
  source 1..42: mol_type = other DNA
aacaatttgaaggccccacaatagactcaatgatgataaaga

SEQ ID NO: 461 - DNA, 39 bp, synthetic construct
  misc_feature 1..39: note = Target Specific Oligonucleotide
  source 1..39: mol_type = other DNA
gcgtctgcaccggagacttagactcaatgatgataaaga

SEQ ID NO: 462 - DNA, 39 bp, synthetic construct
  misc_feature 1..39: note = Target Specific Oligonucleotide
  source 1..39: mol_type = other DNA
gcgctgctcaggcattggtagactcaatgatgataaaga

SEQ ID NO: 463 - DNA, 47 bp, synthetic construct
  misc_feature 1..47: note = Target Specific Oligonucleotide
  source 1..47: mol_type = other DNA
ttgttgtgtaacaacataatttcaagtagactcaatgatgataaaga

SEQ ID NO: 464 - DNA, 38 bp, synthetic construct
  misc_feature 1..38: note = Target Specific Oligonucleotide
  source 1..38: mol_type = other DNA
ctccacgtcggcgtgcatagactcaatgatgataaaga

SEQ ID NO: 465 - DNA, 40 bp, synthetic construct
  misc_feature 1..40: note = Target Specific Oligonucleotide
  source 1..40: mol_type = other DNA
ctgcggggattgtagccggtagactcaatgatgataaaga

SEQ ID NO: 466 - DNA, 42 bp, synthetic construct
  misc_feature 1..42: note = Target Specific Oligonucleotide
  source 1..42: mol_type = other DNA
atcttagctactgaccggctatagactcaatgatgataaaga

SEQ ID NO: 467 - DNA, 43 bp, synthetic construct
  misc_feature 1..43: note = Target Specific Oligonucleotide
  source 1..43: mol_type = other DNA
aagagattatacgcctcacggatagactcaatgatgataaaga

SEQ ID NO: 468 - DNA, 44 bp, synthetic construct
  misc_feature 1..44: note = Target Specific Oligonucleotide
  source 1..44: mol_type = other DNA
tttcgagtaacgaaattagctcctagactcaatgatgataaaga

SEQ ID NO: 469 - DNA, 39 bp, synthetic construct
  misc_feature 1..39: note = Target Specific Oligonucleotide
  source 1..39: mol_type = other DNA
gacccgcagattggcacgtagactcaatgatgataaaga

SEQ ID NO: 470 - DNA, 41 bp, synthetic construct
  misc_feature 1..41: note = Target Specific Oligonucleotide
  source 1..41: mol_type = other DNA
atggccccaatctcgtttggtagactcaatgatgataaaga

SEQ ID NO: 471 - DNA, 44 bp, synthetic construct
  misc_feature 1..44: note = Target Specific Oligonucleotide
  source 1..44: mol_type = other DNA
ccagtagctataacgaagtcctctagactcaatgatgataaaga

SEQ ID NO: 472 - DNA, 43 bp, synthetic construct
  misc_feature 1..43: note = Target Specific Oligonucleotide
  source 1..43: mol_type = other DNA
acaaattcccggacactatggatagactcaatgatgataaaga

SEQ ID NO: 473 - DNA, 43 bp, synthetic construct
  misc_feature 1..43: note = Target Specific Oligonucleotide
  source 1..43: mol_type = other DNA
ttcacagagttgataaggccactagactcaatgatgataaaga

SEQ ID NO: 474 - DNA, 43 bp, synthetic construct
  misc_feature 1..43: note = Target Specific Oligonucleotide
  source 1..43: mol_type = other DNA
aactttgccggtctctttacattagactcaatgatgataaaga

SEQ ID NO: 475 - DNA, 45 bp, synthetic construct
  misc_feature 1..45: note = Target Specific Oligonucleotide
  source 1..45: mol_type = other DNA
ttccaatgtgcaagaatgatttcttagactcaatgatgataaaga

SEQ ID NO: 476 - DNA, 43 bp, synthetic construct
  misc_feature 1..43: note = Target Specific Oligonucleotide
  source 1..43: mol_type = other DNA
ctccttctggggtatttcctgctagactcaatgatgataaaga

SEQ ID NO: 477 - DNA, 40 bp, synthetic construct
  misc_feature 1..40: note = Target Specific Oligonucleotide
  source 1..40: mol_type = other DNA
ccacttcagttggccggtatagactcaatgatgataaaga

SEQ ID NO: 478 - DNA, 39 bp, synthetic construct
  misc_feature 1..39: note = Target Specific Oligonucleotide
  source 1..39: mol_type = other DNA
tccgtcaacgtccgcagttagactcaatgatgataaaga

SEQ ID NO: 479 - DNA, 42 bp, synthetic construct
  misc_feature 1..42: note = Target Specific Oligonucleotide
  source 1..42: mol_type = other DNA
agtgagatcgccatagtgcaatagactcaatgatgataaaga

SEQ ID NO: 480 - DNA, 43 bp, synthetic construct
  misc_feature 1..43: note = Target Specific Oligonucleotide
  source 1..43: mol_type = other DNA
gaaggtgaccctataaggagtcatagactacaacaaaagatcg

SEQ ID NO: 481 - DNA, 41 bp, synthetic construct
  misc_feature 1..41: note = Target Specific Oligonucleotide
  source 1..41: mol_type = other DNA
aacaccgcttgcatagttgtgtagactacaacaaaagatcg

SEQ ID NO: 482 - DNA, 41 bp, synthetic construct
  misc_feature 1..41: note = Target Specific Oligonucleotide
  source 1..41: mol_type = other DNA
tacagacgcggaatcattctctagactacaacaaaagatcg

SEQ ID NO: 483 - DNA, 41 bp, synthetic construct
  misc_feature 1..41: note = Target Specific Oligonucleotide
  source 1..41: mol_type = other DNA
tggaggaaatgagcatgaccttagactacaacaaaagatcg

SEQ ID NO: 484 - DNA, 41 bp, synthetic construct
  misc_feature 1..41: note = Target Specific Oligonucleotide
  source 1..41: mol_type = other DNA
atggtgtacactcgaggctgatagactacaacaaaagatcg

SEQ ID NO: 485 - DNA, 41 bp, synthetic construct
  misc_feature 1..41: note = Target Specific Oligonucleotide
  source 1..41: mol_type = other DNA
ccttgtggtagacgttcagcttagactacaacaaaagatcg

SEQ ID NO: 486 - DNA, 44 bp, synthetic construct
  misc_feature 1..44: note = Target Specific Oligonucleotide
  source 1..44: mol_type = other DNA
ggatcaggtttaatggtcactatgtagactacaacaaaagatcg

SEQ ID NO: 487 - DNA, 40 bp, synthetic construct
  misc_feature 1..40: note = Target Specific Oligonucleotide
  source 1..40: mol_type = other DNA
cacacggtcaacgctgtacatagactacaacaaaagatcg

SEQ ID NO: 488 - DNA, 40 bp, synthetic construct
  misc_feature 1..40: note = Target Specific Oligonucleotide
  source 1..40: mol_type = other DNA
caggtgtttgcggaagttcctagactacaacaaaagatcg

SEQ ID NO: 489 - DNA, 40 bp, synthetic construct
  misc_feature 1..40: note = Target Specific Oligonucleotide
  source 1..40: mol_type = other DNA
gtgctcatggtcgtagaggatagactacaacaaaagatcg

SEQ ID NO: 490 - DNA, 43 bp, synthetic construct
  misc_feature 1..43: note = Target Specific Oligonucleotide
  source 1..43: mol_type = other DNA
aagtcaaagtacgtctcgatcattagactacaacaaaagatcg

SEQ ID NO: 491 - DNA, 39 bp, synthetic construct
  misc_feature 1..39: note = Target Specific Oligonucleotide
  source 1..39: mol_type = other DNA
tcgtagcagccgttggagatagactacaacaaaagatcg

SEQ ID NO: 492 - DNA, 39 bp, synthetic construct
  misc_feature 1..39: note = Target Specific Oligonucleotide
  source 1..39: mol_type = other DNA
tcgtggccagagtaggcattagactacaacaaaagatcg

SEQ ID NO: 493 - DNA, 40 bp, synthetic construct
  misc_feature 1..40: note = Target Specific Oligonucleotide
  source 1..40: mol_type = other DNA
ggtactctccaaacgctcggtagactacaacaaaagatcg

SEQ ID NO: 494 - DNA, 42 bp, synthetic construct
  misc_feature 1..42: note = Target Specific Oligonucleotide
  source 1..42: mol_type = other DNA
aggtacgaatagggatgtcgtctagactacaacaaaagatcg

SEQ ID NO: 495 - DNA, 42 bp, synthetic construct
  misc_feature 1..42: note = Target Specific Oligonucleotide
  source 1..42: mol_type = other DNA
agggtatcgtacatcgttccaatagactacaacaaaagatcg

SEQ ID NO: 496 - DNA, 39 bp, synthetic construct
  misc_feature 1..39: note = Target Specific Oligonucleotide
  source 1..39: mol_type = other DNA
caggtgatctgcgccgttgtagactacaacaaaagatcg

SEQ ID NO: 497 - DNA, 39 bp, synthetic construct
  misc_feature 1..39: note = Target Specific Oligonucleotide
  source 1..39: mol_type = other DNA
ccacaggcgatacaaccggtagactacaacaaaagatcg

SEQ ID NO: 498 - DNA, 39 bp, synthetic construct
  misc_feature 1..39: note = Target Specific Oligonucleotide
  source 1..39: mol_type = other DNA
cagcagcttcgagtgctggtagactacaacaaaagatcg

SEQ ID NO: 499 - DNA, 39 bp, synthetic construct
  misc_feature 1..39: note = Target Specific Oligonucleotide
  source 1..39: mol_type = other DNA
ccctcacaggacgtcgtcatagactacaacaaaagatcg

SEQ ID NO: 500 - DNA, 39 bp, synthetic construct
  misc_feature 1..39: note = Target Specific Oligonucleotide
  source 1..39: mol_type = other DNA
gcacgaagccttcggtgtctagactacaacaaaagatcg

SEQ ID NO: 501 - DNA, 41 bp, synthetic construct
  misc_feature 1..41: note = Target Specific Oligonucleotide
  source 1..41: mol_type = other DNA
tgggaagtgtcggctttcatgtagactacaacaaaagatcg

SEQ ID NO: 502 - DNA, 41 bp, synthetic construct; identical to SEQ ID NO: 501
  misc_feature 1..41: note = Target Specific Oligonucleotide
  source 1..41: mol_type = other DNA

SEQ ID NO: 503 - DNA, 38 bp, synthetic construct
  misc_feature 1..38: note = Target Specific Oligonucleotide
  source 1..38: mol_type = other DNA
tgctcgcactttggccgctagactacaacaaaagatcg

SEQ ID NO: 504 - DNA, 40 bp, synthetic construct
  misc_feature 1..40: note = Target Specific Oligonucleotide
  source 1..40: mol_type = other DNA
gtcttttggcacggtttctgttagactgtattcaacgtcc

SEQ ID NO: 505 - DNA, 40 bp, synthetic construct
  misc_feature 1..40: note = Target Specific Oligonucleotide
  source 1..40: mol_type = other DNA
tacttcttcaacgcgaagagctagactgtattcaacgtcc

SEQ ID NO: 506 - DNA, 40 bp, synthetic construct
  misc_feature 1..40: note = Target Specific Oligonucleotide
  source 1..40: mol_type = other DNA
tttgaggttgtatccgctgcttagactgtattcaacgtcc

SEQ ID NO: 507 - DNA, 44 bp, synthetic construct
  misc_feature 1..44: note = Target Specific Oligonucleotide
  source 1..44: mol_type = other DNA
caagttgactaaatctcgtactttctagactgtattcaacgtcc

SEQ ID NO: 508 - DNA, 43 bp, synthetic construct
  misc_feature 1..43: note = Target Specific Oligonucleotide
  source 1..43: mol_type = other DNA
gccttattaacggtatcttcagaatagactgtattcaacgtcc

SEQ ID NO: 509 - DNA, 40 bp, synthetic construct
  misc_feature 1..40: note = Target Specific Oligonucleotide
  source 1..40: mol_type = other DNA
tgttctggatttcgcaggtcctagactgtattcaacgtcc

SEQ ID NO: 510 - DNA, 42 bp, synthetic construct
  misc_feature 1..42: note = Target Specific Oligonucleotide
  source 1..42: mol_type = other DNA
gctttatcaggttatgttgcatgtagactgtattcaacgtcc

SEQ ID NO: 511 - DNA, 43 bp, synthetic construct
  misc_feature 1..43: note = Target Specific Oligonucleotide
  source 1..43: mol_type = other DNA
gattctggcttatagggtattcactagactgtattcaacgtcc

SEQ ID NO: 512 - DNA, 41 bp, synthetic construct
  misc_feature 1..41: note = Target Specific Oligonucleotide
  source 1..41: mol_type = other DNA
ttttcctcccgcaattcctagatagactgtattcaacgtcc

SEQ ID NO: 513 - DNA, 40 bp, synthetic construct
  misc_feature 1..40: note = Target Specific Oligonucleotide
  source 1..40: mol_type = other DNA
tgtttccgtcaaatcgtgtggtagactgtattcaacgtcc

SEQ ID NO: 514 - DNA, 41 bp, synthetic construct
  misc_feature 1..41: note = Target Specific Oligonucleotide
  source 1..41: mol_type = other DNA
ggttccctctagatcttgcctttagactgtattcaacgtcc

SEQ ID NO: 515 - DNA, 43 bp, synthetic construct
  misc_feature 1..43: note = Target Specific Oligonucleotide
  source 1..43: mol_type = other DNA
gcatgtaccacctatcatctaatgtagactgtattcaacgtcc

SEQ ID NO: 516 - DNA, 39 bp, synthetic construct
  misc_feature 1..39: note = Target Specific Oligonucleotide
  source 1..39: mol_type = other DNA
gttgccaacacgagctgacttagactgtattcaacgtcc

SEQ ID NO: 517 - DNA, 41 bp, synthetic construct
  misc_feature 1..41: note = Target Specific Oligonucleotide
  source 1..41: mol_type = other DNA
actgactactagttcaagcgcatagactgtattcaacgtcc

SEQ ID NO: 518 - DNA, 39 bp, synthetic construct
  misc_feature 1..39: note = Target Specific Oligonucleotide
  source 1..39: mol_type = other DNA
tctcttgctcgctttggacctagactgtattcaacgtcc

SEQ ID NO: 519 - DNA, 44 bp, synthetic construct
  misc_feature 1..44: note = Target Specific Oligonucleotide
  source 1..44: mol_type = other DNA
cactgctagaacaactatcaatttgtagactgtattcaacgtcc

SEQ ID NO: 520 - DNA, 41 bp, synthetic construct
  misc_feature 1..41: note = Target Specific Oligonucleotide
  source 1..41: mol_type = other DNA
ttacatggcttaagttggggagtagactgtattcaacgtcc

SEQ ID NO: 521 - DNA, 40 bp, synthetic construct
  misc_feature 1..40: note = Target Specific Oligonucleotide
  source 1..40: mol_type = other DNA
gtgaggggacgctcttgtatttagactgtattcaacgtcc

SEQ ID NO: 522 - DNA, 40 bp, synthetic construct
  misc_feature 1..40: note = Target Specific Oligonucleotide
  source 1..40: mol_type = other DNA
aacggtgctatgcctagtagatagactgtattcaacgtcc

SEQ ID NO: 523 - DNA, 40 bp, synthetic construct
  misc_feature 1..40: note = Target Specific Oligonucleotide
  source 1..40: mol_type = other DNA
tttgccttccctagagtgctatagactgtattcaacgtcc

SEQ ID NO: 524 - DNA, 43 bp, synthetic construct
  misc_feature 1..43: note = Target Specific Oligonucleotide
  source 1..43: mol_type = other DNA
atgtcccaatggatacttaaagcctagactgtattcaacgtcc

SEQ ID NO: 525 - DNA, 43 bp, synthetic construct
  misc_feature 1..43: note = Target Specific Oligonucleotide
  source 1..43: mol_type = other DNA
cttccagtaacgagatactttccttagactgtattcaacgtcc

SEQ ID NO: 526 - DNA, 42 bp, synthetic construct
  misc_feature 1..42: note = Target Specific Oligonucleotide
  source 1..42: mol_type = other DNA
caaccatgaattagtcccttgggtagactgtattcaacgtcc

SEQ ID NO: 527 - DNA, 44 bp, synthetic construct
  misc_feature 1..44: note = Target Specific Oligonucleotide
  source 1..44: mol_type = other DNA
cagcattattagacactttaactgttagactgtattcaacgtcc

SEQ ID NO: 528 - DNA, 43 bp, synthetic construct
  misc_feature 1..43: note = Target Specific Oligonucleotide
  source 1..43: mol_type = other DNA
tgcacatatgattgacgctcagtagactcttatattgagtggt

SEQ ID NO: 529 - DNA, 40 bp, synthetic construct
  misc_feature 1..40: note = Target Specific Oligonucleotide
  source 1..40: mol_type = other DNA
ttcaccgcctgcaacaagatagactcttatattgagtggt

SEQ ID NO: 530 - DNA, 44 bp, synthetic construct
  misc_feature 1..44: note = Target Specific Oligonucleotide
  source 1..44: mol_type = other DNA
ttcacttacaggtaacaccaagttagactcttatattgagtggt

SEQ ID NO: 531 - DNA, 45 bp, synthetic construct
  misc_feature 1..45: note = Target Specific Oligonucleotide
  source 1..45: mol_type = other DNA
aagcaatagatcgtccataagttatagactcttatattgagtggt

SEQ ID NO: 532 - DNA, 48 bp, synthetic construct
  misc_feature 1..48: note = Target Specific Oligonucleotide
  source 1..48: mol_type = other DNA
tacaagaaccctaattgtaataatagatagactcttatattgagtggt

SEQ ID NO: 533 - DNA, 44 bp, synthetic construct
  misc_feature 1..44: note = Target Specific Oligonucleotide
  source 1..44: mol_type = other DNA
gaataggaccaaagtgtcccttgtagactcttatattgagtggt

SEQ ID NO: 534 - DNA, 44 bp, synthetic construct
  misc_feature 1..44: note = Target Specific Oligonucleotide
  source 1..44: mol_type = other DNA
tccatcaggactaaatctcacactagactcttatattgagtggt

SEQ ID NO: 535 - DNA, 44 bp, synthetic construct
  misc_feature 1..44: note = Target Specific Oligonucleotide
  source 1..44: mol_type = other DNA
aaaggccatacgtttttcctacctagactcttatattgagtggt

SEQ ID NO: 536 - DNA, 44 bp, synthetic construct
  misc_feature 1..44: note = Target Specific Oligonucleotide
  source 1..44: mol_type = other DNA
gcagtgtacaatgaacgagaaattagactcttatattgagtggt

SEQ ID NO: 537 - DNA, 44 bp, synthetic construct
  misc_feature 1..44: note = Target Specific Oligonucleotide
  source 1..44: mol_type = other DNA
ggcattctgctttaagatcagaatagactcttatattgagtggt

SEQ ID NO: 538 - DNA, 40 bp, synthetic construct
  misc_feature 1..40: note = Target Specific Oligonucleotide
  source 1..40: mol_type = other DNA
ggccagccacgattcacagtagactcttatattgagtggt

SEQ ID NO: 539 - DNA, 39 bp, synthetic construct
  misc_feature 1..39: note = Target Specific Oligonucleotide
  source 1..39: mol_type = other DNA
gaagccagcgaccggacttagactcttatattgagtggt

SEQ ID NO: 540 - DNA, 41 bp, synthetic construct
  misc_feature 1..41: note = Target Specific Oligonucleotide
  source 1..41: mol_type = other DNA
ctgagggtcgtcgttgtctttagactcttatattgagtggt

SEQ ID NO: 541 - DNA, 43 bp, synthetic construct
  misc_feature 1..43: note = Target Specific Oligonucleotide
  source 1..43: mol_type = other DNA
ctgaaccactggcatagagttctagactcttatattgagtggt

SEQ ID NO: 542 - DNA, 40 bp, synthetic construct
  misc_feature 1..40: note = Target Specific Oligonucleotide
  source 1..40: mol_type = other DNA
aaatcaaccacgggtcgcgtagactcttatattgagtggt

SEQ ID NO: 543 - DNA, 40 bp, synthetic construct
  misc_feature 1..40: note = Target Specific Oligonucleotide
  source 1..40: mol_type = other DNA
agcaacagtcgacgagggatagactcttatattgagtggt

SEQ ID NO: 544 - DNA, 48 bp, synthetic construct
  misc_feature 1..48: note = Target Specific Oligonucleotide
  source 1..48: mol_type = other DNA
atatattccatactactaacagacatatagactcttatattgagtggt

SEQ ID NO: 545 - DNA, 38 bp, synthetic construct
  misc_feature 1..38: note = Target Specific Oligonucleotide
  source 1..38: mol_type = other DNA
tccacaccggcatcggctagactcttatattgagtggt

SEQ ID NO: 546 - DNA, 40 bp, synthetic construct
  misc_feature 1..40: note = Target Specific Oligonucleotide
  source 1..40: mol_type = other DNA
agaagggcaatccggtggctagactcttatattgagtggt

SEQ ID NO: 547 - DNA, 40 bp, synthetic construct
  misc_feature 1..40: note = Target Specific Oligonucleotide
  source 1..40: mol_type = other DNA
tcagggagtctgcgaccagtagactcttatattgagtggt

SEQ ID NO: 548 - DNA, 40 bp, synthetic construct
  misc_feature 1..40: note = Target Specific Oligonucleotide
  source 1..40: mol_type = other DNA
gctttgccagctcaccacttagactcttatattgagtggt

SEQ ID NO: 549 - DNA, 43 bp, synthetic construct
  misc_feature 1..43: note = Target Specific Oligonucleotide
  source 1..43: mol_type = other DNA
aaatacccataaggcgtgatgctagactcttatattgagtggt

SEQ ID NO: 550 - DNA, 44 bp, synthetic construct
  misc_feature 1..44: note = Target Specific Oligonucleotide
  source 1..44: mol_type = other DNA
attactatcctgcgtgaaatccatagactcttatattgagtggt

SEQ ID NO: 551 - DNA, 43 bp, synthetic construct
  misc_feature 1..43: note = Target Specific Oligonucleotide
  source 1..43: mol_type = other DNA
cccaaagtcgaacagttttgtctagactcttatattgagtggt

SEQ ID NO: 552 - DNA, 41 bp, synthetic construct
  misc_feature 1..41: note = Target Specific Oligonucleotide
  source 1..41: mol_type = other DNA
tcctcaaatgtccgaggatgatagacctattctatgcttcg

SEQ ID NO: 553 - DNA, 42 bp, synthetic construct
  misc_feature 1..42: note = Target Specific Oligonucleotide
  source 1..42: mol_type = other DNA
gtgaacacaacgtaagaacaggtagacctattctatgcttcg

SEQ ID NO: 554 - DNA, 42 bp, synthetic construct
  misc_feature 1..42: note = Target Specific Oligonucleotide
  source 1..42: mol_type = other DNA
actcctctggttacgcttcatttagacctattctatgcttcg

SEQ ID NO: 555 - DNA, 41 bp, synthetic construct
  misc_feature 1..41: note = Target Specific Oligonucleotide
  source 1..41: mol_type = other DNA
acctaacataaccgtgctgcctagacctattctatgcttcg

SEQ ID NO: 556 - DNA, 41 bp, synthetic construct
  misc_feature 1..41: note = Target Specific Oligonucleotide
  source 1..41: mol_type = other DNA
ttcagttgaccgtctggacactagacctattctatgcttcg

SEQ ID NO: 557 - DNA, 43 bp, synthetic construct
  misc_feature 1..43: note = Target Specific Oligonucleotide
  source 1..43: mol_type = other DNA
ctctgacacacgtaacaataacatagacctattctatgcttcg

SEQ ID NO: 558 - DNA, 43 bp, synthetic construct
  misc_feature 1..43: note = Target Specific Oligonucleotide
  source 1..43: mol_type = other DNA
agtaatgtgaggtacaactgcattagacctattctatgcttcg

SEQ ID NO: 559 - DNA, 41 bp, synthetic construct
  misc_feature 1..41: note = Target Specific Oligonucleotide
  source 1..41: mol_type = other DNA
gcttctttcccgcccaaaatatagacctattctatgcttcg

SEQ ID NO: 560 - DNA, 44 bp, synthetic construct
  misc_feature 1..44: note = Target Specific Oligonucleotide
  source 1..44: mol_type = other DNA
aaagaaaagcggtctactagattatagacctattctatgcttcg

SEQ ID NO: 561 - DNA, 41 bp, synthetic construct
  misc_feature 1..41: note = Target Specific Oligonucleotide
  source 1..41: mol_type = other DNA
tgacgtgcggcgaaatttatgtagacctattctatgcttcg

SEQ ID NO: 562 - DNA, 41 bp, synthetic construct
  misc_feature 1..41: note = Target Specific Oligonucleotide
  source 1..41: mol_type = other DNA
gcttattgcagcgatggatgatagacctattctatgcttcg

SEQ ID NO: 563 - DNA, 42 bp, synthetic construct
  misc_feature 1..42: note = Target Specific Oligonucleotide
  source 1..42: mol_type = other DNA
tgtcagtagacgatagaggaggtagacctattctatgcttcg

SEQ ID NO: 564 - DNA, 41 bp, synthetic construct
  misc_feature 1..41: note = Target Specific Oligonucleotide
  source 1..41: mol_type = other DNA
ttggttccgactacccaacagtagacctattctatgcttcg

SEQ ID NO: 565 - DNA, 45 bp, synthetic construct
  misc_feature 1..45: note = Target Specific Oligonucleotide
  source 1..45: mol_type = other DNA
ctcttaagtacgcaataattctctctagacctattctatgcttcg

SEQ ID NO: 566 - DNA, 43 bp, synthetic construct
  misc_feature 1..43: note = Target Specific Oligonucleotide
  source 1..43: mol_type = other DNA
gttccgtatatgtcggatctctctagacctattctatgcttcg

SEQ ID NO: 567 - DNA, 41 bp, synthetic construct
  misc_feature 1..41: note = Target Specific Oligonucleotide
  source 1..41: mol_type = other DNA
aaattcaccggacggagtgtttagacctattctatgcttcg

SEQ ID NO: 568 - DNA, 42 bp, synthetic construct
  misc_feature 1..42: note = Target Specific Oligonucleotide
  source 1..42: mol_type = other DNA
tttgtgaaaccgtagtggctcttagacctattctatgcttcg

SEQ ID NO: 569 - DNA, 42 bp, synthetic construct
  misc_feature 1..42: note = Target Specific Oligonucleotide
  source 1..42: mol_type = other DNA
acctctttaacgaaggtgtcagtagacctattctatgcttcg

SEQ ID NO: 570 - DNA, 41 bp, synthetic construct
  misc_feature 1..41: note = Target Specific Oligonucleotide
  source 1..41: mol_type = other DNA
ggactccggttctaacttggttagacctattctatgcttcg

SEQ ID NO: 571 - DNA, 43 bp, synthetic construct
  misc_feature 1..43: note = Target Specific Oligonucleotide
  source 1..43: mol_type = other DNA
atctctatatgacgtgctgttggtagacctattctatgcttcg

SEQ ID NO: 572 - DNA, 43 bp, synthetic construct
  misc_feature 1..43: note = Target Specific Oligonucleotide
  source 1..43: mol_type = other DNA
gttggaattattcggagactgagtagacctattctatgcttcg

SEQ ID NO: 573 - DNA, 40 bp, synthetic construct
  misc_feature 1..40: note = Target Specific Oligonucleotide
  source 1..40: mol_type = other DNA
gcacatttgacgacggcttctagacctattctatgcttcg

SEQ ID NO: 574 - DNA, 40 bp, synthetic construct
  misc_feature 1..40: note = Target Specific Oligonucleotide
  source 1..40: mol_type = other DNA
actccgtgtaaacgcagtggtagacctattctatgcttcg

SEQ ID NO: 575 - DNA, 43 bp, synthetic construct
  misc_feature 1..43: note = Target Specific Oligonucleotide
  source 1..43: mol_type = other DNA
acacataactcgttaacacgttctagacctattctatgcttcg

SEQ ID NO: 576 - DNA, 42 bp, synthetic construct
  misc_feature 1..42: note = Target Specific Oligonucleotide
  source 1..42: mol_type = other DNA
cagatctgttgagctaacagggtagacatgttataccatgcg

SEQ ID NO: 577 - DNA, 44 bp, synthetic construct
  misc_feature 1..44: note = Target Specific Oligonucleotide
  source 1..44: mol_type = other DNA
ttctagactatgcaaccctctaggtagacatgttataccatgcg

SEQ ID NO: 578 - DNA, 43 bp, synthetic construct
  misc_feature 1..43: note = Target Specific Oligonucleotide
  source 1..43: mol_type = other DNA
cacccatgtgagtaatacactgctagacatgttataccatgcg

SEQ ID NO: 579 - DNA, 42 bp, synthetic construct
  misc_feature 1..42: note = Target Specific Oligonucleotide
  source 1..42: mol_type = other DNA
agtcccatattgccgttcatgctagacatgttataccatgcg

SEQ ID NO: 580 - DNA, 42 bp, synthetic construct
  misc_feature 1..42: note = Target Specific Oligonucleotide
  source 1..42: mol_type = other DNA
atttcctcataacggtcatggctagacatgttataccatgcg

SEQ ID NO: 581 - DNA, 42 bp, synthetic construct
  misc_feature 1..42: note = Target Specific Oligonucleotide
  source 1..42: mol_type = other DNA
ttactgcctagctagcaggttatagacatgttataccatgcg

SEQ ID NO: 582 - DNA, 41 bp, synthetic construct
  misc_feature 1..41: note = Target Specific Oligonucleotide
  source 1..41: mol_type = other DNA
acgtgcccttggtactatgactagacatgttataccatgcg

SEQ ID NO: 583 - DNA, 41 bp, synthetic construct
  misc_feature 1..41: note = Target Specific Oligonucleotide
  source 1..41: mol_type = other DNA
cttgccaaaccctagcttggatagacatgttataccatgcg

SEQ ID NO: 584 - DNA, 45 bp, synthetic construct
  misc_feature 1..45: note = Target Specific Oligonucleotide
  source 1..45: mol_type = other DNA
attatcacttaacgaaggtcctttgtagacatgttataccatgcg

SEQ ID NO: 585 - DNA, 45 bp, synthetic construct
  misc_feature 1..45: note = Target Specific Oligonucleotide
  source 1..45: mol_type = other DNA
atatacagcctaagcaccaattatgtagacatgttataccatgcg

SEQ ID NO: 586 - DNA, 40 bp, synthetic construct
  misc_feature 1..40: note = Target Specific Oligonucleotide
  source 1..40: mol_type = other DNA
ggcaacaaaacgtcatggcatagacatgttataccatgcg

SEQ ID NO: 587 - DNA, 43 bp, synthetic construct
  misc_feature 1..43: note = Target Specific Oligonucleotide
  source 1..43: mol_type = other DNA
gtctgaggactaaccctaaagggtagacatgttataccatgcg

SEQ ID NO: 588 - DNA, 46 bp, synthetic construct
  misc_feature 1..46: note = Target Specific Oligonucleotide
  source 1..46: mol_type = other DNA
cttaaaatagatcgaaactctgtctctagacatgttataccatgcg

SEQ ID NO: 589 - DNA, 44 bp, synthetic construct
  misc_feature 1..44: note = Target Specific Oligonucleotide
  source 1..44: mol_type = other DNA
tgatctgtacaagctacgattttatagacatgttataccatgcg

SEQ ID NO: 590 - DNA, 43 bp, synthetic construct
  misc_feature 1..43: note = Target Specific Oligonucleotide
  source 1..43: mol_type = other DNA
aaatcagttataccaaggggagatagacatgttataccatgcg

SEQ ID NO: 591 - DNA, 45 bp, synthetic construct
  misc_feature 1..45: note = Target Specific Oligonucleotide
  source 1..45: mol_type = other DNA
taggaaaacatacgtatactgaatatagacatgttataccatgcg

SEQ ID NO: 592 - DNA, 40 bp, synthetic construct
  misc_feature 1..40: note = Target Specific Oligonucleotide
  source 1..40: mol_type = other DNA
agttggcctcacgttgcatttagacatgttataccatgcg

SEQ ID NO: 593 - DNA, 40 bp, synthetic construct
  misc_feature 1..40: note = Target Specific Oligonucleotide
  source 1..40: mol_type = other DNA
tttggtctcggcttgcgaattagacatgttataccatgcg

SEQ ID NO: 594 - DNA, 41 bp, synthetic construct
  misc_feature 1..41: note = Target Specific Oligonucleotide
  source 1..41: mol_type = other DNA
cagtagtcaacgcagcactcatagacatgttataccatgcg

SEQ ID NO: 595 - DNA, 44 bp, synthetic construct
  misc_feature 1..44: note = Target Specific Oligonucleotide
  source 1..44: mol_type = other DNA
caacaggatcacctaatattcccatagacatgttataccatgcg

SEQ ID NO: 596 - DNA, 43 bp, synthetic construct
  misc_feature 1..43: note = Target Specific Oligonucleotide
  source 1..43: mol_type = other DNA
tttggacagatatctcctcgaaatagacatgttataccatgcg

SEQ ID NO: 597 - DNA, 43 bp, synthetic construct
  misc_feature 1..43: note = Target Specific Oligonucleotide
  source 1..43: mol_type = other DNA
aaaggctatctacactttggcaatagacatgttataccatgcg

SEQ ID NO: 598 - DNA, 40 bp, synthetic construct
  misc_feature 1..40: note = Target Specific Oligonucleotide
  source 1..40: mol_type = other DNA
tgcctggatcctatcccgactagacatgttataccatgcg

SEQ ID NO: 599 - DNA, 40 bp, synthetic construct
  misc_feature 1..40: note = Target Specific Oligonucleotide
  source 1..40: mol_type = other DNA
tgtggtcacctacacgctgctagacatgttataccatgcg

SEQ ID NO: 600 - DNA, 43 bp, synthetic construct
  misc_feature 1..43: note = Target Specific Oligonucleotide
  source 1..43: mol_type = other DNA
ggtgagctggtaatctgaccttagacaatctatttaccctacg

SEQ ID NO: 601 - DNA, 41 bp, synthetic construct
  misc_feature 1..41: note = Target Specific Oligonucleotide
  source 1..41: mol_type = other DNA
gttgcaggcatgacgcaagtagacaatctatttaccctacg

SEQ ID NO: 602 - DNA, 43 bp, synthetic construct
  misc_feature 1..43: note = Target Specific Oligonucleotide
  source 1..43: mol_type = other DNA
aaaacgcctacgcatcatgtctagacaatctatttaccctacg

SEQ ID NO: 603 - DNA, 40 bp, synthetic construct
  misc_feature 1..40: note = Target Specific Oligonucleotide
  source 1..40: mol_type = other DNA
tggtcctgcgcggatgtctagacaatctatttaccctacg

SEQ ID NO: 604 - DNA, 41 bp, synthetic construct
  misc_feature 1..41: note = Target Specific Oligonucleotide
  source 1..41: mol_type = other DNA
ggtgagcttctccgtggcgtagacaatctatttaccctacg

SEQ ID NO: 605 - DNA, 41 bp, synthetic construct
  misc_feature 1..41: note = Target Specific Oligonucleotide
  source 1..41: mol_type = other DNA
agcgcagggccaattgacttagacaatctatttaccctacg

SEQ ID NO: 606 - DNA, 43 bp, synthetic construct
  misc_feature 1..43: note = Target Specific Oligonucleotide
  source 1..43: mol_type = other DNA
ccgggtacacggttttgatcttagacaatctatttaccctacg

SEQ ID NO: 607 - DNA, 40 bp, synthetic construct
  misc_feature 1..40: note = Target Specific Oligonucleotide
  source 1..40: mol_type = other DNA
ccggctcgatgtcgggtatagacaatctatttaccctacg

SEQ ID NO: 608 - DNA, 40 bp, synthetic construct
  misc_feature 1..40: note = Target Specific Oligonucleotide
  source 1..40: mol_type = other DNA
ggcgccttctcgccacattagacaatctatttaccctacg

SEQ ID NO: 609 - DNA, 40 bp, synthetic construct
  misc_feature 1..40: note = Target Specific Oligonucleotide
  source 1..40: mol_type = other DNA
cacgttgaagcgcgggtgtagacaatctatttaccctacg

SEQ ID NO: 610 - DNA, 44 bp, synthetic construct
  misc_feature 1..44: note = Target Specific Oligonucleotide
  source 1..44: mol_type = other DNA
gcccacagaaaccggtttaatgtagacaatctatttaccctacg

SEQ ID NO: 611 - DNA, 43 bp, synthetic construct
  misc_feature 1..43: note = Target Specific Oligonucleotide
  source 1..43: mol_type = other DNA
tcagaatgagcgcaatccaggtagacaatctatttaccctacg

SEQ ID NO: 612 - DNA, 42 bp, synthetic construct
  misc_feature 1..42: note = Target Specific Oligonucleotide
  source 1..42: mol_type = other DNA
ttcggacacaaagacgctcctagacaatctatttaccctacg

SEQ ID NO: 613 - DNA, 42 bp, synthetic construct
  misc_feature 1..42: note = Target Specific Oligonucleotide
  source 1..42: mol_type = other DNA
agcttgacgtaggtgtcggttagacaatctatttaccctacg

SEQ ID NO: 614 - DNA, 42 bp, synthetic construct
  misc_feature 1..42: note = Target Specific Oligonucleotide
  source 1..42: mol_type = other DNA
ggttcccgccaaatttcccgtagacaatctatttaccctacg

SEQ ID NO: 615 - DNA, 45 bp, synthetic construct
  misc_feature 1..45: note = Target Specific Oligonucleotide
  source 1..45: mol_type = other DNA
cagggctcatgatagtacaacagtagacaatctatttaccctacg

SEQ ID NO: 616 - DNA, 41 bp, synthetic construct
  misc_feature 1..41: note = Target Specific Oligonucleotide
  source 1..41: mol_type = other DNA
ggactttagcgcggtctcctagacaatctatttaccctacg

SEQ ID NO: 617 - DNA, 41 bp, synthetic construct
  misc_feature 1..41: note = Target Specific Oligonucleotide
  source 1..41: mol_type = other DNA
gcagccgttctaagcgctgtagacaatctatttaccctacg

SEQ ID NO: 618 - DNA, 41 bp, synthetic construct
  misc_feature 1..41: note = Target Specific Oligonucleotide
  source 1..41: mol_type = other DNA
gctggtaaaggcgcttccctagacaatctatttaccctacg

SEQ ID NO: 619 - DNA, 41 bp, synthetic construct
  misc_feature 1..41: note = Target Specific Oligonucleotide
  source 1..41: mol_type = other DNA
gaagaagtcggtgacgcggtagacaatctatttaccctacg

SEQ ID NO: 620 - DNA, 41 bp, synthetic construct
  misc_feature 1..41: note = Target Specific Oligonucleotide
  source 1..41: mol_type = other DNA
ggctggaaacctcgtccactagacaatctatttaccctacg

SEQ ID NO: 621 - DNA, 48 bp, synthetic construct
  misc_feature 1..48: note = Target Specific Oligonucleotide
  source 1..48: mol_type = other DNA
tttattagagtttaggaggtcagaaatagacaatctatttaccctacg

SEQ ID NO: 622 - DNA, 44 bp, synthetic construct
  misc_feature 1..44: note = Target Specific Oligonucleotide
  source 1..44: mol_type = other DNA
tgggaggtcccatattcagaggtagacaatctatttaccctacg

SEQ ID NO: 623 - DNA, 44 bp, synthetic construct
  misc_feature 1..44: note = Target Specific Oligonucleotide
  source 1..44: mol_type = other DNA
tccagggatgtcctacttgtcctagacaatctatttaccctacg

SEQ ID NO: 624 - DNA, 40 bp, synthetic construct
  misc_feature 1..40: note = Target Specific Oligonucleotide
  source 1..40: mol_type = other DNA
ccaggtttccggcacagtgggtaactgaattgtcacttta

SEQ ID NO: 625 - DNA, 46 bp, synthetic construct
  misc_feature 1..46: note = Target Specific Oligonucleotide
  source 1..46: mol_type = other DNA
tgttatactttgtcgctcttagtagagtaactgaattgtcacttta

SEQ ID NO: 626 - DNA, 44 bp, synthetic construct
  misc_feature 1..44: note = Target Specific Oligonucleotide
  source 1..44: mol_type = other DNA
agcttttaaccaggtttcgacttcgtaactgaattgtcacttta

SEQ ID NO: 627 - DNA, 45 bp, synthetic construct
  misc_feature 1..45: note = Target Specific Oligonucleotide
  source 1..45: mol_type = other DNA
gtatgagaatcccgataaaactggtgtaactgaattgtcacttta

SEQ ID NO: 628 - DNA, 43 bp, synthetic construct
  misc_feature 1..43: note = Target Specific Oligonucleotide
  source 1..43: mol_type = other DNA
aagaggacatcgaccaatcctcagtaactgaattgtcacttta

SEQ ID NO: 629 - DNA, 42 bp, synthetic construct
  misc_feature 1..42: note = Target Specific Oligonucleotide
  source 1..42: mol_type = other DNA
ggtttgtgcaagggtcgaaaacgtaactgaattgtcacttta

SEQ ID NO: 630 - DNA, 44 bp, synthetic construct
  misc_feature 1..44: note = Target Specific Oligonucleotide
  source 1..44: mol_type = other DNA
acacctctcgtagctatagatgtggtaactgaattgtcacttta

SEQ ID NO: 631 - DNA, 41 bp, synthetic construct
  misc_feature 1..41: note = Target Specific Oligonucleotide
  source 1..41: mol_type = other DNA
atgagagggcaaccgaggtgagtaactgaattgtcacttta

SEQ ID NO: 632 - DNA, 43 bp, synthetic construct
  misc_feature 1..43: note = Target Specific Oligonucleotide
  source 1..43: mol_type = other DNA
ccgctgtcagggtctatcattccgtaactgaattgtcacttta

SEQ ID NO: 633 - DNA, 41 bp, synthetic construct
  misc_feature 1..41: note = Target Specific Oligonucleotide
  source 1..41: mol_type = other DNA
gcaatgagcatatcctcgggcgtaactgaattgtcacttta

SEQ ID NO: 634 - DNA, 41 bp, synthetic construct
  misc_feature 1..41: note = Target Specific Oligonucleotide
  source 1..41: mol_type = other DNA
ggcttgagtgggttcacccaggtaactgaattgtcacttta

SEQ ID NO: 635 - DNA, 43 bp, synthetic construct
  misc_feature 1..43: note = Target Specific Oligonucleotide
  source 1..43: mol_type = other DNA
gcaaggtatggcaatagctgagtgtaactgaattgtcacttta

SEQ ID NO: 636 - DNA, 45 bp, synthetic construct
  misc_feature 1..45: note = Target Specific Oligonucleotide
  source 1..45: mol_type = other DNA
cagtaatagtagagacgccactacagtaactgaattgtcacttta

SEQ ID NO: 637 - DNA, 43 bp, synthetic construct
  misc_feature 1..43: note = Target Specific Oligonucleotide
  source 1..43: mol_type = other DNA
cttccaaagtgtcgcttcagagggtaactgaattgtcacttta

SEQ ID NO: 638 - DNA, 46 bp, synthetic construct
  misc_feature 1..46: note = Target Specific Oligonucleotide
  source 1..46: mol_type = other DNA
aggcaattttcccgatactttttattgtaactgaattgtcacttta

SEQ ID NO: 639 - DNA, 46 bp, synthetic construct
  misc_feature 1..46: note = Target Specific Oligonucleotide
  source 1..46: mol_type = other DNA
tgttagcttctatagtcactattcgagtaactgaattgtcacttta

SEQ ID NO: 640 - DNA, 45 bp, synthetic construct
  misc_feature 1..45: note = Target Specific Oligonucleotide
  source 1..45: mol_type = other DNA
tcaacaagtaatgtatcccgttcatgtaactgaattgtcacttta

SEQ ID NO: 641 - DNA, 44 bp, synthetic construct
  misc_feature 1..44: note = Target Specific Oligonucleotide
  source 1..44: mol_type = other DNA
tttccttggccgtaagttgttttcgtaactgaattgtcacttta

SEQ ID NO: 642 - DNA, 42 bp, synthetic construct
  misc_feature 1..42: note = Target Specific Oligonucleotide
  source 1..42: mol_type = other DNA
gggtcaacccagtctgttacctgtaactgaattgtcacttta

SEQ ID NO: 643 - DNA, 46 bp, synthetic construct
  misc_feature 1..46: note = Target Specific Oligonucleotide
  source 1..46: mol_type = other DNA
tctgagactgatagggaaacatatgggtaactgaattgtcacttta

SEQ ID NO: 644 - DNA, 42 bp, synthetic construct
  misc_feature 1..42: note = Target Specific Oligonucleotide
  source 1..42: mol_type = other DNA
tctttgccaccaatagcttggagtaactgaattgtcacttta

SEQ ID NO: 645 - DNA, 45 bp, synthetic construct
  misc_feature 1..45: note = Target Specific Oligonucleotide
  source 1..45: mol_type = other DNA
ctcattggaatggttagtagagcaagtaactgaattgtcacttta

SEQ ID NO: 646 - DNA, 44 bp, synthetic construct
  misc_feature 1..44: note = Target Specific Oligonucleotide
  source 1..44: mol_type = other DNA
ctgagtaaagagcgtgtattccaggtaactgaattgtcacttta

SEQ ID NO: 647 - DNA, 42 bp, synthetic construct
  misc_feature 1..42: note = Target Specific Oligonucleotide
  source 1..42: mol_type = other DNA
tggaggcataaagctggtaggcgtaactgaattgtcacttta

SEQ ID NO: 648 - DNA, 42 bp, synthetic construct
  misc_feature 1..42: note = Target Specific Oligonucleotide
  source 1..42: mol_type = other DNA
ggatctcaagcgttgcaggcgtaacgatagatttatacgacg

SEQ ID NO: 649 - DNA, 39 bp, synthetic construct
  misc_feature 1..39: note = Target Specific Oligonucleotide
  source 1..39: mol_type = other DNA
gcaccgcgagcggactagtaacgatagatttatacgacg

SEQ ID NO: 650 - DNA, 41 bp, synthetic construct
  misc_feature 1..41: note = Target Specific Oligonucleotide
  source 1..41: mol_type = other DNA
tgctgaggtcgctcacgaagtaacgatagatttatacgacg

SEQ ID NO: 651 - DNA, 44 bp, synthetic construct
  misc_feature 1..44: note = Target Specific Oligonucleotide
  source 1..44: mol_type = other DNA
ccggaccacgtagttaaatcttgtaacgatagatttatacgacg

SEQ ID NO: 652 - DNA, 43 bp, synthetic construct
  misc_feature 1..43: note = Target Specific Oligonucleotide
  source 1..43: mol_type = other DNA
aagttcttttgggcgatgccagtaacgatagatttatacgacg

SEQ ID NO: 653 - DNA, 48 bp, synthetic construct
  misc_feature 1..48: note = Target Specific Oligonucleotide
  source 1..48: mol_type = other DNA
gttcccttattagtctaatgttttgcgtaacgatagatttatacgacg

SEQ ID NO: 654 - DNA, 45 bp, synthetic construct
  misc_feature 1..45: note = Target Specific Oligonucleotide
  source 1..45: mol_type = other DNA
ttggaccagtgtacataaggatggtaacgatagatttatacgacg

SEQ ID NO: 655 - DNA, 41 bp, synthetic construct
  misc_feature 1..41: note = Target Specific Oligonucleotide
  source 1..41: mol_type = other DNA
tggcagtgcacggatggtcgtaacgatagatttatacgacg

SEQ ID NO: 656 - DNA, 47 bp, synthetic construct
  misc_feature 1..47: note = Target Specific Oligonucleotide
  source 1..47: mol_type = other DNA
ataccaattctagtgagaagttcacgtaacgatagatttatacgacg

SEQ ID NO: 657 - DNA, 44 bp, synthetic construct
  misc_feature 1..44: note = Target Specific Oligonucleotide
  source 1..44: mol_type = other DNA
tctctgtagggtaaggctctgtgtaacgatagatttatacgacg

SEQ ID NO: 658 - DNA, 45 bp, synthetic construct
  misc_feature 1..45: note = Target Specific Oligonucleotide
  source 1..45: mol_type = other DNA
tttagaggtagaccattgtgtgggtaacgatagatttatacgacg

SEQ ID NO: 659 - DNA, 42 bp, synthetic construct
  misc_feature 1..42: note = Target Specific Oligonucleotide
  source 1..42: mol_type = other DNA
agagagggcactctacgcttgtaacgatagatttatacgacg

SEQ ID NO: 660 - DNA, 44 bp, synthetic construct
  misc_feature 1..44: note = Target Specific Oligonucleotide
  source 1..44: mol_type = other DNA
caaaaagccctagctcagatgggtaacgatagatttatacgacg

SEQ ID NO: 661 - DNA, 43 bp, synthetic construct
  misc_feature 1..43: note = Target Specific Oligonucleotide
  source 1..43: mol_type = other DNA
cctctcctccctatttggctggtaacgatagatttatacgacg

SEQ ID NO: 662 - DNA, 46 bp, synthetic construct
  misc_feature 1..46: note = Target Specific Oligonucleotide
  source 1..46: mol_type = other DNA
ttttacaacgaactcattaggtccgtaacgatagatttatacgacg

SEQ ID NO: 663 - DNA, 45 bp, synthetic construct
  misc_feature 1..45: note = Target Specific Oligonucleotide
  source 1..45: mol_type = other DNA
ggagtagatcccccatctattccgtaacgatagatttatacgacg

SEQ ID NO: 664 - DNA, 44 bp, synthetic construct
  misc_feature 1..44: note = Target Specific Oligonucleotide
  source 1..44: mol_type = other DNA
gtctcttgcctcgtttctctccgtaacgatagatttatacgacg

SEQ ID NO: 665 - DNA, 43 bp, synthetic construct
  misc_feature 1..43: note = Target Specific Oligonucleotide
  source 1..43: mol_type = other DNA
aattctggcgtagcacaaacagtaacgatagatttatacgacg

SEQ ID NO: 666 - DNA, 45 bp, synthetic construct
  misc_feature 1..45: note = Target Specific Oligonucleotide
  source 1..45: mol_type = other DNA
ggccatgaacccctaaatctaaagtaacgatagatttatacgacg

SEQ ID NO: 667 - DNA, 42 bp, synthetic construct
  misc_feature 1..42: note = Target Specific Oligonucleotide
  source 1..42: mol_type = other DNA
gcccactggtaccatcttgggtaacgatagatttatacgacg

SEQ ID NO: 668 - DNA, 42 bp, synthetic construct
  misc_feature 1..42: note = Target Specific Oligonucleotide
  source 1..42: mol_type = other DNA
taccacgtggcactaacacagtaacgatagatttatacgacg

SEQ ID NO: 669 - DNA, 45 bp, synthetic construct
  misc_feature 1..45: note = Target Specific Oligonucleotide
  source 1..45: mol_type = other DNA
ttctagcttttagaccagcagttgtaacgatagatttatacgacg

SEQ ID NO: 670 - DNA, 44 bp, synthetic construct
  misc_feature 1..44: note = Target Specific Oligonucleotide
  source 1..44: mol_type = other DNA
cccaagtgctagtagaacctgcgtaacgatagatttatacgacg

SEQ ID NO: 671 - DNA, 47 bp, synthetic construct
  misc_feature 1..47: note = Target Specific Oligonucleotide
  source 1..47: mol_type = other DNA
aaacacatctatactcaaagacagagtaacgatagatttatacgacg

SEQ ID NO: 672 - DNA, 43 bp, synthetic construct
  misc_feature 1..43: note = Target Specific Oligonucleotide
  source 1..43: mol_type = other DNA
cacagacttgccgactctttggtaacgatagatttatacgacg

SEQ ID NO: 673 - DNA, 44 bp, synthetic construct
  misc_feature 1..44: note = Target Specific Oligonucleotide
  source 1..44: mol_type = other DNA
cacatgttaatgttcccgaccagtaacgatagatttatacgacg

SEQ ID NO: 674 - DNA, 44 bp, synthetic construct
  misc_feature 1..44: note = Target Specific Oligonucleotide
  source 1..44: mol_type = other DNA
attaatcgtttgcggatctgccgtaacgatagatttatacgacg

SEQ ID NO: 675 - DNA, 44 bp, synthetic construct
  misc_feature 1..44: note = Target Specific Oligonucleotide
  source 1..44: mol_type = other DNA
tgggtaacatcggacaagtttggtaacgatagatttatacgacg

SEQ ID NO: 676 - DNA, 44 bp, synthetic construct
  misc_feature 1..44: note = Target Specific Oligonucleotide
  source 1..44: mol_type = other DNA
tctgaagtttcgagccaatgttgtaacgatagatttatacgacg

SEQ ID NO: 677 - DNA, 44 bp, synthetic construct
  misc_feature 1..44: note = Target Specific Oligonucleotide
  source 1..44: mol_type = other DNA
ccattttcaccgctgaaatagagtaacgatagatttatacgacg

SEQ ID NO: 678 - DNA, 43 bp, synthetic construct
  misc_feature 1..43: note = Target Specific Oligonucleotide
  source 1..43: mol_type = other DNA
ctggatcacatgcgttgtcaggtaacgatagatttatacgacg

SEQ ID NO: 679 - DNA, 45 bp, synthetic construct
  misc_feature 1..45: note = Target Specific Oligonucleotide
  source 1..45: mol_type = other DNA
atatttgcctcgtaagatcccctgtaacgatagatttatacgacg

SEQ ID NO: 680 - DNA, 45 bp, synthetic construct
  misc_feature 1..45: note = Target Specific Oligonucleotide
  source 1..45: mol_type = other DNA
ctgaagcggtgttgtatcatagcgtaacgatagatttatacgacg

SEQ ID NO: 681 - DNA, 45 bp, synthetic construct
  misc_feature 1..45: note = Target Specific Oligonucleotide
  source 1..45: mol_type = other DNA
tagaataatggttcgtgaccttcgtaacgatagatttatacgacg

SEQ ID NO: 682 - DNA, 41 bp, synthetic construct
  misc_feature 1..41: note = Target Specific Oligonucleotide
  source 1..41: mol_type = other DNA
acctgaaggcgacgaggaggtaacgatagatttatacgacg

SEQ ID NO: 683 - DNA, 44 bp, synthetic construct
  misc_feature 1..44: note = Target Specific Oligonucleotide
  source 1..44: mol_type = other DNA
gcctggagtctatcgtacaatcgtaacgatagatttatacgacg

SEQ ID NO: 684 - DNA, 47 bp, synthetic construct
  misc_feature 1..47: note = Target Specific Oligonucleotide
  source 1..47: mol_type = other DNA
acatttaattagaccgtaacccttcgtaacgatagatttatacgacg

SEQ ID NO: 685 - DNA, 45 bp, synthetic construct
  misc_feature 1..45: note = Target Specific Oligonucleotide
  source 1..45: mol_type = other DNA
gctctggccatacttaacagatagtaacgatagatttatacgacg

SEQ ID NO: 686 - DNA, 46 bp, synthetic construct
  misc_feature 1..46: note = Target Specific Oligonucleotide
  source 1..46: mol_type = other DNA
cagcattgagtgataatgcaatctgtaacgatagatttatacgacg

SEQ ID NO: 687 - DNA, 44 bp, synthetic construct
  misc_feature 1..44: note = Target Specific Oligonucleotide
  source 1..44: mol_type = other DNA
atacacacccgctaccttactggtaacgatagatttatacgacg

SEQ ID NO: 688 - DNA, 44 bp, synthetic construct
  misc_feature 1..44: note = Target Specific Oligonucleotide
  source 1..44: mol_type = other DNA
acaaagacgagaactatggcaagtaacgatagatttatacgacg

SEQ ID NO: 689 - DNA, 44 bp, synthetic construct
  misc_feature 1..44: note = Target Specific Oligonucleotide
  source 1..44: mol_type = other DNA
aggcagacgctctaagtctaaagtaacgatagatttatacgacg

SEQ ID NO: 690 - DNA, 44 bp, synthetic construct
  misc_feature 1..44: note = Target Specific Oligonucleotide
  source 1..44: mol_type = other DNA
tctcttactcatcgtgaaaggcgtaacgatagatttatacgacg

SEQ ID NO: 691 - DNA, 42 bp, synthetic construct
  misc_feature 1..42: note = Target Specific Oligonucleotide
  source 1..42: mol_type = other DNA
gcctcaagttcgcattcagcgtaacgatagatttatacgacg

SEQ ID NO: 692 - DNA, 44 bp, synthetic construct
  misc_feature 1..44: note = Target Specific Oligonucleotide
  source 1..44: mol_type = other DNA
gaaatggaaacgttaacagccagtaacgatagatttatacgacg

SEQ ID NO: 693 - DNA, 43 bp, synthetic construct
  misc_feature 1..43: note = Target Specific Oligonucleotide
  source 1..43: mol_type = other DNA
cacctgcttcggaatctcagtgtaacgatagatttatacgacg

SEQ ID NO: 694 - DNA, 46 bp, synthetic construct
  misc_feature 1..46: note = Target Specific Oligonucleotide
  source 1..46: mol_type = other DNA
gacttgtgcttcgttaattaaacagtaacgatagatttatacgacg

SEQ ID NO: 695 - DNA, 46 bp, synthetic construct
  misc_feature 1..46: note = Target Specific Oligonucleotide
  source 1..46: mol_type = other DNA
gctgtaatatacgcccactttagcgtaacgatagatttatacgacg

SEQ ID NO: 696 - DNA, 44 bp, synthetic construct
  misc_feature 1..44: note = Target Specific Oligonucleotide
  source 1..44: mol_type = other DNA
ttccattgtgcggttgggattgtaacttataaaggatagacatc

SEQ ID NO: 697 - DNA, 45 bp, synthetic construct
  misc_feature 1..45: note = Target Specific Oligonucleotide
  source 1..45: mol_type = other DNA
ctccagtaatcgcttatggtccgtaacttataaaggatagacatc

SEQ ID NO: 698 - DNA, 45 bp, synthetic construct
  misc_feature 1..45: note = Target Specific Oligonucleotide
  source 1..45: mol_type = other DNA
cctcttctccgtcaagaagttcgtaacttataaaggatagacatc

SEQ ID NO: 699 - DNA, 45 bp, synthetic construct
  misc_feature 1..45: note = Target Specific Oligonucleotide
  source 1..45: mol_type = other DNA
tgattgagatggcggtatttgagtaacttataaaggatagacatc

SEQ ID NO: 700 - DNA, 45 bp, synthetic construct
  misc_feature 1..45: note = Target Specific Oligonucleotide
  source 1..45: mol_type = other DNA
gccaattataagtactcgggctgtaacttataaaggatagacatc

SEQ ID NO: 701 - DNA, 42 bp, synthetic construct
  misc_feature 1..42: note = Target Specific Oligonucleotide
  source 1..42: mol_type = other DNA
ccaggccagcgtatgttccgtaacttataaaggatagacatc

SEQ ID NO: 702 - DNA, 43 bp, synthetic construct
  misc_feature 1..43: note = Target Specific Oligonucleotide
  source 1..43: mol_type = other DNA
ctggggcaaccaacacttgtgtaacttataaaggatagacatc

SEQ ID NO: 703 - DNA, 43 bp, synthetic construct
  misc_feature 1..43: note = Target Specific Oligonucleotide
  source 1..43: mol_type = other DNA
ggctggacaataggctcccagtaacttataaaggatagacatc

SEQ ID NO: 704 - DNA, 44 bp, synthetic construct
  misc_feature 1..44: note = Target Specific Oligonucleotide
  source 1..44: mol_type = other DNA
aaagctatggcacgaaagccggtaacttataaaggatagacatc

SEQ ID NO: 705 - DNA, 44 bp, synthetic construct
  misc_feature 1..44: note = Target Specific Oligonucleotide
  source 1..44: mol_type = other DNA
gcagtccatctaaggtggactgtaacttataaaggatagacatc

SEQ ID NO: 706 - DNA, 46 bp, synthetic construct
  misc_feature 1..46: note = Target Specific Oligonucleotide
  source 1..46: mol_type = other DNA
tgtatatggagtaccctcttgctgtaacttataaaggatagacatc

SEQ ID NO: 707 - DNA, 44 bp, synthetic construct
  misc_feature 1..44: note = Target Specific Oligonucleotide
  source 1..44: mol_type = other DNA
ctggatcaccaaaacggcaatgtaacttataaaggatagacatc

SEQ ID NO: 708 - DNA, 45 bp, synthetic construct
  misc_feature 1..45: note = Target Specific Oligonucleotide
  source 1..45: mol_type = other DNA
ccaggataacctttacttgccagtaacttataaaggatagacatc

SEQ ID NO: 709 - DNA, 46 bp, synthetic construct
  misc_feature 1..46: note = Target Specific Oligonucleotide
  source 1..46: mol_type = other DNA
atttccagctgcgatatctactcgtaacttataaaggatagacatc

SEQ ID NO: 710 - DNA, 47 bp, synthetic construct
  misc_feature 1..47: note = Target Specific Oligonucleotide
  source 1..47: mol_type = other DNA
tttatagcagctagtcctttcttggtaacttataaaggatagacatc

SEQ ID NO: 711 - DNA, 46 bp, synthetic construct
  misc_feature 1..46: note = Target Specific Oligonucleotide
  source 1..46: mol_type = other DNA
tgatatgagattttcccggatgggtaacttataaaggatagacatc

SEQ ID NO: 712 - DNA, 43 bp, synthetic construct
  misc_feature 1..43: note = Target Specific Oligonucleotide
  source 1..43: mol_type = other DNA
tgacaacagttagggcggtggtaacttataaaggatagacatc

SEQ ID NO: 713 - DNA, 44 bp, synthetic construct
  misc_feature 1..44: note = Target Specific Oligonucleotide
  source 1..44: mol_type = other DNA
ttggttcccgagtactgtctagtaacttataaaggatagacatc

SEQ ID NO: 714 - DNA, 45 bp, synthetic construct
  misc_feature 1..45: note = Target Specific Oligonucleotide
  source 1..45: mol_type = other DNA
gtttagttccaacgccatctgtgtaacttataaaggatagacatc

SEQ ID NO: 715 - DNA, 45 bp, synthetic construct
  misc_feature 1..45: note = Target Specific Oligonucleotide
  source 1..45: mol_type = other DNA
aagagttgcgacagtatcacccgtaacttataaaggatagacatc

SEQ ID NO: 716 - DNA, 44 bp, synthetic construct
  misc_feature 1..44: note = Target Specific Oligonucleotide
  source 1..44: mol_type = other DNA
gctgctggatatccctcagaagtaacttataaaggatagacatc

SEQ ID NO: 717 - DNA, 46 bp, synthetic construct
  misc_feature 1..46: note = Target Specific Oligonucleotide
  source 1..46: mol_type = other DNA
tgcaagacagactatgtctatgggtaacttataaaggatagacatc

SEQ ID NO: 718 - DNA, 46 bp, synthetic construct
  misc_feature 1..46: note = Target Specific Oligonucleotide
  source 1..46: mol_type = other DNA
cttcaaggactaggtcaattgcagtaacttataaaggatagacatc

SEQ ID NO: 719 - DNA, 47 bp, synthetic construct
  misc_feature 1..47: note = Target Specific Oligonucleotide
  source 1..47: mol_type = other DNA
gatatgctgcactaactagtcttggtaacttataaaggatagacatc

SEQ ID NO: 720 - DNA, 40 bp, synthetic construct
  misc_feature 1..40: note = Target Specific Oligonucleotide
  source 1..40: mol_type = other DNA
atctcgagcaagacgttcagtgtaacggttatcgtggaaa

SEQ ID NO: 721 - DNA, 43 bp, synthetic construct
  misc_feature 1..43: note = Target Specific Oligonucleotide
  source 1..43: mol_type = other DNA
ctgtccataattagtccatgaggagtaacggttatcgtggaaa

SEQ ID NO: 722 - DNA, 43 bp, synthetic construct
  misc_feature 1..43: note = Target Specific Oligonucleotide
  source 1..43: mol_type = other DNA
atctttggattatactgcctgaccgtaacggttatcgtggaaa

SEQ ID NO: 723 - DNA, 39 bp, synthetic construct
  misc_feature 1..39: note = Target Specific Oligonucleotide
  source 1..39: mol_type = other DNA
cagcaagcttgcgaccttgagtaacggttatcgtggaaa

SEQ ID NO: 724 - DNA, 44 bp, synthetic construct
  misc_feature 1..44: note = Target Specific Oligonucleotide
  source 1..44: mol_type = other DNA
agttaaagttgagagatcatctccagtaacggttatcgtggaaa

SEQ ID NO: 725 - DNA, 44 bp, synthetic construct
  misc_feature 1..44: note = Target Specific Oligonucleotide
  source 1..44: mol_type = other DNA
aggaatggatctatcactatttctagtaacggttatcgtggaaa

SEQ ID NO: 726 - DNA, 44 bp, synthetic construct
  misc_feature 1..44: note = Target Specific Oligonucleotide
  source 1..44: mol_type = other DNA
cagcataatgattaggtatgcaaaagtaacggttatcgtggaaa

SEQ ID NO: 727 - DNA, 44 bp, synthetic construct
  misc_feature 1..44: note = Target Specific Oligonucleotide
  source 1..44: mol_type = other DNA
ttcagtctgataaaatctacagtcagtaacggttatcgtggaaa

SEQ ID NO: 728 - DNA, 39 bp, synthetic construct
  misc_feature 1..39: note = Target Specific Oligonucleotide
  source 1..39: mol_type = other DNA
tccaacacttcgtggggtccgtaacggttatcgtggaaa

SEQ ID NO: 729 - DNA, 39 bp, synthetic construct
  misc_feature 1..39: note = Target Specific Oligonucleotide
  source 1..39: mol_type = other DNA
agggctacaatgtgatggccgtaacggttatcgtggaaa

SEQ ID NO: 730 - DNA, 42 bp, synthetic construct
  misc_feature 1..42: note = Target Specific Oligonucleotide
  source 1..42: mol_type = other DNA
tcaaggtcataacctggttcatcgtaacggttatcgtggaaa

SEQ ID NO: 731 - DNA, 42 bp, synthetic construct
  misc_feature 1..42: note = Target Specific Oligonucleotide
  source 1..42: mol_type = other DNA
cctacaacaaacttgtctggaatgtaacggttatcgtggaaa

SEQ ID NO: 732 - DNA, 40 bp, synthetic construct
  misc_feature 1..40: note = Target Specific Oligonucleotide
  source 1..40: mol_type = other DNA
aaacaacaatccgcccaaagggtaacggttatcgtggaaa

SEQ ID NO: 733 - DNA, 41 bp, synthetic construct
  misc_feature 1..41: note = Target Specific Oligonucleotide
  source 1..41: mol_type = other DNA
aaagctctactaagcagatggcgtaacggttatcgtggaaa

SEQ ID NO: 734 - DNA, 41 bp, synthetic construct
  misc_feature 1..41: note = Target Specific Oligonucleotide
  source 1..41: mol_type = other DNA
actgctgacaaagattcactgggtaacggttatcgtggaaa

SEQ ID NO: 735 - DNA, 44 bp, synthetic construct
  misc_feature 1..44: note = Target Specific Oligonucleotide
  source 1..44: mol_type = other DNA
ctgatagtctataggctcatagtgcgtaacggttatcgtggaaa

SEQ ID NO: 736 - DNA, 40 bp, synthetic construct
  misc_feature 1..40: note = Target Specific Oligonucleotide
  source 1..40: mol_type = other DNA
atcactaatcacgacgccagggtaacggttatcgtggaaa

SEQ ID NO: 737 - DNA, 40 bp, synthetic construct
  misc_feature 1..40: note = Target Specific Oligonucleotide
  source 1..40: mol_type = other DNA
tggcgatgtcaataggactccgtaacggttatcgtggaaa

SEQ ID NO: 738 - DNA, 42 bp, synthetic construct
  misc_feature 1..42: note = Target Specific Oligonucleotide
  source 1..42: mol_type = other DNA
gaactctcatcttaggctttgtagtaacggttatcgtggaaa

SEQ ID NO: 739 - DNA, 44 bp, synthetic construct
  misc_feature 1..44: note = Target Specific Oligonucleotide
  source 1..44: mol_type = other DNA
tcaacattactgaaacactactaaagtaacggttatcgtggaaa

SEQ ID NO: 740 - DNA, 38 bp, synthetic construct
  misc_feature 1..38: note = Target Specific Oligonucleotide
  source 1..38: mol_type = other DNA
ggtcgccataacggagccggtaacggttatcgtggaaa

SEQ ID NO: 741 - DNA, 45 bp, synthetic construct
  misc_feature 1..45: note = Target Specific Oligonucleotide
  source 1..45: mol_type = other DNA
ttcttacagatatgagttcaatgtttgtaacggttatcgtggaaa

SEQ ID NO: 742 - DNA, 44 bp, synthetic construct
  misc_feature 1..44: note = Target Specific Oligonucleotide
  source 1..44: mol_type = other DNA
aggacagaacaaaacttcttagatggtaacggttatcgtggaaa

SEQ ID NO: 743 - DNA, 36 bp, synthetic construct
  misc_feature 1..36: note = Target Specific Oligonucleotide
  source 1..36: mol_type = other DNA
tcgcagccgcctgaagcgtaacggttatcgtggaaa

SEQ ID NO: 744 - DNA, 41 bp, synthetic construct
  misc_feature 1..41: note = Target Specific Oligonucleotide
  source 1..41: mol_type = other DNA
ggaatttggaaccggcttgcgtaacggtactttatctagct

SEQ ID NO: 745 - DNA, 46 bp, synthetic construct
  misc_feature 1..46: note = Target Specific Oligonucleotide
  source 1..46: mol_type = other DNA
agagtcttgagtataatcttggtaggtaacggtactttatctagct

SEQ ID NO: 746 - DNA, 46 bp, synthetic construct
  misc_feature 1..46: note = Target Specific Oligonucleotide
  source 1..46: mol_type = other DNA
attcaggaagcatacactaattcttgtaacggtactttatctagct

SEQ ID NO: 747 - DNA, 44 bp, synthetic construct
  misc_feature 1..44: note = Target Specific Oligonucleotide
  source 1..44: mol_type = other DNA
tccagaaataagcgaaaatagcagtaacggtactttatctagct

SEQ ID NO: 748 - DNA, 47 bp, synthetic construct
  misc_feature 1..47: note = Target Specific Oligonucleotide
  source 1..47: mol_type = other DNA
atcttttgaactactagctacaaaatgtaacggtactttatctagct

SEQ ID NO: 749 - DNA, 42 bp, synthetic construct
  misc_feature 1..42: note = Target Specific Oligonucleotide
  source 1..42: mol_type = other DNA
taacaagctcgtaatggcccagtaacggtactttatctagct

SEQ ID NO: 750 - DNA, 42 bp, synthetic construct
  misc_feature 1..42: note = Target Specific Oligonucleotide
  source 1..42: mol_type = other DNA
catccaaaccgtgtgaaagctgtaacggtactttatctagct

SEQ ID NO: 751 - DNA, 41 bp, synthetic construct
  misc_feature 1..41: note = Target Specific Oligonucleotide
  source 1..41: mol_type = other DNA
acaacgccatgtgcgatttggtaacggtactttatctagct

SEQ ID NO: 752 - DNA, 45 bp, synthetic construct
  misc_feature 1..45: note = Target Specific Oligonucleotide
  source 1..45: mol_type = other DNA
ctacctaccactaggtacctatcagtaacggtactttatctagct

SEQ ID NO: 753 - DNA, 43 bp, synthetic construct
  misc_feature 1..43: note = Target Specific Oligonucleotide
  source 1..43: mol_type = other DNA
aggacatttacgtgtacagcacgtaacggtactttatctagct

SEQ ID NO: 754 - DNA, 43 bp, synthetic construct
  misc_feature 1..43: note = Target Specific Oligonucleotide
  source 1..43: mol_type = other DNA
cgcctgaatacaacgagttaacgtaacggtactttatctagct

SEQ ID NO: 755 - DNA, 44 bp, synthetic construct
  misc_feature 1..44: note = Target Specific Oligonucleotide
  source 1..44: mol_type = other DNA
cttccagattgtcgccgttaattgtaacggtactttatctagct

SEQ ID NO: 756 - DNA, 44 bp, synthetic construct
  misc_feature 1..44: note = Target Specific Oligonucleotide
  source 1..44: mol_type = other DNA
cagatttacctaaaccaccaccagtaacggtactttatctagct

SEQ ID NO: 757 - DNA, 45 bp, synthetic construct
  misc_feature 1..45: note = Target Specific Oligonucleotide
  source 1..45: mol_type = other DNA
tttgagctgatctagtaggtcttcgtaacggtactttatctagct

SEQ ID NO: 758 - DNA, 41 bp, synthetic construct
  misc_feature 1..41: note = Target Specific Oligonucleotide
  source 1..41: mol_type = other DNA
tctgtagctcgatccctggagtaacggtactttatctagct

SEQ ID NO: 759 - DNA, 44 bp, synthetic construct
  misc_feature 1..44: note = Target Specific Oligonucleotide
  source 1..44: mol_type = other DNA
caactgtcattcggttaaactgagtaacggtactttatctagct

SEQ ID NO: 760 - DNA, 44 bp, synthetic construct
  misc_feature 1..44: note = Target Specific Oligonucleotide
  source 1..44: mol_type = other DNA
tttgcttccgttcatcattagtcgtaacggtactttatctagct

SEQ ID NO: 761 - DNA, 45 bp, synthetic construct
  misc_feature 1..45: note = Target Specific Oligonucleotide
  source 1..45: mol_type = other DNA
acttccaatagtctggaaatcacagtaacggtactttatctagct

SEQ ID NO: 762 - DNA, 45 bp, synthetic construct
  misc_feature 1..45: note = Target Specific Oligonucleotide
  source 1..45: mol_type = other DNA
tcatctgctggattaagctaatacgtaacggtactttatctagct

SEQ ID NO: 763 - DNA, 41 bp, synthetic construct
  misc_feature 1..41: note = Target Specific Oligonucleotide
  source 1..41: mol_type = other DNA
agataggctcccgtatgcccgtaacggtactttatctagct

SEQ ID NO: 764 - DNA, 41 bp, synthetic construct
  misc_feature 1..41: note = Target Specific Oligonucleotide
  source 1..41: mol_type = other DNA
gcttctcggctaccacagacgtaacggtactttatctagct

SEQ ID NO: 765 - DNA, 46 bp, synthetic construct
  misc_feature 1..46: note = Target Specific Oligonucleotide
  source 1..46: mol_type = other DNA
agacttactcttaagaccatacttcgtaacggtactttatctagct

SEQ ID NO: 766 - DNA, 42 bp, synthetic construct
  misc_feature 1..42: note = Target Specific Oligonucleotide
  source 1..42: mol_type = other DNA
gttgagaggtggcgtttttgagtaacggtactttatctagct

SEQ ID NO: 767 - DNA, 44 bp, synthetic construct
  misc_feature 1..44: note = Target Specific Oligonucleotide
  source 1..44: mol_type = other DNA
tcaatacgtttctgcaagagtttgtaacggtactttatctagct

SEQ ID NO: 768 - DNA, 41 bp, synthetic construct
  misc_feature 1..41: note = Target Specific Oligonucleotide
  source 1..41: mol_type = other DNA
ttatggcctctatagcatctcccgtaactccatctagaccg

SEQ ID NO: 769 - DNA, 40 bp, synthetic construct
  misc_feature 1..40: note = Target Specific Oligonucleotide
  source 1..40: mol_type = other DNA
cagtccgggcaactatcttattgtaactccatctagaccg

SEQ ID NO: 770 - DNA, 42 bp, synthetic construct
  misc_feature 1..42: note = Target Specific Oligonucleotide
  source 1..42: mol_type = other DNA
ttcaagatacgaataatcctccgagtaactccatctagaccg

SEQ ID NO: 771 - DNA, 40 bp, synthetic construct
  misc_feature 1..40: note = Target Specific Oligonucleotide
  source 1..40: mol_type = other DNA
gtaggcgcttagcttgattttcgtaactccatctagaccg

SEQ ID NO: 772 - DNA, 38 bp, synthetic construct
  misc_feature 1..38: note = Target Specific Oligonucleotide
  source 1..38: mol_type = other DNA
cttcaagtcgggctcttgcagtaactccatctagaccg

SEQ ID NO: 773 - DNA, 38 bp, synthetic construct
  misc_feature 1..38: note = Target Specific Oligonucleotide
  source 1..38: mol_type = other DNA
agaatgaggcacgcaaagctgtaactccatctagaccg

SEQ ID NO: 774 - DNA, 40 bp, synthetic construct
  misc_feature 1..40: note = Target Specific Oligonucleotide
  source 1..40: mol_type = other DNA
ctcagcatccgataggactttcgtaactccatctagaccg

SEQ ID NO: 775 - DNA, 40 bp, synthetic construct
  misc_feature 1..40: note = Target Specific Oligonucleotide
  source 1..40: mol_type = other DNA
aagtcactataacacccgtcctgtaactccatctagaccg

SEQ ID NO: 776 - DNA, 39 bp, synthetic construct
  misc_feature 1..39: note = Target Specific Oligonucleotide
  source 1..39: mol_type = other DNA
ttggcatggtagatcgtccaggtaactccatctagaccg

SEQ ID NO: 777 - DNA, 39 bp, synthetic construct
  misc_feature 1..39: note = Target Specific Oligonucleotide
  source 1..39: mol_type = other DNA
caccttccaacgactcaatccgtaactccatctagaccg

SEQ ID NO: 778 - DNA, 42 bp, synthetic construct
  misc_feature 1..42: note = Target Specific Oligonucleotide
  source 1..42: mol_type = other DNA
acaacctgtaagtgtagttctctggtaactccatctagaccg

SEQ ID NO: 779 - DNA, 43 bp, synthetic construct
  misc_feature 1..43: note = Target Specific Oligonucleotide
  source 1..43: mol_type = other DNA
aaatcagatactcgtctacagaatggtaactccatctagaccg

SEQ ID NO: 780 - DNA, 38 bp, synthetic construct
  misc_feature 1..38: note = Target Specific Oligonucleotide
  source 1..38: mol_type = other DNA
agcagcaagtcgcattttccgtaactccatctagaccg

SEQ ID NO: 781 - DNA, 39 bp, synthetic construct
  misc_feature 1..39: note = Target Specific Oligonucleotide
  source 1..39: mol_type = other DNA
actggcatggcggataaaaaggtaactccatctagaccg

SEQ ID NO: 782 - DNA, 38 bp, synthetic construct
  misc_feature 1..38: note = Target Specific Oligonucleotide
  source 1..38: mol_type = other DNA
cgggtgctctcgtgaacaaagtaactccatctagaccg

SEQ ID NO: 783 - DNA, 41 bp, synthetic construct
  misc_feature 1..41: note = Target Specific Oligonucleotide
  source 1..41: mol_type = other DNA
gatcgaagagtcgagataaggatgtaactccatctagaccg

SEQ ID NO: 784 - DNA, 41 bp, synthetic construct
  misc_feature 1..41: note = Target Specific Oligonucleotide
  source 1..41: mol_type = other DNA
ttgttgaagacgcttccataagtgtaactccatctagaccg

SEQ ID NO: 785 - DNA, 37 bp, synthetic construct
  misc_feature 1..37: note = Target Specific Oligonucleotide
  source 1..37: mol_type = other DNA
gtggtgacgcagaatcccggtaactccatctagaccg

SEQ ID NO: 786 - DNA, 45 bp, synthetic construct
  misc_feature 1..45: note = Target Specific Oligonucleotide
  source 1..45: mol_type = other DNA
cattataaagacgtaataatttagggtgtaactccatctagaccg

SEQ ID NO: 787 - DNA, 39 bp, synthetic construct
  misc_feature 1..39: note = Target Specific Oligonucleotide
  source 1..39: mol_type = other DNA
gctcccactcctagacatgttgtaactccatctagaccg

SEQ ID NO: 788 - DNA, 40 bp, synthetic construct
  misc_feature 1..40: note = Target Specific Oligonucleotide
  source 1..40: mol_type = other DNA
tttgttacacggttaaacagccgtaactccatctagaccg

SEQ ID NO: 789 - DNA, 42 bp, synthetic construct
  misc_feature 1..42: note = Target Specific Oligonucleotide
  source 1..42: mol_type = other DNA
gaggtaaataaacgtcgataggaagtaactccatctagaccg

SEQ ID NO: 790 - DNA, 40 bp, synthetic construct
  misc_feature 1..40: note = Target Specific Oligonucleotide
  source 1..40: mol_type = other DNA
ttaatgtggagtgcaagttggggtaactccatctagaccg

SEQ ID NO: 791 - DNA, 41 bp, synthetic construct
  misc_feature 1..41: note = Target Specific Oligonucleotide
  source 1..41: mol_type = other DNA
ccttgtatcttagcttgggatgtgtaactccatctagaccg

SEQ ID NO: 792 - DNA, 43 bp, synthetic construct
  misc_feature 1..43: note = Target Specific Oligonucleotide
  source 1..43: mol_type = other DNA
tcaatgatcagcggatacctattgtaactcagtagatatagcg

SEQ ID NO: 793 - DNA, 43 bp, synthetic construct
  misc_feature 1..43: note = Target Specific Oligonucleotide
  source 1..43: mol_type = other DNA
cgtgtgatcttacgatccttatagtaactcagtagatatagcg

SEQ ID NO: 794 - DNA, 43 bp, synthetic construct
  misc_feature 1..43: note = Target Specific Oligonucleotide
  source 1..43: mol_type = other DNA
tcatcctctacgagtctatcttggtaactcagtagatatagcg

SEQ ID NO: 795 - DNA, 40 bp, synthetic construct
  misc_feature 1..40: note = Target Specific Oligonucleotide
  source 1..40: mol_type = other DNA
tcaaagtaacccgcgtaggcgtaactcagtagatatagcg

SEQ ID NO: 796 - DNA, 41 bp, synthetic construct
  misc_feature 1..41: note = Target Specific Oligonucleotide
  source 1..41: mol_type = other DNA
ataggacgcatactgtcgcaagtaactcagtagatatagcg

SEQ ID NO: 797 - DNA, 41 bp, synthetic construct
  misc_feature 1..41: note = Target Specific Oligonucleotide
  source 1..41: mol_type = other DNA
ttatgtccgtcgaccttgcatgtaactcagtagatatagcg

SEQ ID NO: 798 - DNA, 42 bp, synthetic construct
  misc_feature 1..42: note = Target Specific Oligonucleotide
  source 1..42: mol_type = other DNA
ttccaaggaacggacttctagggtaactcagtagatatagcg

SEQ ID NO: 799 - DNA, 42 bp, synthetic construct
  misc_feature 1..42: note = Target Specific Oligonucleotide
  source 1..42: mol_type = other DNA
ataggtacgaacgctctcgatcgtaactcagtagatatagcg

SEQ ID NO: 800 - DNA, 42 bp, synthetic construct
  misc_feature 1..42: note = Target Specific Oligonucleotide
  source 1..42: mol_type = other DNA
tcttggatgatcgcatgaaaccgtaactcagtagatatagcg

SEQ ID NO: 801 - DNA, 42 bp, synthetic construct
  misc_feature 1..42: note = Target Specific Oligonucleotide
  source 1..42: mol_type = other DNA
acaacccaattaacgtgaagccgtaactcagtagatatagcg

SEQ ID NO: 802 - DNA, 41 bp, synthetic construct
  misc_feature 1..41: note = Target Specific Oligonucleotide
  source 1..41: mol_type = other DNA
atgcggtataacgcacgttccgtaactcagtagatatagcg

SEQ ID NO: 803 - DNA, 41 bp, synthetic construct
  misc_feature 1..41: note = Target Specific Oligonucleotide
  source 1..41: mol_type = other DNA
ctcaagtcacgacgcagttctgtaactcagtagatatagcg

SEQ ID NO: 804 - DNA, 40 bp, synthetic construct
  misc_feature 1..40: note = Target Specific Oligonucleotide
  source 1..40: mol_type = other DNA
gcaagtcacgaacgtgactcgtaactcagtagatatagcg

SEQ ID NO: 805 - DNA, 40 bp, synthetic construct
  misc_feature 1..40: note = Target Specific Oligonucleotide
  source 1..40: mol_type = other DNA
ttggcgttatactgcgccacgtaactcagtagatatagcg

SEQ ID NO: 806 - DNA, 40 bp, synthetic construct
  misc_feature 1..40: note = Target Specific Oligonucleotide
  source 1..40: mol_type = other DNA
agtggtgcgtatcgtaagcggtaactcagtagatatagcg

SEQ ID NO: 807 - DNA, 40 bp, synthetic construct
  misc_feature 1..40: note = Target Specific Oligonucleotide
  source 1..40: mol_type = other DNA
atccaggcgacgaaacgagagtaactcagtagatatagcg

SEQ ID NO: 808 - DNA, 40 bp, synthetic construct
  misc_feature 1..40: note = Target Specific Oligonucleotide
  source 1..40: mol_type = other DNA
ttggatgaatcggcaggctggtaactcagtagatatagcg

SEQ ID NO: 809 - DNA, 43 bp, synthetic construct
  misc_feature 1..43: note = Target Specific Oligonucleotide
  source 1..43: mol_type = other DNA
tcagtcaattcgtaatgtacaccgtaactcagtagatatagcg

SEQ ID NO: 810 - DNA, 41 bp, synthetic construct
  misc_feature 1..41: note = Target Specific Oligonucleotide
  source 1..41: mol_type = other DNA
catcgaagacgatccactggcgtaactcagtagatatagcg

SEQ ID NO: 811 - DNA, 39 bp, synthetic construct
  misc_feature 1..39: note = Target Specific Oligonucleotide
  source 1..39: mol_type = other DNA
cacggatcaagcggcacttgtaactcagtagatatagcg

SEQ ID NO: 812 - DNA, 39 bp, synthetic construct
  misc_feature 1..39: note = Target Specific Oligonucleotide
  source 1..39: mol_type = other DNA
tccaccgtatcgcaagctggtaactcagtagatatagcg

SEQ ID NO: 813 - DNA, 41 bp, synthetic construct
  misc_feature 1..41: note = Target Specific Oligonucleotide
  source 1..41: mol_type = other DNA
atgcaaagtttcgtagggcgagtaactcagtagatatagcg

SEQ ID NO: 814 - DNA, 38 bp, synthetic construct
  misc_feature 1..38: note = Target Specific Oligonucleotide
  source 1..38: mol_type = other DNA
gcgttggcacgacgacatgtaactcagtagatatagcg

SEQ ID NO: 815 - DNA, 38 bp, synthetic construct
  misc_feature 1..38: note = Target Specific Oligonucleotide
  source 1..38: mol_type = other DNA
ttgcagacggacgcccaagtaactcagtagatatagcg

SEQ ID NO: 816 - DNA, 40 bp, synthetic construct
  misc_feature 1..40: note = Target Specific Oligonucleotide
  source 1..40: mol_type = other DNA
agctgtatcgtcaaggcactcgtaaccttttgaaacgcta

SEQ ID NO: 817 - DNA, 39 bp, synthetic construct
  misc_feature 1..39: note = Target Specific Oligonucleotide
  source 1..39: mol_type = other DNA
ctcgctcccagtccgaaatggtaaccttttgaaacgcta

SEQ ID NO: 818 - DNA, 44 bp, synthetic construct
  misc_feature 1..44: note = Target Specific Oligonucleotide
  source 1..44: mol_type = other DNA
acttgtactagtatgccttaagaaagtaaccttttgaaacgcta

SEQ ID NO: 819 - DNA, 42 bp, synthetic construct
  misc_feature 1..42: note = Target Specific Oligonucleotide
  source 1..42: mol_type = other DNA
gtgaccatgactaatagcagtgggtaaccttttgaaacgcta

SEQ ID NO: 820 - DNA, 41 bp, synthetic construct
  misc_feature 1..41: note = Target Specific Oligonucleotide
  source 1..41: mol_type = other DNA
gctgtgtcgagaatatccaagagtaaccttttgaaacgcta

SEQ ID NO: 821 - DNA, 41 bp, synthetic construct
  misc_feature 1..41: note = Target Specific Oligonucleotide
  source 1..41: mol_type = other DNA
cctactgtcgctaatggattgggtaaccttttgaaacgcta

SEQ ID NO: 822 - DNA, 41 bp, synthetic construct
  misc_feature 1..41: note = Target Specific Oligonucleotide
  source 1..41: mol_type = other DNA
acactagcactacctaaggaccgtaaccttttgaaacgcta

SEQ ID NO: 823 - DNA, 41 bp, synthetic construct
  misc_feature 1..41: note = Target Specific Oligonucleotide
  source 1..41: mol_type = other DNA
gtctgtgaactagttcaggcacgtaaccttttgaaacgcta

SEQ ID NO: 824 - DNA, 40 bp, synthetic construct
  misc_feature 1..40: note = Target Specific Oligonucleotide
  source 1..40: mol_type = other DNA
ctaggtcagcgcaaccaaatggtaaccttttgaaacgcta

SEQ ID NO: 825 - DNA, 42 bp, synthetic construct
  misc_feature 1..42: note = Target Specific Oligonucleotide
  source 1..42: mol_type = other DNA
cctaataagctataactggcccagtaaccttttgaaacgcta

SEQ ID NO: 826 - DNA, 43 bp, synthetic construct
  misc_feature 1..43: note = Target Specific Oligonucleotide
  source 1..43: mol_type = other DNA
ctaaattcctatgcagtgtgactcgtaaccttttgaaacgcta

SEQ ID NO: 827 - DNA, 42 bp, synthetic construct
  misc_feature 1..42: note = Target Specific Oligonucleotide
  source 1..42: mol_type = other DNA
atcttgttgagctatccaaactggtaaccttttgaaacgcta

SEQ ID NO: 828 - DNA, 42 bp, synthetic construct
  misc_feature 1..42: note = Target Specific Oligonucleotide
  source 1..42: mol_type = other DNA
aaatacgcatcgtgttatctctggtaaccttttgaaacgcta

SEQ ID NO: 829 - DNA, 42 bp, synthetic construct
  misc_feature 1..42: note = Target Specific Oligonucleotide
  source 1..42: mol_type = other DNA
tgttaagagaactagccaaacctgtaaccttttgaaacgcta

SEQ ID NO: 830 - DNA, 43 bp, synthetic construct
  misc_feature 1..43: note = Target Specific Oligonucleotide
  source 1..43: mol_type = other DNA
cataaagtagcttgatcgaagagtgtaaccttttgaaacgcta

SEQ ID NO: 831 - DNA, 41 bp, synthetic construct
  misc_feature 1..41: note = Target Specific Oligonucleotide
  source 1..41: mol_type = other DNA
taagcaaacacgcctttacatagtaaccttttgaaacgcta

SEQ ID NO: 832 - DNA, 44 bp, synthetic construct
  misc_feature 1..44: note = Target Specific Oligonucleotide
  source 1..44: mol_type = other DNA
aaggccttagtaagatattacagacgtaaccttttgaaacgcta

SEQ ID NO: 833 - DNA, 45 bp, synthetic construct
  misc_feature 1..45: note = Target Specific Oligonucleotide
  source 1..45: mol_type = other DNA
acaatatacgtctgctatattcttccgtaaccttttgaaacgcta

SEQ ID NO: 834 - DNA, 41 bp, synthetic construct
  misc_feature 1..41: note = Target Specific Oligonucleotide
  source 1..41: mol_type = other DNA
tccactggatagggttctgtctgtaaccttttgaaacgcta

SEQ ID NO: 835 - DNA, 44 bp, synthetic construct
  misc_feature 1..44: note = Target Specific Oligonucleotide
  source 1..44: mol_type = other DNA
aagttatactatgaaagagcagtctgtaaccttttgaaacgcta

SEQ ID NO: 836 - DNA, 44 bp, synthetic construct
  misc_feature 1..44: note = Target Specific Oligonucleotide
  source 1..44: mol_type = other DNA
acatgttaatgcctaagtctatgtagtaaccttttgaaacgcta

SEQ ID NO: 837 - DNA, 40 bp, synthetic construct
  misc_feature 1..40: note = Target Specific Oligonucleotide
  source 1..40: mol_type = other DNA
gcctagaatgcctacttgggagtaaccttttgaaacgcta

SEQ ID NO: 838 - DNA, 41 bp, synthetic construct
  misc_feature 1..41: note = Target Specific Oligonucleotide
  source 1..41: mol_type = other DNA
tcagtggaatcgtagcaaaacagtaaccttttgaaacgcta

SEQ ID NO: 839 - DNA, 45 bp, synthetic construct
  misc_feature 1..45: note = Target Specific Oligonucleotide
  source 1..45: mol_type = other DNA
acaataattaggagtagtacagttcagtaaccttttgaaacgcta

SEQ ID NO: 840 - DNA, 42 bp, synthetic construct
  misc_feature 1..42: note = Target Specific Oligonucleotide
  source 1..42: mol_type = other DNA
ttccactcggataagatgctgagtaactcagacatgtagatt

SEQ ID NO: 841 - DNA, 42 bp, synthetic construct
  misc_feature 1..42: note = Target Specific Oligonucleotide
  source 1..42: mol_type = other DNA
aatactccacacgcaaatttccgtaactcagacatgtagatt

SEQ ID NO: 842 - DNA, 40 bp, synthetic construct
  misc_feature 1..40: note = Target Specific Oligonucleotide
  source 1..40: mol_type = other DNA
ggccagaccatcgctatctggtaactcagacatgtagatt

SEQ ID NO: 843 - DNA, 42 bp, synthetic construct
  misc_feature 1..42: note = Target Specific Oligonucleotide
  source 1..42: mol_type = other DNA
caccacactatgtcgaaaagtggtaactcagacatgtagatt

SEQ ID NO: 844 - DNA, 42 bp, synthetic construct
  misc_feature 1..42: note = Target Specific Oligonucleotide
  source 1..42: mol_type = other DNA
ccctttcttgcggagattctctgtaactcagacatgtagatt

SEQ ID NO: 845 - DNA, 40 bp, synthetic construct
  misc_feature 1..40: note = Target Specific Oligonucleotide
  source 1..40: mol_type = other DNA
acaaacacgcacctcaaagcgtaactcagacatgtagatt

SEQ ID NO: 846 - DNA, 42 bp, synthetic construct
  misc_feature 1..42: note = Target Specific Oligonucleotide
  source 1..42: mol_type = other DNA
cccagtagattaccactggagtgtaactcagacatgtagatt

SEQ ID NO: 847 - DNA, 39 bp, synthetic construct
  misc_feature 1..39: note = Target Specific Oligonucleotide
  source 1..39: mol_type = other DNA
gcagtgctcgcttagtgctgtaactcagacatgtagatt

SEQ ID NO: 848 - DNA, 40 bp, synthetic construct
  misc_feature 1..40: note = Target Specific Oligonucleotide
  source 1..40: mol_type = other DNA
ggctcgacgctaggatctgagtaactcagacatgtagatt

SEQ ID NO: 849 - DNA, 39 bp, synthetic construct
  misc_feature 1..39: note = Target Specific Oligonucleotide
  source 1..39: mol_type = other DNA
aggatgggcctccggttcagtaactcagacatgtagatt

SEQ ID NO: 850 - DNA, 40 bp, synthetic construct
  misc_feature 1..40: note = Target Specific Oligonucleotide
  source 1..40: mol_type = other DNA
ggaacatctcgaagcgctcagtaactcagacatgtagatt

SEQ ID NO: 851 - DNA, 40 bp, synthetic construct
  misc_feature 1..40: note = Target Specific Oligonucleotide
  source 1..40: mol_type = other DNA
agacggaaaccgtagctgccgtaactcagacatgtagatt

SEQ ID NO: 852 - DNA, 41 bp, synthetic construct
  misc_feature 1..41: note = Target Specific Oligonucleotide
  source 1..41: mol_type = other DNA
tgttcaatatcgtccggggacgtaactcagacatgtagatt

SEQ ID NO: 853 - DNA, 40 bp, synthetic construct
  misc_feature 1..40: note = Target Specific Oligonucleotide
  source 1..40: mol_type = other DNA
cattgcttgggacggcaagggtaactcagacatgtagatt

SEQ ID NO: 854 - DNA, 42 bp, synthetic construct
  misc_feature 1..42: note = Target Specific Oligonucleotide
  source 1..42: mol_type = other DNA
agtggagaatgtcagtctgagtgtaactcagacatgtagatt

SEQ ID NO: 855 - DNA, 43 bp, synthetic construct
  misc_feature 1..43: note = Target Specific Oligonucleotide
  source 1..43: mol_type = other DNA
agttttttatggcgggaggtagagtaactcagacatgtagatt

SEQ ID NO: 856 - DNA, 41 bp, synthetic construct
  misc_feature 1..41: note = Target Specific Oligonucleotide
  source 1..41: mol_type = other DNA
tagaaactaccaacccaccgagtaactcagacatgtagatt

SEQ ID NO: 857 - DNA, 42 bp, synthetic construct
  misc_feature 1..42: note = Target Specific Oligonucleotide
  source 1..42: mol_type = other DNA
ttccctggttagtacggtgaaggtaactcagacatgtagatt

SEQ ID NO: 858 - DNA, 42 bp, synthetic construct
  misc_feature 1..42: note = Target Specific Oligonucleotide
  source 1..42: mol_type = other DNA
taagctggtatgtcctactcccgtaactcagacatgtagatt

SEQ ID NO: 859 - DNA, 41 bp, synthetic construct
  misc_feature 1..41: note = Target Specific Oligonucleotide
  source 1..41: mol_type = other DNA
ctgacgcacacctattgcaaggtaactcagacatgtagatt

SEQ ID NO: 860 - DNA, 39 bp, synthetic construct
  misc_feature 1..39: note = Target Specific Oligonucleotide
  source 1..39: mol_type = other DNA
tcaccgtcgtggaaagcacgtaactcagacatgtagatt

SEQ ID NO: 861 - DNA, 44 bp, synthetic construct
  misc_feature 1..44: note = Target Specific Oligonucleotide
  source 1..44: mol_type = other DNA
gtaaactaacccttaactgcaagagtaactcagacatgtagatt

SEQ ID NO: 862 - DNA, 44 bp, synthetic construct
  misc_feature 1..44: note = Target Specific Oligonucleotide
  source 1..44: mol_type = other DNA
tttaggtactaaggttcaccaagagtaactcagacatgtagatt

SEQ ID NO: 863 - DNA, 46 bp, synthetic construct
  misc_feature 1..46: note = Target Specific Oligonucleotide
  source 1..46: mol_type = other DNA
tcatcatatacaagagatgaaatcctgtaactcagacatgtagatt

SEQ ID NO: 864 - DNA, 41 bp, synthetic construct
  misc_feature 1..41: note = Target Specific Oligonucleotide
  source 1..41: mol_type = other DNA
ccatggtgacgatcctcacggtaactaacataaattcgatg

SEQ ID NO: 865 - DNA, 42 bp, synthetic construct
  misc_feature 1..42: note = Target Specific Oligonucleotide
  source 1..42: mol_type = other DNA
gtgaacgtcttgggttgcttcgtaactaacataaattcgatg

SEQ ID NO: 866 - DNA, 39 bp, synthetic construct
  misc_feature 1..39: note = Target Specific Oligonucleotide
  source 1..39: mol_type = other DNA
ggcctggacggcgtaagagtaactaacataaattcgatg

SEQ ID NO: 867 - DNA, 40 bp, synthetic construct
  misc_feature 1..40: note = Target Specific Oligonucleotide
  source 1..40: mol_type = other DNA
gaagctcatgcgggaagcggtaactaacataaattcgatg

SEQ ID NO: 868 - DNA, 43 bp, synthetic construct
  misc_feature 1..43: note = Target Specific Oligonucleotide
  source 1..43: mol_type = other DNA
tgtcactgtacgagatgtttcggtaactaacataaattcgatg

SEQ ID NO: 869 - DNA, 43 bp, synthetic construct
  misc_feature 1..43: note = Target Specific Oligonucleotide
  source 1..43: mol_type = other DNA
ttgaagcttggtatgtcaggaggtaactaacataaattcgatg

SEQ ID NO: 870 - DNA, 42 bp, synthetic construct
  misc_feature 1..42: note = Target Specific Oligonucleotide
  source 1..42: mol_type = other DNA
ggttcccgatacatagctggagtaactaacataaattcgatg

SEQ ID NO: 871 - DNA, 44 bp, synthetic construct
  misc_feature 1..44: note = Target Specific Oligonucleotide
  source 1..44: mol_type = other DNA
atctttgaagtcgaaagacaggcgtaactaacataaattcgatg

SEQ ID NO: 872 - DNA, 44 bp, synthetic construct
  misc_feature 1..44: note = Target Specific Oligonucleotide
  source 1..44: mol_type = other DNA
gcttattaacacgaagctttgaggtaactaacataaattcgatg

SEQ ID NO: 873 - DNA, 42 bp, synthetic construct
  misc_feature 1..42: note = Target Specific Oligonucleotide
  source 1..42: mol_type = other DNA
tttcattccacgggaaggagagtaactaacataaattcgatg

SEQ ID NO: 874 - DNA, 41 bp, synthetic construct
  misc_feature 1..41: note = Target Specific Oligonucleotide
  source 1..41: mol_type = other DNA
tcagtgcttcgttggccattgtaactaacataaattcgatg

SEQ ID NO: 875 - DNA, 43 bp, synthetic construct
  misc_feature 1..43: note = Target Specific Oligonucleotide
  source 1..43: mol_type = other DNA
ctctgcgtaccaagcagtaattgtaactaacataaattcgatg

SEQ ID NO: 876 - DNA, 43 bp, synthetic construct
  misc_feature 1..43: note = Target Specific Oligonucleotide
  source 1..43: mol_type = other DNA
tttcaaggcctcgatttctgtcgtaactaacataaattcgatg

SEQ ID NO: 877 - DNA, 43 bp, synthetic construct
  misc_feature 1..43: note = Target Specific Oligonucleotide
  source 1..43: mol_type = other DNA
tagttcacaccgtacatctccagtaactaacataaattcgatg

SEQ ID NO: 878 - DNA, 42 bp, synthetic construct
  misc_feature 1..42: note = Target Specific Oligonucleotide
  source 1..42: mol_type = other DNA
cccacatttccggagtcatctgtaactaacataaattcgatg

SEQ ID NO: 879 - DNA, 45 bp, synthetic construct
  misc_feature 1..45: note = Target Specific Oligonucleotide
  source 1..45: mol_type = other DNA
ggtcctgagctatcttcagatattgtaactaacataaattcgatg

SEQ ID NO: 880 - DNA, 39 bp, synthetic construct
  misc_feature 1..39: note = Target Specific Oligonucleotide
  source 1..39: mol_type = other DNA
tcctccgtgcgaatcgctgtaactaacataaattcgatg

SEQ ID NO: 881 - DNA, 43 bp, synthetic construct
  misc_feature 1..43: note = Target Specific Oligonucleotide
  source 1..43: mol_type = other DNA
gccctttttattccggattgcagtaactaacataaattcgatg

SEQ ID NO: 882 - DNA, 40 bp, synthetic construct
  misc_feature 1..40: note = Target Specific Oligonucleotide
  source 1..40: mol_type = other DNA
gctgtctcctcagaccgcagtaactaacataaattcgatg

SEQ ID NO: 883 - DNA, 41 bp, synthetic construct
  misc_feature 1..41: note = Target Specific Oligonucleotide
  source 1..41: mol_type = other DNA
cacccctgtcggagttctcagtaactaacataaattcgatg

SEQ ID NO: 884 - DNA, 46 bp, synthetic construct
  misc_feature 1..46: note = Target Specific Oligonucleotide
  source 1..46: mol_type = other DNA
cagatttattaccctttttggaagcgtaactaacataaattcgatg

SEQ ID NO: 885 - DNA, 39 bp, synthetic construct
  misc_feature 1..39: note = Target Specific Oligonucleotide
  source 1..39: mol_type = other DNA
tcatgggcgggtacgtgggtaactaacataaattcgatg

SEQ ID NO: 886 - DNA, 42 bp, synthetic construct
  misc_feature 1..42: note = Target Specific Oligonucleotide
  source 1..42: mol_type = other DNA
caaaaatccccgcttgtgaacgtaactaacataaattcgatg

SEQ ID NO: 887 - DNA, 42 bp, synthetic construct
  misc_feature 1..42: note = Target Specific Oligonucleotide
  source 1..42: mol_type = other DNA
ctggggtcgtagtcaccatacgtaactaacataaattcgatg

SEQ ID NO: 888 - DNA, 39 bp, synthetic construct
  misc_feature 1..39: note = Target Specific Oligonucleotide
  source 1..39: mol_type = other DNA
cacacgataccggcaaagaaggtaacgtgacgattaccc

SEQ ID NO: 889 - DNA, 38 bp, synthetic construct
  misc_feature 1..38: note = Target Specific Oligonucleotide
  source 1..38: mol_type = other DNA
ggtgtcagtctccgacgtgagtaacgtgacgattaccc

SEQ ID NO: 890 - DNA, 39 bp, synthetic construct
  misc_feature 1..39: note = Target Specific Oligonucleotide
  source 1..39: mol_type = other DNA
gtgatggtgatcatctgggccgtaacgtgacgattaccc

SEQ ID NO: 891 - DNA, 36 bp, synthetic construct
  misc_feature 1..36: note = Target Specific Oligonucleotide
  source 1..36: mol_type = other DNA
ttggcctcgggaccaagcgtaacgtgacgattaccc

SEQ ID NO: 892 - DNA, 39 bp, synthetic construct
  misc_feature 1..39: note = Target Specific Oligonucleotide
  source 1..39: mol_type = other DNA
ctgtcatcttggtcaggtggtgtaacgtgacgattaccc

SEQ ID NO: 893 - DNA, 38 bp, synthetic construct
  misc_feature 1..38: note = Target Specific Oligonucleotide
  source 1..38: mol_type = other DNA
atcaccttgccgaaagtgccgtaacgtgacgattaccc

SEQ ID NO: 894 - DNA, 37 bp, synthetic construct
  misc_feature 1..37: note = Target Specific Oligonucleotide
  source 1..37: mol_type = other DNA
actgcacggccgtagtcatgtaacgtgacgattaccc

SEQ ID NO: 895 - DNA, 37 bp, synthetic construct
  misc_feature 1..37: note = Target Specific Oligonucleotide
  source 1..37: mol_type = other DNA
aggtactcaggtgtgccgcgtaacgtgacgattaccc

SEQ ID NO: 896 - DNA, 38 bp, synthetic construct
  misc_feature 1..38: note = Target Specific Oligonucleotide
  source 1..38: mol_type = other DNA
gaaggtgcgttcgatgacaggtaacgtgacgattaccc

SEQ ID NO: 897 - DNA, 39 bp, synthetic construct
  misc_feature 1..39: note = Target Specific Oligonucleotide
  source 1..39: mol_type = other DNA
ctcctcaggagtctccacatggtaacgtgacgattaccc

SEQ ID NO: 898 - DNA, 40 bp, synthetic construct
  misc_feature 1..40: note = Target Specific Oligonucleotide
  source 1..40: mol_type = other DNA
gtctggaaagagtacttcaggggtaacgtgacgattaccc

SEQ ID NO: 899 - DNA, 36 bp, synthetic construct
  misc_feature 1..36: note = Target Specific Oligonucleotide
  source 1..36: mol_type = other DNA
caggacgcggttctcggtgtaacgtgacgattaccc

SEQ ID NO: 900 - DNA, 38 bp, synthetic construct
  misc_feature 1..38: note = Target Specific Oligonucleotide
  source 1..38: mol_type = other DNA
atctcagcgccatagaagcggtaacgtgacgattaccc

SEQ ID NO: 901 - DNA, 37 bp, synthetic construct
  misc_feature 1..37: note = Target Specific Oligonucleotide
  source 1..37: mol_type = other DNA
tcgttcatggtcacgcggtgtaacgtgacgattaccc

SEQ ID NO: 902 - DNA, 39 bp, synthetic construct
  misc_feature 1..39: note = Target Specific Oligonucleotide
  source 1..39: mol_type = other DNA
cagcccgaagtctgtgatcttgtaacgtgacgattaccc

SEQ ID NO: 903 - DNA, 37 bp, synthetic construct
  misc_feature 1..37: note = Target Specific Oligonucleotide
  source 1..37: mol_type = other DNA
tcatggtggcaccgtccttgtaacgtgacgattaccc

SEQ ID NO: 904 - DNA, 38 bp, synthetic construct
  misc_feature 1..38: note = Target Specific Oligonucleotide
  source 1..38: mol_type = other DNA
ggtagtccagggctgacacagtaacgtgacgattaccc

SEQ ID NO: 905 - DNA, 41 bp, synthetic construct
  misc_feature 1..41: note = Target Specific Oligonucleotide
  source 1..41: mol_type = other DNA
ccatcattcttgaggaggaagtagtaacgtgacgattaccc

SEQ ID NO: 906 - DNA, 37 bp, synthetic construct
  misc_feature 1..37: note = Target Specific Oligonucleotide
  source 1..37: mol_type = other DNA
acaaagcagaggcggtcgtgtaacgtgacgattaccc

SEQ ID NO: 907 - DNA, 38 bp, synthetic construct
  misc_feature 1..38: note = Target Specific Oligonucleotide
  source 1..38: mol_type = other DNA
cggtcctcggagaacacacggtaacgtgacgattaccc

SEQ ID NO: 908 - DNA, 37 bp, synthetic construct
  misc_feature 1..37: note = Target Specific Oligonucleotide
  source 1..37: mol_type = other DNA
gagcctcacgttggtccacgtaacgtgacgattaccc

SEQ ID NO: 909 - DNA, 40 bp, synthetic construct
  misc_feature 1..40: note = Target Specific Oligonucleotide
  source 1..40: mol_type = other DNA
ctccttgtagccaatgaaggtggtaacgtgacgattaccc

SEQ ID NO: 910 - DNA, 38 bp, synthetic construct
  misc_feature 1..38: note = Target Specific Oligonucleotide
  source 1..38: mol_type = other DNA
ttcacaatagccacgtcgctgtaacgtgacgattaccc

SEQ ID NO: 911 - DNA, 37 bp, synthetic construct
  misc_feature 1..37: note = Target Specific Oligonucleotide
  source 1..37: mol_type = other DNA
ccctcgtttgtgcagccaagtaacgtgacgattaccc

SEQ ID NO: 912 - DNA, 43 bp, synthetic construct
  misc_feature 1..43: note = Target Specific Oligonucleotide
  source 1..43: mol_type = other DNA
agctatgtccgctatcttcatcggtaactctcttctattgcag

SEQ ID NO: 913 - DNA, 41 bp, synthetic construct
  misc_feature 1..41: note = Target Specific Oligonucleotide
  source 1..41: mol_type = other DNA
ttggcacatcgagacatggttgtaactctcttctattgcag

SEQ ID NO: 914 - DNA, 42 bp, synthetic construct
  misc_feature 1..42: note = Target Specific Oligonucleotide
  source 1..42: mol_type = other DNA
ccatcttggtcgtactttgtgagtaactctcttctattgcag

SEQ ID NO: 915 - DNA, 41 bp, synthetic construct
  misc_feature 1..41: note = Target Specific Oligonucleotide
  source 1..41: mol_type = other DNA
ccaactgagcatacgctaggagtaactctcttctattgcag

SEQ ID NO: 916 - DNA, 41 bp, synthetic construct
  misc_feature 1..41: note = Target Specific Oligonucleotide
  source 1..41: mol_type = other DNA
tcacgtactagccgttccatcgtaactctcttctattgcag

SEQ ID NO: 917 - DNA, 43 bp, synthetic construct
  misc_feature 1..43: note = Target Specific Oligonucleotide
  source 1..43: mol_type = other DNA
tttctccaagtcgtctctcatctgtaactctcttctattgcag

SEQ ID NO: 918 - DNA, 42 bp, synthetic construct
  misc_feature 1..42: note = Target Specific Oligonucleotide
  source 1..42: mol_type = other DNA
tcgtaagaaacgccactagaaagtaactctcttctattgcag

SEQ ID NO: 919 - DNA, 39 bp, synthetic construct
  misc_feature 1..39: note = Target Specific Oligonucleotide
  source 1..39: mol_type = other DNA
cactggcgtgcctaaaccagtaactctcttctattgcag

SEQ ID NO: 920 - DNA, 45 bp, synthetic construct
  misc_feature 1..45: note = Target Specific Oligonucleotide
  source 1..45: mol_type = other DNA
acatatcatacgtggacattagaacgtaactctcttctattgcag

SEQ ID NO: 921 - DNA, 40 bp, synthetic construct
  misc_feature 1..40: note = Target Specific Oligonucleotide
  source 1..40: mol_type = other DNA
gccgatggaatgctccatccgtaactctcttctattgcag

SEQ ID NO: 922 - DNA, 43 bp, synthetic construct
  misc_feature 1..43: note = Target Specific Oligonucleotide
  source 1..43: mol_type = other DNA
gattagcaatcggtcacaaagacgtaactctcttctattgcag

SEQ ID NO: 923 - DNA, 43 bp, synthetic construct
  misc_feature 1..43: note = Target Specific Oligonucleotide
  source 1..43: mol_type = other DNA
ggtgtagtagtacacattggagcgtaactctcttctattgcag

SEQ ID NO: 924 - DNA, 42 bp, synthetic construct
  misc_feature 1..42: note = Target Specific Oligonucleotide
  source 1..42: mol_type = other DNA
gatgaaacttcggttgtcagctgtaactctcttctattgcag

SEQ ID NO: 925 - DNA, 42 bp, synthetic construct
  misc_feature 1..42: note = Target Specific Oligonucleotide
  source 1..42: mol_type = other DNA
ttcttgaggctagcaacttgtggtaactctcttctattgcag

SEQ ID NO: 926 - DNA, 43 bp, synthetic construct
  misc_feature 1..43: note = Target Specific Oligonucleotide
  source 1..43: mol_type = other DNA
gtcccaaaactcgattagcttccgtaactctcttctattgcag

SEQ ID NO: 927 - DNA, 42 bp, synthetic construct
  misc_feature 1..42: note = Target Specific Oligonucleotide
  source 1..42: mol_type = other DNA
tattcgtggaacccctaacagcgtaactctcttctattgcag

SEQ ID NO: 928 - DNA, 43 bp, synthetic construct
  misc_feature 1..43: note = Target Specific Oligonucleotide
  source 1..43: mol_type = other DNA
caaagttgatatcgcccaaaatggtaactctcttctattgcag

SEQ ID NO: 929 - DNA, 42 bp, synthetic construct
  misc_feature 1..42: note = Target Specific Oligonucleotide
  source 1..42: mol_type = other DNA
tagatccaagcggttccatttcgtaactctcttctattgcag

SEQ ID NO: 930 - DNA, 42 bp, synthetic construct
  misc_feature 1..42: note = Target Specific Oligonucleotide
  source 1..42: mol_type = other DNA
tgaccagttcccgtaaaacactgtaactctcttctattgcag

SEQ ID NO: 931 - DNA, 41 bp, synthetic construct
  misc_feature 1..41: note = Target Specific Oligonucleotide
  source 1..41: mol_type = other DNA
tggcacatggtcgatacacatgtaactctcttctattgcag

SEQ ID NO: 932 - DNA, 41 bp, synthetic construct
  misc_feature 1..41: note = Target Specific Oligonucleotide
  source 1..41: mol_type = other DNA
tgacagcacaacgatcacaacgtaactctcttctattgcag

SEQ ID NO: 933 - DNA, 42 bp, synthetic construct
  misc_feature 1..42: note = Target Specific Oligonucleotide
  source 1..42: mol_type = other DNA
aagctcatgaactatgccagaggtaactctcttctattgcag

SEQ ID NO: 934 - DNA, 41 bp, synthetic construct
  misc_feature 1..41: note = Target Specific Oligonucleotide
  source 1..41: mol_type = other DNA
cgtcatacctgaccgagtactgtaactctcttctattgcag

SEQ ID NO: 935 - DNA, 43 bp, synthetic construct
  misc_feature 1..43: note = Target Specific Oligonucleotide
  source 1..43: mol_type = other DNA
tcttgattgtcgagaaagacttggtaactctcttctattgcag

SEQ ID NO: 936 - DNA, 42 bp, synthetic construct
  misc_feature 1..42: note = Target Specific Oligonucleotide
  source 1..42: mol_type = other DNA
tactgagccctatcggaaagtgtaactgatcttcatattacg

SEQ ID NO: 937 - DNA, 42 bp, synthetic construct
  misc_feature 1..42: note = Target Specific Oligonucleotide
  source 1..42: mol_type = other DNA
ccaaatcccttcgcagcaattgtaactgatcttcatattacg

SEQ ID NO: 938 - DNA, 42 bp, synthetic construct
  misc_feature 1..42: note = Target Specific Oligonucleotide
  source 1..42: mol_type = other DNA
gccatgatcaatcgcatcactgtaactgatcttcatattacg

SEQ ID NO: 939 - DNA, 43 bp, synthetic construct
  misc_feature 1..43: note = Target Specific Oligonucleotide
  source 1..43: mol_type = other DNA
atcatccagattcgaaccgtccgtaactgatcttcatattacg

SEQ ID NO: 940 - DNA, 43 bp, synthetic construct
  misc_feature 1..43: note = Target Specific Oligonucleotide
  source 1..43: mol_type = other DNA
ggactacattcgtgaagaagctgtaactgatcttcatattacg

SEQ ID NO: 941 - DNA, 42 bp, synthetic construct
  misc_feature 1..42: note = Target Specific Oligonucleotide
  source 1..42: mol_type = other DNA
ggagaggatccgtccaagaaagtaactgatcttcatattacg

SEQ ID NO: 942 - DNA, 42 bp, synthetic construct
  misc_feature 1..42: note = Target Specific Oligonucleotide
  source 1..42: mol_type = other DNA
gtcccagcattagaacctgtggtaactgatcttcatattacg

SEQ ID NO: 943 - DNA, 42 bp, synthetic construct
  misc_feature 1..42: note = Target Specific Oligonucleotide
  source 1..42: mol_type = other DNA
actctcagccagacctttagcgtaactgatcttcatattacg

SEQ ID NO: 944 - DNA, 44 bp, synthetic construct
  misc_feature 1..44: note = Target Specific Oligonucleotide
  source 1..44: mol_type = other DNA
catagtgtcatgtgcatgtagtcgtaactgatcttcatattacg

SEQ ID NO: 945 - DNA, 44 bp, synthetic construct
  misc_feature 1..44: note = Target Specific Oligonucleotide
  source 1..44: mol_type = other DNA
ccctgaccagcatattatctacagtaactgatcttcatattacg

SEQ ID NO: 946 - DNA, 41 bp, synthetic construct
  misc_feature 1..41: note = Target Specific Oligonucleotide
  source 1..41: mol_type = other DNA
cagcgcctgttacaagctctgtaactgatcttcatattacg

SEQ ID NO: 947 - DNA, 41 bp, synthetic construct
  misc_feature 1..41: note = Target Specific Oligonucleotide
  source 1..41: mol_type = other DNA
cgccagtcttaactgccatggtaactgatcttcatattacg

SEQ ID NO: 948 - DNA, 43 bp, synthetic construct
  misc_feature 1..43: note = Target Specific Oligonucleotide
  source 1..43: mol_type = other DNA
tcttcccaacaccgtaatctttgtaactgatcttcatattacg

SEQ ID NO: 949 - DNA, 43 bp, synthetic construct
  misc_feature 1..43: note = Target Specific Oligonucleotide
  source 1..43: mol_type = other DNA
gtgacttatgttcgggtctctcgtaactgatcttcatattacg

SEQ ID NO: 950 - DNA, 43 bp, synthetic construct
  misc_feature 1..43: note = Target Specific Oligonucleotide
  source 1..43: mol_type = other DNA
tgttaggttctagggccatagcgtaactgatcttcatattacg

SEQ ID NO: 951 - DNA, 42 bp, synthetic construct
  misc_feature 1..42: note = Target Specific Oligonucleotide
  source 1..42: mol_type = other DNA
ctggatagctttgggcaactcgtaactgatcttcatattacg

SEQ ID NO: 952 - DNA, 45 bp, synthetic construct
  misc_feature 1..45: note = Target Specific Oligonucleotide
  source 1..45: mol_type = other DNA
tgcagacagggtatgtatatttgggtaactgatcttcatattacg

SEQ ID NO: 953 - DNA, 44 bp, synthetic construct
  misc_feature 1..44: note = Target Specific Oligonucleotide
  source 1..44: mol_type = other DNA
aagaaaatatagctgagctccctgtaactgatcttcatattacg

SEQ ID NO: 954 - DNA, 40 bp, synthetic construct
  misc_feature 1..40: note = Target Specific Oligonucleotide
  source 1..40: mol_type = other DNA
gagaccggagaaacccggcgtaactgatcttcatattacg

SEQ ID NO: 955 - DNA, 40 bp, synthetic construct
  misc_feature 1..40: note = Target Specific Oligonucleotide
  source 1..40: mol_type = other DNA
ccgcaggagaccgaggtctgtaactgatcttcatattacg

SEQ ID NO: 956 - DNA, 42 bp, synthetic construct
  misc_feature 1..42: note = Target Specific Oligonucleotide
  source 1..42: mol_type = other DNA
aggctagggctcaagacaagggtaactgatcttcatattacg

SEQ ID NO: 957 - DNA, 38 bp, synthetic construct
  misc_feature 1..38: note = Target Specific Oligonucleotide
  source 1..38: mol_type = other DNA
gcgtccggtgtcgccatgtaactgatcttcatattacg

SEQ ID NO: 958 - DNA, 41 bp, synthetic construct
  misc_feature 1..41: note = Target Specific Oligonucleotide
  source 1..41: mol_type = other DNA
actctgggtcggcttgatccgtaactgatcttcatattacg

SEQ ID NO: 959 - DNA, 41 bp, synthetic construct
  misc_feature 1..41: note = Target Specific Oligonucleotide
  source 1..41: mol_type = other DNA
catgggaggatcgagcctgggtaactgatcttcatattacg

SEQ ID NO: 960 - DNA, 39 bp, synthetic construct
  misc_feature 1..39: note = Target Specific Oligonucleotide
  source 1..39: mol_type = other DNA
ggcactggaaacgattgacttgtaacggcaatacatcgt

SEQ ID NO: 961 - DNA, 38 bp, synthetic construct
  misc_feature 1..38: note = Target Specific Oligonucleotide
  source 1..38: mol_type = other DNA
tcaggcattcgttcacctgtgtaacggcaatacatcgt

SEQ ID NO: 962 - DNA, 40 bp, synthetic construct
  misc_feature 1..40: note = Target Specific Oligonucleotide
  source 1..40: mol_type = other DNA
actgtagcgattaatgccatccgtaacggcaatacatcgt

SEQ ID NO: 963 - DNA, 38 bp, synthetic construct
  misc_feature 1..38: note = Target Specific Oligonucleotide
  source 1..38: mol_type = other DNA
atagcctccattgcggttgggtaacggcaatacatcgt

SEQ ID NO: 964 - DNA, 40 bp, synthetic construct
  misc_feature 1..40: note = Target Specific Oligonucleotide
  source 1..40: mol_type = other DNA
cattcgggtgatcgatacacttgtaacggcaatacatcgt

SEQ ID NO: 965 - DNA, 39 bp, synthetic construct
  misc_feature 1..39: note = Target Specific Oligonucleotide
  source 1..39: mol_type = other DNA
gcacactcatcgagttgctccgtaacggcaatacatcgt

SEQ ID NO: 966 - DNA, 37 bp, synthetic construct
  misc_feature 1..37: note = Target Specific Oligonucleotide
  source 1..37: mol_type = other DNA
tcccgcttaatgcgcaggtgtaacggcaatacatcgt

SEQ ID NO: 967 - DNA, 37 bp, synthetic construct
  misc_feature 1..37: note = Target Specific Oligonucleotide
  source 1..37: mol_type = other DNA
ggtcccctgtatggcgtgagtaacggcaatacatcgt

SEQ ID NO: 968 - DNA, 38 bp, synthetic construct
  misc_feature 1..38: note = Target Specific Oligonucleotide
  source 1..38: mol_type = other DNA
aacacactggcggttgtcaagtaacggcaatacatcgt

SEQ ID NO: 969 - DNA, 39 bp, synthetic construct
  misc_feature 1..39: note = Target Specific Oligonucleotide
  source 1..39: mol_type = other DNA
cacacatcgacgaaggtttcagtaacggcaatacatcgt

SEQ ID NO: 970 - DNA, 39 bp, synthetic construct
  misc_feature 1..39: note = Target Specific Oligonucleotide
  source 1..39: mol_type = other DNA
ggctcttgcacgagttaacttgtaacggcaatacatcgt

SEQ ID NO: 971 - DNA, 39 bp, synthetic construct
  misc_feature 1..39: note = Target Specific Oligonucleotide
  source 1..39: mol_type = other DNA
atgtcaatggtacaccgctgagtaacggcaatacatcgt

SEQ ID NO: 972 - DNA, 38 bp, synthetic construct
  misc_feature 1..38: note = Target Specific Oligonucleotide
  source 1..38: mol_type = other DNA
gccatgcttacgctttcgttgtaacggcaatacatcgt

SEQ ID NO: 973 - DNA, 40 bp, synthetic construct
  misc_feature 1..40: note = Target Specific Oligonucleotide
  source 1..40: mol_type = other DNA
ggtataccagtaacacggaccagtaacggcaatacatcgt

SEQ ID NO: 974 - DNA, 40 bp, synthetic construct
  misc_feature 1..40: note = Target Specific Oligonucleotide
  source 1..40: mol_type = other DNA
gactctctcacgcataaacctggtaacggcaatacatcgt

SEQ ID NO: 975 - DNA, 40 bp, synthetic construct
  misc_feature 1..40: note = Target Specific Oligonucleotide
  source 1..40: mol_type = other DNA
aggagatgcgtaggtcaattcagtaacggcaatacatcgt

SEQ ID NO: 976 - DNA, 39 bp, synthetic construct
  misc_feature 1..39: note = Target Specific Oligonucleotide
  source 1..39: mol_type = other DNA
ccaacaggacgctagtgtagagtaacggcaatacatcgt

SEQ ID NO: 977 - DNA, 42 bp, synthetic construct
  misc_feature 1..42: note = Target Specific Oligonucleotide
  source 1..42: mol_type = other DNA
cagtaccaattaggttagcttctggtaacggcaatacatcgt

SEQ ID NO: 978 - DNA, 38 bp, synthetic construct
  misc_feature 1..38: note = Target Specific Oligonucleotide
  source 1..38: mol_type = other DNA
tccatggccgtcgatcaatggtaacggcaatacatcgt

SEQ ID NO: 979 - DNA, 40 bp, synthetic construct
  misc_feature 1..40: note = Target Specific Oligonucleotide
  source 1..40: mol_type = other DNA
tagtcaggaatatgcggtcattgtaacggcaatacatcgt

SEQ ID NO: 980 - DNA, 41 bp, synthetic construct
  misc_feature 1..41: note = Target Specific Oligonucleotide
  source 1..41: mol_type = other DNA
tatagcaactacttcgcatttccgtaacggcaatacatcgt

SEQ ID NO: 981 - DNA, 39 bp, synthetic construct
  misc_feature 1..39: note = Target Specific Oligonucleotide
  source 1..39: mol_type = other DNA
cgatggtgtcctacggatgtcgtaacggcaatacatcgt

SEQ ID NO: 982 - DNA, 44 bp, synthetic construct
  misc_feature 1..44: note = Target Specific Oligonucleotide
  source 1..44: mol_type = other DNA
gtaaccatagtaccacttattagtgggtaacggcaatacatcgt

SEQ ID NO: 983 - DNA, 37 bp, synthetic construct
  misc_feature 1..37: note = Target Specific Oligonucleotide
  source 1..37: mol_type = other DNA
cagcatcagcccgtgagtagtaacggcaatacatcgt

SEQ ID NO: 984 - DNA, 39 bp, synthetic construct
  misc_feature 1..39: note = Target Specific Oligonucleotide
  source 1..39: mol_type = other DNA
tcagatgctactggccgcttagacaagttaagatcggaa

SEQ ID NO: 985 - DNA, 41 bp, synthetic construct
  misc_feature 1..41: note = Target Specific Oligonucleotide
  source 1..41: mol_type = other DNA
cttgatcaaggcgctgaacaatagacaagttaagatcggaa

SEQ ID NO: 986 - DNA, 41 bp, synthetic construct
  misc_feature 1..41: note = Target Specific Oligonucleotide
  source 1..41: mol_type = other DNA
tcccttcgtatctcagcgagatagacaagttaagatcggaa

SEQ ID NO: 987 - DNA, 41 bp, synthetic construct
  misc_feature 1..41: note = Target Specific Oligonucleotide
  source 1..41: mol_type = other DNA
agactgttgactggcgtgatgtagacaagttaagatcggaa

SEQ ID NO: 988 - DNA, 41 bp, synthetic construct
  misc_feature 1..41: note = Target Specific Oligonucleotide
  source 1..41: mol_type = other DNA
ccaacatgctcgcatgagttctagacaagttaagatcggaa

SEQ ID NO: 989 - DNA, 41 bp, synthetic construct
  misc_feature 1..41: note = Target Specific Oligonucleotide
  source 1..41: mol_type = other DNA
ttccttcaccgaactgaggagtagacaagttaagatcggaa

SEQ ID NO: 990 - DNA, 40 bp, synthetic construct
  misc_feature 1..40: note = Target Specific Oligonucleotide
  source 1..40: mol_type = other DNA
agttccaacgagcggcttcatagacaagttaagatcggaa

SEQ ID NO: 991 - DNA, 40 bp, synthetic construct
  misc_feature 1..40: note = Target Specific Oligonucleotide
  source 1..40: mol_type = other DNA
ccatggctgacgagatctgatagacaagttaagatcggaa

SEQ ID NO: 992 - DNA, 40 bp, synthetic construct
  misc_feature 1..40: note = Target Specific Oligonucleotide
  source 1..40: mol_type = other DNA
tagcctaagacccggagctttagacaagttaagatcggaa

SEQ ID NO: 993 - DNA, 40 bp, synthetic construct
  misc_feature 1..40: note = Target Specific Oligonucleotide
  source 1..40: mol_type = other DNA
gcagatactcagcggcattgtagacaagttaagatcggaa

SEQ ID NO: 994 - DNA, 40 bp, synthetic construct
  misc_feature 1..40: note = Target Specific Oligonucleotide
  source 1..40: mol_type = other DNA
catagctcacgcagaacgtgtagacaagttaagatcggaa

SEQ ID NO: 995 - DNA, 39 bp, synthetic construct
  misc_feature 1..39: note = Target Specific Oligonucleotide
  source 1..39: mol_type = other DNA
gtcggccaccgttgaatgatagacaagttaagatcggaa

SEQ ID NO: 996 - DNA, 39 bp, synthetic construct
  misc_feature 1..39: note = Target Specific Oligonucleotide
  source 1..39: mol_type = other DNA
agaacggtcagcgagcgtatagacaagttaagatcggaa

SEQ ID NO: 997 - DNA, 44 bp, synthetic construct
  misc_feature 1..44: note = Target Specific Oligonucleotide
  source 1..44: mol_type = other DNA
gttatgcttagagtgttatctccatagacaagttaagatcggaa

SEQ ID NO: 998 - DNA, 40 bp, synthetic construct
  misc_feature 1..40: note = Target Specific Oligonucleotide
  source 1..40: mol_type = other DNA
tggtgatgtccgtgcgttcctagacaagttaagatcggaa

SEQ ID NO: 999 - DNA, 40 bp, synthetic construct
  misc_feature 1..40: note = Target Specific Oligonucleotide
  source 1..40: mol_type = other DNA
ggtccagaggatcgctctcttagacaagttaagatcggaa

SEQ ID NO: 1000 - DNA, 39 bp, synthetic construct
  misc_feature 1..39: note = Target Specific Oligonucleotide
  source 1..39: mol_type = other DNA
cgtggactgcaagtcccgatagacaagttaagatcggaa

SEQ ID NO: 1001 - DNA, 41 bp, synthetic construct
  misc_feature 1..41: note = Target Specific Oligonucleotide
  source 1..41: mol_type = other DNA
acaggtcaattcccgggtaagtagacaagttaagatcggaa

SEQ ID NO: 1002 - DNA, 41 bp, synthetic construct
  misc_feature 1..41: note = Target Specific Oligonucleotide
  source 1..41: mol_type = other DNA
ctgcaccaggttagggtgttttagacaagttaagatcggaa

SEQ ID NO: 1003 - DNA, 43 bp, synthetic construct
  misc_feature 1..43: note = Target Specific Oligonucleotide
  source 1..43: mol_type = other DNA
ggaaatggcatatacgtgggatttagacaagttaagatcggaa

SEQ ID NO: 1004 - DNA, 40 bp, synthetic construct
  misc_feature 1..40: note = Target Specific Oligonucleotide
  source 1..40: mol_type = other DNA
cttttgtctttgcgcccaggtagacaagttaagatcggaa

SEQ ID NO: 1005 - DNA, 38 bp, synthetic construct
  misc_feature 1..38: note = Target Specific Oligonucleotide
  source 1..38: mol_type = other DNA
tcctgccggttgcactcctagacaagttaagatcggaa

SEQ ID NO: 1006 - DNA, 43 bp, synthetic construct
  misc_feature 1..43: note = Target Specific Oligonucleotide
  source 1..43: mol_type = other DNA
atcatacagtgcaacgaaaaggttagacaagttaagatcggaa

SEQ ID NO: 1007 - DNA, 40 bp, synthetic construct
  misc_feature 1..40: note = Target Specific Oligonucleotide
  source 1..40: mol_type = other DNA
tcccacttgtcgtagttgggtagacaagttaagatcggaa

SEQ ID NO: 1008 - DNA, 39 bp, synthetic construct
  misc_feature 1..39: note = Target Specific Oligonucleotide
  source 1..39: mol_type = other DNA
aggtggtgttccgaacgagctagacagcccaattaaacg

SEQ ID NO: 1009 - DNA, 39 bp, synthetic construct
  misc_feature 1..39: note = Target Specific Oligonucleotide
  source 1..39: mol_type = other DNA
agatccgtgagcggaatgtatagacagcccaattaaacg

SEQ ID NO: 1010 - DNA, 41 bp, synthetic construct
  misc_feature 1..41: note = Target Specific Oligonucleotide
  source 1..41: mol_type = other DNA
ctcactcgctttagtggactcctagacagcccaattaaacg

SEQ ID NO: 1011 - DNA, 37 bp, synthetic construct
  misc_feature 1..37: note = Target Specific Oligonucleotide
  source 1..37: mol_type = other DNA
gccaaagaccgtggcgagtagacagcccaattaaacg

SEQ ID NO: 1012 - DNA, 41 bp, synthetic construct
  misc_feature 1..41: note = Target Specific Oligonucleotide
  source 1..41: mol_type = other DNA
agagttcttggtcgttggatcctagacagcccaattaaacg

SEQ ID NO: 1013 - DNA, 39 bp, synthetic construct
  misc_feature 1..39: note = Target Specific Oligonucleotide
  source 1..39: mol_type = other DNA
ctcctttgcaaccgggtctgtagacagcccaattaaacg

SEQ ID NO: 1014 - DNA, 41 bp, synthetic construct
  misc_feature 1..41: note = Target Specific Oligonucleotide
  source 1..41: mol_type = other DNA
cttgttattgacgtcgaaggcttagacagcccaattaaacg

SEQ ID NO: 1015 - DNA, 40 bp, synthetic construct
  misc_feature 1..40: note = Target Specific Oligonucleotide
  source 1..40: mol_type = other DNA
caggaacgtgtaactcttgcctagacagcccaattaaacg

SEQ ID NO: 1016 - DNA, 40 bp, synthetic construct
  misc_feature 1..40: note = Target Specific Oligonucleotide
  source 1..40: mol_type = other DNA
ggagtttcacacacgagttggtagacagcccaattaaacg

SEQ ID NO: 1017 - DNA, 39 bp, synthetic construct
  misc_feature 1..39: note = Target Specific Oligonucleotide
  source 1..39: mol_type = other DNA
aggttcccgctctacggatgtagacagcccaattaaacg

SEQ ID NO: 1018 - DNA, 38 bp, synthetic construct
  misc_feature 1..38: note = Target Specific Oligonucleotide
  source 1..38: mol_type = other DNA
accgtcatggactgccgtctagacagcccaattaaacg

SEQ ID NO: 1019 - DNA, 40 bp, synthetic construct
  misc_feature 1..40: note = Target Specific Oligonucleotide
  source 1..40: mol_type = other DNA
tgggacctttagacttcggtgtagacagcccaattaaacg

SEQ ID NO: 1020 - DNA, 37 bp, synthetic construct
  misc_feature 1..37: note = Target Specific Oligonucleotide
  source 1..37: mol_type = other DNA
gtccctgtagacgcgcgttagacagcccaattaaacg

SEQ ID NO: 1021 - DNA, 38 bp, synthetic construct
  misc_feature 1..38: note = Target Specific Oligonucleotide
  source 1..38: mol_type = other DNA
ccagagagggcgcatcttgtagacagcccaattaaacg

SEQ ID NO: 1022 - DNA, 40 bp, synthetic construct
  misc_feature 1..40: note = Target Specific Oligonucleotide
  source 1..40: mol_type = other DNA
tccactctgcacgctcatagttagacagcccaattaaacg

SEQ ID NO: 1023 - DNA, 40 bp, synthetic construct
  misc_feature 1..40: note = Target Specific Oligonucleotide
  source 1..40: mol_type = other DNA
gtgaaactcgacgttcacgtatagacagcccaattaaacg

SEQ ID NO: 1024 - DNA, 40 bp, synthetic construct
  misc_feature 1..40: note = Target Specific Oligonucleotide
  source 1..40: mol_type = other DNA
acacctctttgtcgttgaccttagacagcccaattaaacg

SEQ ID NO: 1025 - DNA, 39 bp, synthetic construct
  misc_feature 1..39: note = Target Specific Oligonucleotide
  source 1..39: mol_type = other DNA
actgttgcgagttctgcgagtagacagcccaattaaacg

SEQ ID NO: 1026 - DNA, 39 bp, synthetic construct
  misc_feature 1..39: note = Target Specific Oligonucleotide
  source 1..39: mol_type = other DNA
tggcaactccgtagttgtcctagacagcccaattaaacg

SEQ ID NO: 1027 - DNA, 38 bp, synthetic construct
  misc_feature 1..38: note = Target Specific Oligonucleotide
  source 1..38: mol_type = other DNA
tcctcggacgctaagctcatagacagcccaattaaacg

SEQ ID NO: 1028 - DNA, 38 bp, synthetic construct
  misc_feature 1..38: note = Target Specific Oligonucleotide
  source 1..38: mol_type = other DNA
ttacccggagaaccctcgctagacagcccaattaaacg

SEQ ID NO: 1029 - DNA, 38 bp, synthetic construct
  misc_feature 1..38: note = Target Specific Oligonucleotide
  source 1..38: mol_type = other DNA
tcccggaacatgcggtaggtagacagcccaattaaacg

SEQ ID NO: 1030 - DNA, 38 bp, synthetic construct
  misc_feature 1..38: note = Target Specific Oligonucleotide
  source 1..38: mol_type = other DNA
tgctcgatgtcgcccactgtagacagcccaattaaacg

SEQ ID NO: 1031 - DNA, 37 bp, synthetic construct
  misc_feature 1..37: note = Target Specific Oligonucleotide
  source 1..37: mol_type = other DNA
tgccggtgccgcttatggtagacagcccaattaaacg

SEQ ID NO: 1032 - DNA, 45 bp, synthetic construct
  misc_feature 1..45: note = Target Specific Oligonucleotide
  source 1..45: mol_type = other DNA
ccaaagtctgctagcttgatggtagacggtataatacttatttcc

SEQ ID NO: 1033 - DNA, 48 bp, synthetic construct
  misc_feature 1..48: note = Target Specific Oligonucleotide
  source 1..48: mol_type = other DNA
tattaggatggttaagctccttaagtagacggtataatacttatttcc

SEQ ID NO: 1034 - DNA, 45 bp, synthetic construct
  misc_feature 1..45: note = Target Specific Oligonucleotide
  source 1..45: mol_type = other DNA
catgggtgtaagtacgaacaggtagacggtataatacttatttcc

SEQ ID NO: 1035 - DNA, 43 bp, synthetic construct
  misc_feature 1..43: note = Target Specific Oligonucleotide
  source 1..43: mol_type = other DNA
ggcagaaagctaggccctggtagacggtataatacttatttcc

SEQ ID NO: 1036 - DNA, 43 bp, synthetic construct
  misc_feature 1..43: note = Target Specific Oligonucleotide
  source 1..43: mol_type = other DNA
gtacacaactccgtacgtgctagacggtataatacttatttcc

SEQ ID NO: 1037 - DNA, 45 bp, synthetic construct
  misc_feature 1..45: note = Target Specific Oligonucleotide
  source 1..45: mol_type = other DNA
atggaacgcagtatacctctcgtagacggtataatacttatttcc

SEQ ID NO: 1038 - DNA, 46 bp, synthetic construct
  misc_feature 1..46: note = Target Specific Oligonucleotide
  source 1..46: mol_type = other DNA
cttggcttgtaatcaggcatagatagacggtataatacttatttcc

SEQ ID NO: 1039 - DNA, 41 bp, synthetic construct
  misc_feature 1..41: note = Target Specific Oligonucleotide
  source 1..41: mol_type = other DNA
ctccatgaagcgccagcgtagacggtataatacttatttcc

SEQ ID NO: 1040 - DNA, 43 bp, synthetic construct
  misc_feature 1..43: note = Target Specific Oligonucleotide
  source 1..43: mol_type = other DNA
ccgcttgttagggtcgtagttagacggtataatacttatttcc

SEQ ID NO: 1041 - DNA, 42 bp, synthetic construct
  misc_feature 1..42: note = Target Specific Oligonucleotide
  source 1..42: mol_type = other DNA
ctcggtggaggacccgatgtagacggtataatacttatttcc

SEQ ID NO: 1042 - DNA, 44 bp, synthetic construct
  misc_feature 1..44: note = Target Specific Oligonucleotide
  source 1..44: mol_type = other DNA
ttactaaaatcttgccgggcctagacggtataatacttatttcc

SEQ ID NO: 1043 - DNA, 44 bp, synthetic construct
  misc_feature 1..44: note = Target Specific Oligonucleotide
  source 1..44: mol_type = other DNA
gcagcatttgcgataacaagctagacggtataatacttatttcc

SEQ ID NO: 1044 - DNA, 45 bp, synthetic construct
  misc_feature 1..45: note = Target Specific Oligonucleotide
  source 1..45: mol_type = other DNA
agaaggctatcagagtcgaagatagacggtataatacttatttcc

SEQ ID NO: 1045 - DNA, 43 bp, synthetic construct
  misc_feature 1..43: note = Target Specific Oligonucleotide
  source 1..43: mol_type = other DNA
ttcaggagctcggtaccacatagacggtataatacttatttcc

SEQ ID NO: 1046 - DNA, 44 bp, synthetic construct
  misc_feature 1..44: note = Target Specific Oligonucleotide
  source 1..44: mol_type = other DNA
ccccagagtccgaaagatccgtagacggtataatacttatttcc

SEQ ID NO: 1047 - DNA, 42 bp, synthetic construct
  misc_feature 1..42: note = Target Specific Oligonucleotide
  source 1..42: mol_type = other DNA
acagggcccagtaccgtggtagacggtataatacttatttcc

SEQ ID NO: 1048 - DNA, 46 bp, synthetic construct
  misc_feature 1..46: note = Target Specific Oligonucleotide
  source 1..46: mol_type = other DNA
tcagcaataactaagagaaggggtagacggtataatacttatttcc

SEQ ID NO: 1049 - DNA, 46 bp, synthetic construct
  misc_feature 1..46: note = Target Specific Oligonucleotide
  source 1..46: mol_type = other DNA
gtacggcaaatctaacgtgtaggtagacggtataatacttatttcc

SEQ ID NO: 1050 - DNA, 44 bp, synthetic construct
  misc_feature 1..44: note = Target Specific Oligonucleotide
  source 1..44: mol_type = other DNA
tgaaacaatgttgccgcctcctagacggtataatacttatttcc

SEQ ID NO: 1051 - DNA, 47 bp, synthetic construct
  misc_feature 1..47: note = Target Specific Oligonucleotide
  source 1..47: mol_type = other DNA
taataattatggggcattcagagatagacggtataatacttatttcc

SEQ ID NO: 1052 - DNA, 43 bp, synthetic construct
  misc_feature 1..43: note = Target Specific Oligonucleotide
  source 1..43: mol_type = other DNA
tctcacctgcctcataaggctagacggtataatacttatttcc

SEQ ID NO: 1053 - DNA, 47 bp, synthetic construct
  misc_feature 1..47: note = Target Specific Oligonucleotide
  source 1..47: mol_type = other DNA
atggtgaagcaatagattggaatgtagacggtataatacttatttcc

SEQ ID NO: 1054 - DNA, 49 bp, synthetic construct
  misc_feature 1..49: note = Target Specific Oligonucleotide
  source 1..49: mol_type = other DNA
cactaactagggtataaactgattggtagacggtataatacttatttcc

SEQ ID NO: 1055 - DNA, 44 bp, synthetic construct
  misc_feature 1..44: note = Target Specific Oligonucleotide
  source 1..44: mol_type = other DNA
agaagggacaaacaaggggactagacggtataatacttatttcc

SEQ ID NO: 1056 - DNA, 43 bp, synthetic construct
  misc_feature 1..43: note = Target Specific Oligonucleotide
  source 1..43: mol_type = other DNA
agtccgatactcaagcgcaaatagacaataaattctaacgagc

SEQ ID NO: 1057 - DNA, 42 bp, synthetic construct
  misc_feature 1..42: note = Target Specific Oligonucleotide
  source 1..42: mol_type = other DNA
cttgttgcgctcacggtatgtagacaataaattctaacgagc

SEQ ID NO: 1058 - DNA, 43 bp, synthetic construct
  misc_feature 1..43: note = Target Specific Oligonucleotide
  source 1..43: mol_type = other DNA
ccagagttgtagacgagcagctagacaataaattctaacgagc

SEQ ID NO: 1059 - DNA, 41 bp, synthetic construct
  misc_feature 1..41: note = Target Specific Oligonucleotide
  source 1..41: mol_type = other DNA
ttagcatggcaacacggcgtagacaataaattctaacgagc

SEQ ID NO: 1060 - DNA, 41 bp, synthetic construct
  misc_feature 1..41: note = Target Specific Oligonucleotide
  source 1..41: mol_type = other DNA
atgatgcgcacttcacgggtagacaataaattctaacgagc

SEQ ID NO: 1061 - DNA, 42 bp, synthetic construct
  misc_feature 1..42: note = Target Specific Oligonucleotide
  source 1..42: mol_type = other DNA
cccaccgctaggagggtagctagacaataaattctaacgagc

SEQ ID NO: 1062 - DNA, 42 bp, synthetic construct
  misc_feature 1..42: note = Target Specific Oligonucleotide
  source 1..42: mol_type = other DNA
gcagtgtggttaggccgatgtagacaataaattctaacgagc

SEQ ID NO: 1063 - DNA, 41 bp, synthetic construct
  misc_feature 1..41: note = Target Specific Oligonucleotide
  source 1..41: mol_type = other DNA
gacacggcggtgcactatctagacaataaattctaacgagc

SEQ ID NO: 1064 - DNA, 40 bp, synthetic construct
  misc_feature 1..40: note = Target Specific Oligonucleotide
  source 1..40: mol_type = other DNA
gcccaaagcggcttgcagtagacaataaattctaacgagc

SEQ ID NO: 1065 - DNA, 44 bp, synthetic construct
  misc_feature 1..44: note = Target Specific Oligonucleotide
  source 1..44: mol_type = other DNA
atacacacacggctaatactgctagacaataaattctaacgagc

SEQ ID NO: 1066 - DNA, 43 bp, synthetic construct
  misc_feature 1..43: note = Target Specific Oligonucleotide
  source 1..43: mol_type = other DNA
gtgaccgtgtacaccaacaactagacaataaattctaacgagc

SEQ ID NO: 1067 - DNA, 46 bp, synthetic construct
  misc_feature 1..46: note = Target Specific Oligonucleotide
  source 1..46: mol_type = other DNA
ctcttcatactagcatgactgtcatagacaataaattctaacgagc

SEQ ID NO: 1068 - DNA, 42 bp, synthetic construct
  misc_feature 1..42: note = Target Specific Oligonucleotide
  source 1..42: mol_type = other DNA
agaaggctttcgtcgttccctagacaataaattctaacgagc

SEQ ID NO: 1069 - DNA, 42 bp, synthetic construct
  misc_feature 1..42: note = Target Specific Oligonucleotide
  source 1..42: mol_type = other DNA
tttgctccgtgcgttcaaggtagacaataaattctaacgagc

SEQ ID NO: 1070 - DNA, 42 bp, synthetic construct
  misc_feature 1..42: note = Target Specific Oligonucleotide
  source 1..42: mol_type = other DNA
tccagtgcatccgtcacatctagacaataaattctaacgagc

SEQ ID NO: 1071 - DNA, 41 bp, synthetic construct
  misc_feature 1..41: note = Target Specific Oligonucleotide
  source 1..41: mol_type = other DNA
gatgaacagcggtgcgttgtagacaataaattctaacgagc

SEQ ID NO: 1072 - DNA, 42 bp, synthetic construct
  misc_feature 1..42: note = Target Specific Oligonucleotide
  source 1..42: mol_type = other DNA
cactgataccggctctccgttagacaataaattctaacgagc

SEQ ID NO: 1073 - DNA, 42 bp, synthetic construct
  misc_feature 1..42: note = Target Specific Oligonucleotide
  source 1..42: mol_type = other DNA
gaacgcttgcgttccctagctagacaataaattctaacgagc

SEQ ID NO: 1074 - DNA, 45 bp, synthetic construct
  misc_feature 1..45: note = Target Specific Oligonucleotide
  source 1..45: mol_type = other DNA
cagatagatttccgggatacagctagacaataaattctaacgagc

SEQ ID NO: 1075 - DNA, 40 bp, synthetic construct
  misc_feature 1..40: note = Target Specific Oligonucleotide
  source 1..40: mol_type = other DNA
tctgctgcggcgattgtgtagacaataaattctaacgagc

SEQ ID NO: 1076 - DNA, 41 bp, synthetic construct
  misc_feature 1..41: note = Target Specific Oligonucleotide
  source 1..41: mol_type = other DNA
ctcggtgatcatgcgtccctagacaataaattctaacgagc

SEQ ID NO: 1077 - DNA, 43 bp, synthetic construct
  misc_feature 1..43: note = Target Specific Oligonucleotide
  source 1..43: mol_type = other DNA
tccaatttcagggcgttctcgtagacaataaattctaacgagc

SEQ ID NO: 1078 - DNA, 40 bp, synthetic construct
  misc_feature 1..40: note = Target Specific Oligonucleotide
  source 1..40: mol_type = other DNA
tgcgcaggtcgacgtcagtagacaataaattctaacgagc

SEQ ID NO: 1079 - DNA, 43 bp, synthetic construct
  misc_feature 1..43: note = Target Specific Oligonucleotide
  source 1..43: mol_type = other DNA
gtccaggtagtatccggagggtagacaataaattctaacgagc

SEQ ID NO: 1080 - DNA, 40 bp, synthetic construct
  misc_feature 1..40: note = Target Specific Oligonucleotide
  source 1..40: mol_type = other DNA
attcccgacagactcatcgctagacgataaattgcgaacg

SEQ ID NO: 1081 - DNA, 40 bp, synthetic construct
  misc_feature 1..40: note = Target Specific Oligonucleotide
  source 1..40: mol_type = other DNA
cagttacatgttcgcgcacgtagacgataaattgcgaacg

SEQ ID NO: 1082 - DNA, 39 bp, synthetic construct
  misc_feature 1..39: note = Target Specific Oligonucleotide
  source 1..39: mol_type = other DNA
acgagcactagggtcgtcgtagacgataaattgcgaacg

SEQ ID NO: 1083 - DNA, 46 bp, synthetic construct
  misc_feature 1..46: note = Target Specific Oligonucleotide
  source 1..46: mol_type = other DNA
ttttgataatcgaatgaaaaagtcactagacgataaattgcgaacg

SEQ ID NO: 1084 - DNA, 43 bp, synthetic construct
  misc_feature 1..43: note = Target Specific Oligonucleotide
  source 1..43: mol_type = other DNA
ctgaatactgctagacgagaagctagacgataaattgcgaacg

SEQ ID NO: 1085 - DNA, 43 bp, synthetic construct
  misc_feature 1..43: note = Target Specific Oligonucleotide
  source 1..43: mol_type = other DNA
ctccttggaacgaactaatcctgtagacgataaattgcgaacg

SEQ ID NO: 1086 - DNA, 42 bp, synthetic construct
  misc_feature 1..42: note = Target Specific Oligonucleotide
  source 1..42: mol_type = other DNA
ttcaggcggttaattggtaccctagacgataaattgcgaacg

SEQ ID NO: 1087 - DNA, 42 bp, synthetic construct
  misc_feature 1..42: note = Target Specific Oligonucleotide
  source 1..42: mol_type = other DNA
gttaggaatggcgaacagacagtagacgataaattgcgaacg

SEQ ID NO: 1088 - DNA, 42 bp, synthetic construct
  misc_feature 1..42: note = Target Specific Oligonucleotide
  source 1..42: mol_type = other DNA
gatggtcttaaagcgtgaagcctagacgataaattgcgaacg

SEQ ID NO: 1089 - DNA, 42 bp, synthetic construct
  misc_feature 1..42: note = Target Specific Oligonucleotide
  source 1..42: mol_type = other DNA
ctgtgcctagccctaacttatatagacgataaattgcgaacg

SEQ ID NO: 1090 - DNA, 42 bp, synthetic construct
  misc_feature 1..42: note = Target Specific Oligonucleotide
  source 1..42: mol_type = other DNA
agagaccacccataacaagagttagacgataaattgcgaacg

SEQ ID NO: 1091 - DNA, 43 bp, synthetic construct
  misc_feature 1..43: note = Target Specific Oligonucleotide
  source 1..43: mol_type = other DNA
ttggagcaccgatatagatatggtagacgataaattgcgaacg

SEQ ID NO: 1092 - DNA, 41 bp, synthetic construct
  misc_feature 1..41: note = Target Specific Oligonucleotide
  source 1..41: mol_type = other DNA
tcaaagacgcaaacgtccaaatagacgataaattgcgaacg

SEQ ID NO: 1093 - DNA, 42 bp, synthetic construct
  misc_feature 1..42: note = Target Specific Oligonucleotide
  source 1..42: mol_type = other DNA
gagagctgattaggtgctcaggtagacgataaattgcgaacg

SEQ ID NO: 1094 - DNA, 40 bp, synthetic construct
  misc_feature 1..40: note = Target Specific Oligonucleotide
  source 1..40: mol_type = other DNA
tgcttgtacgcggagaaggttagacgataaattgcgaacg

SEQ ID NO: 1095 - DNA, 40 bp, synthetic construct
  misc_feature 1..40: note = Target Specific Oligonucleotide
  source 1..40: mol_type = other DNA
ctgcagacacgtgtatgtgctagacgataaattgcgaacg

SEQ ID NO: 1096 - DNA, 40 bp, synthetic construct
  misc_feature 1..40: note = Target Specific Oligonucleotide
  source 1..40: mol_type = other DNA
catccaatgcaagtccggtgtagacgataaattgcgaacg

SEQ ID NO: 1097 - DNA, 42 bp, synthetic construct
  misc_feature 1..42: note = Target Specific Oligonucleotide
  source 1..42: mol_type = other DNA
accaagtgataacgtgttcagatagacgataaattgcgaacg

SEQ ID NO: 1098 - DNA, 42 bp, synthetic construct
  misc_feature 1..42: note = Target Specific Oligonucleotide
  source 1..42: mol_type = other DNA
aatctgagctttgcgaaatggttagacgataaattgcgaacg

SEQ ID NO: 1099 - DNA, 44 bp, synthetic construct
  misc_feature 1..44: note = Target Specific Oligonucleotide
  source 1..44: mol_type = other DNA
caaagcccacataacactatcttttagacgataaattgcgaacg

SEQ ID NO: 1100 - DNA, 44 bp, synthetic construct
  misc_feature 1..44: note = Target Specific Oligonucleotide
  source 1..44: mol_type = other DNA
tgtactggactatagacaccaatttagacgataaattgcgaacg

SEQ ID NO: 1101 - DNA, 45 bp, synthetic construct
  misc_feature 1..45: note = Target Specific Oligonucleotide
  source 1..45: mol_type = other DNA
atcaatataccacgttagtagtcactagacgataaattgcgaacg

SEQ ID NO: 1102 - DNA, 42 bp, synthetic construct
  misc_feature 1..42: note = Target Specific Oligonucleotide
  source 1..42: mol_type = other DNA
tgtattttaacgccaagcaggctagacgataaattgcgaacg

SEQ ID NO: 1103 - DNA, 42 bp, synthetic construct
  misc_feature 1..42: note = Target Specific Oligonucleotide
  source 1..42: mol_type = other DNA
cactgaaaacacggttatgtcctagacgataaattgcgaacg

SEQ ID NO: 1104 - DNA, 40 bp, synthetic construct
  misc_feature 1..40: note = Target Specific Oligonucleotide
  source 1..40: mol_type = other DNA
cgagacagatcggagtagctgtagacgaccgaatttacgg

SEQ ID NO: 1105 - DNA, 41 bp, synthetic construct
  misc_feature 1..41: note = Target Specific Oligonucleotide
  source 1..41: mol_type = other DNA
tctctcaatgacgggacaaagatagacgaccgaatttacgg

SEQ ID NO: 1106 - DNA, 41 bp, synthetic construct
  misc_feature 1..41: note = Target Specific Oligonucleotide
  source 1..41: mol_type = other DNA
cagatgtggtgtatggtccacatagacgaccgaatttacgg

SEQ ID NO: 1107 - DNA, 40 bp, synthetic construct
  misc_feature 1..40: note = Target Specific Oligonucleotide
  source 1..40: mol_type = other DNA
ttctcctcggttacttcgtgatagacgaccgaatttacgg

SEQ ID NO: 1108 - DNA, 39 bp, synthetic construct
  misc_feature 1..39: note = Target Specific Oligonucleotide
  source 1..39: mol_type = other DNA
tgtgctaagccgaaggaggttagacgaccgaatttacgg

SEQ ID NO: 1109 - DNA, 44 bp, synthetic construct
  misc_feature 1..44: note = Target Specific Oligonucleotide
  source 1..44: mol_type = other DNA
gtaaacatagaacgactcatagtcatagacgaccgaatttacgg

SEQ ID NO: 1110 - DNA, 43 bp, synthetic construct
  misc_feature 1..43: note = Target Specific Oligonucleotide
  source 1..43: mol_type = other DNA
ttccacttcaattagctcttgaattagacgaccgaatttacgg

SEQ ID NO: 1111 - DNA, 40 bp, synthetic construct
  misc_feature 1..40: note = Target Specific Oligonucleotide
  source 1..40: mol_type = other DNA
ctggggtagagatagctcgcttagacgaccgaatttacgg

SEQ ID NO: 1112 - DNA, 41 bp, synthetic construct
  misc_feature 1..41: note = Target Specific Oligonucleotide
  source 1..41: mol_type = other DNA
gctataagctcgcctaccattctagacgaccgaatttacgg

SEQ ID NO: 1113 - DNA, 39 bp, synthetic construct
  misc_feature 1..39: note = Target Specific Oligonucleotide
  source 1..39: mol_type = other DNA
ttcttggggcgggtagagtgtagacgaccgaatttacgg

SEQ ID NO: 1114 - DNA, 40 bp, synthetic construct
  misc_feature 1..40: note = Target Specific Oligonucleotide
  source 1..40: mol_type = other DNA
aagacctcagaccgtcagaagtagacgaccgaatttacgg

SEQ ID NO: 1115 - DNA, 39 bp, synthetic construct
  misc_feature 1..39: note = Target Specific Oligonucleotide
  source 1..39: mol_type = other DNA
tcagatcctgacgacctgcatagacgaccgaatttacgg

SEQ ID NO: 1116 - DNA, 40 bp, synthetic construct
  misc_feature 1..40: note = Target Specific Oligonucleotide
  source 1..40: mol_type = other DNA
gcagaaatctcgagaggacgctagacgaccgaatttacgg

SEQ ID NO: 1117 - DNA, 39 bp, synthetic construct
  misc_feature 1..39: note = Target Specific Oligonucleotide
  source 1..39: mol_type = other DNA
ctcgcagtctaggccgaagatagacgaccgaatttacgg

SEQ ID NO: 1118 - DNA, 39 bp, synthetic construct
  misc_feature 1..39: note = Target Specific Oligonucleotide
  source 1..39: mol_type = other DNA
ccggtctccctcgagaatcatagacgaccgaatttacgg

SEQ ID NO: 1119 - DNA, 39 bp, synthetic construct
  misc_feature 1..39: note = Target Specific Oligonucleotide
  source 1..39: mol_type = other DNA
tcctggtgagaacgtcctgctagacgaccgaatttacgg

SEQ ID NO: 1120 - DNA, 38 bp, synthetic construct
  misc_feature 1..38: note = Target Specific Oligonucleotide
  source 1..38: mol_type = other DNA
tgccctttggtaaggcgcctagacgaccgaatttacgg

SEQ ID NO: 1121 - DNA, 38 bp, synthetic construct
  misc_feature 1..38: note = Target Specific Oligonucleotide
  source 1..38: mol_type = other DNA
cacagacacagccgaggactagacgaccgaatttacgg

SEQ ID NO: 1122 - DNA, 39 bp, synthetic construct
  misc_feature 1..39: note = Target Specific Oligonucleotide
  source 1..39: mol_type = other DNA
tcccaaaagctaccgctgagtagacgaccgaatttacgg

SEQ ID NO: 1123 - DNA, 39 bp, synthetic construct
  misc_feature 1..39: note = Target Specific Oligonucleotide
  source 1..39: mol_type = other DNA
taaggtagagtcgggcgaagtagacgaccgaatttacgg

SEQ ID NO: 1124 - DNA, 38 bp, synthetic construct
  misc_feature 1..38: note = Target Specific Oligonucleotide
  source 1..38: mol_type = other DNA
gagtggccggaaaaacccgtagacgaccgaatttacgg

SEQ ID NO: 1125 - DNA, 37 bp, synthetic construct
  misc_feature 1..37: note = Target Specific Oligonucleotide
  source 1..37: mol_type = other DNA
atgcggacatggtcgccctagacgaccgaatttacgg

SEQ ID NO: 1126 - DNA, 37 bp, synthetic construct
  misc_feature 1..37: note = Target Specific Oligonucleotide
  source 1..37: mol_type = other DNA
ggctcccaaacgccctgatagacgaccgaatttacgg

SEQ ID NO: 1127 - DNA, 40 bp, synthetic construct
  misc_feature 1..40: note = Target Specific Oligonucleotide
  source 1..40: mol_type = other DNA
tccatttcaccgtcagaaaggtagacgaccgaatttacgg

SEQ ID NO: 1128 - DNA, 43 bp, synthetic construct
  misc_feature 1..43: note = Target Specific Oligonucleotide
  source 1..43: mol_type = other DNA
ttgcctagacagcaccgtaatgtagacacgaatattccaattc

SEQ ID NO: 1129 - DNA, 40 bp, synthetic construct
  misc_feature 1..40: note = Target Specific Oligonucleotide
  source 1..40: mol_type = other DNA
ttcccagagcgtggttccatagacacgaatattccaattc

SEQ ID NO: 1130 - DNA, 42 bp, synthetic construct
  misc_feature 1..42: note = Target Specific Oligonucleotide
  source 1..42: mol_type = other DNA
taaggacatcgcttttccggttagacacgaatattccaattc

SEQ ID NO: 1131 - DNA, 40 bp, synthetic construct
  misc_feature 1..40: note = Target Specific Oligonucleotide
  source 1..40: mol_type = other DNA
ttctccacgtcgcggacactagacacgaatattccaattc

SEQ ID NO: 1132 - DNA, 46 bp, synthetic construct
  misc_feature 1..46: note = Target Specific Oligonucleotide
  source 1..46: mol_type = other DNA
gttctcatgatagaggttccttaagtagacacgaatattccaattc

SEQ ID NO: 1133 - DNA, 38 bp, synthetic construct
  misc_feature 1..38: note = Target Specific Oligonucleotide
  source 1..38: mol_type = other DNA
ggccacgtcggtgcagatagacacgaatattccaattc

SEQ ID NO: 1134 - DNA, 41 bp, synthetic construct
  misc_feature 1..41: note = Target Specific Oligonucleotide
  source 1..41: mol_type = other DNA
gttgtggacgatcaacggggtagacacgaatattccaattc

SEQ ID NO: 1135 - DNA, 42 bp, synthetic construct
  misc_feature 1..42: note = Target Specific Oligonucleotide
  source 1..42: mol_type = other DNA
tgtccccttcggggtcatacctagacacgaatattccaattc

SEQ ID NO: 1136 - DNA, 44 bp, synthetic construct
  misc_feature 1..44: note = Target Specific Oligonucleotide
  source 1..44: mol_type = other DNA
aatagaacctcatccggtagtggtagacacgaatattccaattc

SEQ ID NO: 1137 - DNA, 42 bp, synthetic construct
  misc_feature 1..42: note = Target Specific Oligonucleotide
  source 1..42: mol_type = other DNA
cagtgcagcgtatgtggtatttagacacgaatattccaattc

SEQ ID NO: 1138 - DNA, 42 bp, synthetic construct
  misc_feature 1..42: note = Target Specific Oligonucleotide
  source 1..42: mol_type = other DNA
aaagcttgtccgattggatggtagacacgaatattccaattc

SEQ ID NO: 1139 - DNA, 42 bp, synthetic construct
  misc_feature 1..42: note = Target Specific Oligonucleotide
  source 1..42: mol_type = other DNA
aacccttgtagatcggtggtatagacacgaatattccaattc

SEQ ID NO: 1140 - DNA, 42 bp, synthetic construct
  misc_feature 1..42: note = Target Specific Oligonucleotide
  source 1..42: mol_type = other DNA
agtagagaacgtttccaccgttagacacgaatattccaattc

SEQ ID NO: 1141 - DNA, 42 bp, synthetic construct
  misc_feature 1..42: note = Target Specific Oligonucleotide
  source 1..42: mol_type = other DNA
actgctcattgtcgttggttctagacacgaatattccaattc

SEQ ID NO: 1142 - DNA, 41 bp, synthetic construct
  misc_feature 1..41: note = Target Specific Oligonucleotide
  source 1..41: mol_type = other DNA
aacgtattgccgagaacccatagacacgaatattccaattc

SEQ ID NO: 1143 - DNA, 43 bp, synthetic construct
  misc_feature 1..43: note = Target Specific Oligonucleotide
  source 1..43: mol_type = other DNA
acaaagtgcatatagagtggcctagacacgaatattccaattc

SEQ ID NO: 1144 - DNA, 42 bp, synthetic construct
  misc_feature 1..42: note = Target Specific Oligonucleotide
  source 1..42: mol_type = other DNA
agccatccctagacactcgtttagacacgaatattccaattc

SEQ ID NO: 1145 - DNA, 42 bp, synthetic construct
  misc_feature 1..42: note = Target Specific Oligonucleotide
  source 1..42: mol_type = other DNA
gcgatttggagcataccagagtagacacgaatattccaattc

SEQ ID NO: 1146 - DNA, 42 bp, synthetic construct
  misc_feature 1..42: note = Target Specific Oligonucleotide
  source 1..42: mol_type = other DNA
aggatccgatcgaaactcagctagacacgaatattccaattc

SEQ ID NO: 1147 - DNA, 44 bp, synthetic construct
  misc_feature 1..44: note = Target Specific Oligonucleotide
  source 1..44: mol_type = other DNA
ctggaatatatcgcttgtagctgtagacacgaatattccaattc

SEQ ID NO: 1148 - DNA, 41 bp, synthetic construct
  misc_feature 1..41: note = Target Specific Oligonucleotide
  source 1..41: mol_type = other DNA
cttcaggtcatgcgtggacatagacacgaatattccaattc

SEQ ID NO: 1149 - DNA, 41 bp, synthetic construct
  misc_feature 1..41: note = Target Specific Oligonucleotide
  source 1..41: mol_type = other DNA
agagaagcgcacttccgtgttagacacgaatattccaattc

SEQ ID NO: 1150 - DNA, 41 bp, synthetic construct
  misc_feature 1..41: note = Target Specific Oligonucleotide
  source 1..41: mol_type = other DNA
tgatgttatccgtgcgcaggtagacacgaatattccaattc

SEQ ID NO: 1151 - DNA, 44 bp, synthetic construct
  misc_feature 1..44: note = Target Specific Oligonucleotide
  source 1..44: mol_type = other DNA
aaagaccgtaatcgttcacattgtagacacgaatattccaattc

SEQ ID NO: 1152 - DNA, 42 bp, synthetic construct
  misc_feature 1..42: note = Target Specific Oligonucleotide
  source 1..42: mol_type = other DNA
agagatttgtctacgtagagccgtagactcagaaatctcacg

SEQ ID NO: 1153 - DNA, 41 bp, synthetic construct
  misc_feature 1..41: note = Target Specific Oligonucleotide
  source 1..41: mol_type = other DNA
tcctttgcatacggtctcttcgtagactcagaaatctcacg

SEQ ID NO: 1154 - DNA, 43 bp, synthetic construct
  misc_feature 1..43: note = Target Specific Oligonucleotide
  source 1..43: mol_type = other DNA
aagtttgtttacatccgatgttactagactcagaaatctcacg

SEQ ID NO: 1155 - DNA, 39 bp, synthetic construct
  misc_feature 1..39: note = Target Specific Oligonucleotide
  source 1..39: mol_type = other DNA
ttcccatacagaacgtggcctagactcagaaatctcacg

SEQ ID NO: 1156 - DNA, 40 bp, synthetic construct
  misc_feature 1..40: note = Target Specific Oligonucleotide
  source 1..40: mol_type = other DNA
aacagatcaacggcaaaagcctagactcagaaatctcacg

SEQ ID NO: 1157 - DNA, 42 bp, synthetic construct
  misc_feature 1..42: note = Target Specific Oligonucleotide
  source 1..42: mol_type = other DNA
catccttgggtagtaggatgaactagactcagaaatctcacg

SEQ ID NO: 1158 - DNA, 40 bp, synthetic construct
  misc_feature 1..40: note = Target Specific Oligonucleotide
  source 1..40: mol_type = other DNA
gaatttgctagttgcagggcatagactcagaaatctcacg

SEQ ID NO: 1159 - DNA, 45 bp, synthetic construct
  misc_feature 1..45: note = Target Specific Oligonucleotide
  source 1..45: mol_type = other DNA
tgatcttacaattgatactgtcaatgtagactcagaaatctcacg

SEQ ID NO: 1160 - DNA, 38 bp, synthetic construct
  misc_feature 1..38: note = Target Specific Oligonucleotide
  source 1..38: mol_type = other DNA
tggatgtggaggcgaccgttagactcagaaatctcacg

SEQ ID NO: 1161 - DNA, 42 bp, synthetic construct
  misc_feature 1..42: note = Target Specific Oligonucleotide
  source 1..42: mol_type = other DNA
acttctggacctatagtagcctgtagactcagaaatctcacg

SEQ ID NO: 1162 - DNA, 42 bp, synthetic construct
  misc_feature 1..42: note = Target Specific Oligonucleotide
  source 1..42: mol_type = other DNA
caacacggatagcttatccaacctagactcagaaatctcacg

SEQ ID NO: 1163 - DNA, 40 bp, synthetic construct
  misc_feature 1..40: note = Target Specific Oligonucleotide
  source 1..40: mol_type = other DNA
tgtcaaggtaacgtgagcacttagactcagaaatctcacg

SEQ ID NO: 1164 - DNA, 41 bp, synthetic construct
  misc_feature 1..41: note = Target Specific Oligonucleotide
  source 1..41: mol_type = other DNA
tttacagaaatcggcatccacatagactcagaaatctcacg

SEQ ID NO: 1165 - DNA, 44 bp, synthetic construct
  misc_feature 1..44: note = Target Specific Oligonucleotide
  source 1..44: mol_type = other DNA
cagctactagaggtctataattccttagactcagaaatctcacg

SEQ ID NO: 1166 - DNA, 40 bp, synthetic construct
  misc_feature 1..40: note = Target Specific Oligonucleotide
  source 1..40: mol_type = other DNA
ctggcacctctatggaatccctagactcagaaatctcacg

SEQ ID NO: 1167 - DNA, 43 bp, synthetic construct
  misc_feature 1..43: note = Target Specific Oligonucleotide
  source 1..43: mol_type = other DNA
attctgatatcggctattgtgagatagactcagaaatctcacg

SEQ ID NO: 1168 - DNA, 39 bp, synthetic construct
  misc_feature 1..39: note = Target Specific Oligonucleotide
  source 1..39: mol_type = other DNA
gccaccagtctagtgccaactagactcagaaatctcacg

SEQ ID NO: 1169 - DNA, 40 bp, synthetic construct
  misc_feature 1..40: note = Target Specific Oligonucleotide
  source 1..40: mol_type = other DNA
caactaccccggacaatttgatagactcagaaatctcacg

SEQ ID NO: 1170 - DNA, 41 bp, synthetic construct
  misc_feature 1..41: note = Target Specific Oligonucleotide
  source 1..41: mol_type = other DNA
aggacttaacatgggctatgcctagactcagaaatctcacg

SEQ ID NO: 1171 - DNA, 41 bp, synthetic construct
  misc_feature 1..41: note = Target Specific Oligonucleotide
  source 1..41: mol_type = other DNA
ctctgcgaacgaagtgtttttgtagactcagaaatctcacg

SEQ ID NO: 1172 - DNA, 43 bp, synthetic construct
  misc_feature 1..43: note = Target Specific Oligonucleotide
  source 1..43: mol_type = other DNA
tgcagcatattaaggtgttgattttagactcagaaatctcacg

SEQ ID NO: 1173 - DNA, 44 bp, synthetic construct
  misc_feature 1..44: note = Target Specific Oligonucleotide
  source 1..44: mol_type = other DNA
aagtaactaaacccatagactgaaatagactcagaaatctcacg

SEQ ID NO: 1174 - DNA, 40 bp, synthetic construct
  misc_feature 1..40: note = Target Specific Oligonucleotide
  source 1..40: mol_type = other DNA
ctgccagggcttaacataaggtagactcagaaatctcacg

SEQ ID NO: 1175 - DNA, 42 bp, synthetic construct
  misc_feature 1..42: note = Target Specific Oligonucleotide
  source 1..42: mol_type = other DNA
ataacatttgatagggccactcctagactcagaaatctcacg

SEQ ID NO: 1176 - DNA, 41 bp, synthetic construct
  misc_feature 1..41: note = Target Specific Oligonucleotide
  source 1..41: mol_type = other DNA
ctgaagataatcgcagacaccctagacgtctcccgtatttt

SEQ ID NO: 1177 - DNA, 41 bp, synthetic construct
  misc_feature 1..41: note = Target Specific Oligonucleotide
  source 1..41: mol_type = other DNA
tgactgaacacgtgttctgttctagacgtctcccgtatttt

SEQ ID NO: 1178 - DNA, 39 bp, synthetic construct
  misc_feature 1..39: note = Target Specific Oligonucleotide
  source 1..39: mol_type = other DNA
tttcagccatacccggatggtagacgtctcccgtatttt

SEQ ID NO: 1179 - DNA, 41 bp, synthetic construct
  misc_feature 1..41: note = Target Specific Oligonucleotide
  source 1..41: mol_type = other DNA
tgagaagagtaaccgctgaatatagacgtctcccgtatttt

SEQ ID NO: 1180 - DNA, 38 bp, synthetic construct
  misc_feature 1..38: note = Target Specific Oligonucleotide
  source 1..38: mol_type = other DNA
acactgcaattccgccgtctagacgtctcccgtatttt

SEQ ID NO: 1181 - DNA, 38 bp, synthetic construct
  misc_feature 1..38: note = Target Specific Oligonucleotide
  source 1..38: mol_type = other DNA
ttgtcgtggccggtactgatagacgtctcccgtatttt

SEQ ID NO: 1182 - DNA, 39 bp, synthetic construct
  misc_feature 1..39: note = Target Specific Oligonucleotide
  source 1..39: mol_type = other DNA
ggcaggcgacactaccttcatagacgtctcccgtatttt

SEQ ID NO: 1183 - DNA, 40 bp, synthetic construct
  misc_feature 1..40: note = Target Specific Oligonucleotide
  source 1..40: mol_type = other DNA
ctgggccagtattgaccactgtagacgtctcccgtatttt

SEQ ID NO: 1184 - DNA, 40 bp, synthetic construct
  misc_feature 1..40: note = Target Specific Oligonucleotide
  source 1..40: mol_type = other DNA
tctcagatcagtgcggagaaatagacgtctcccgtatttt

SEQ ID NO: 1185 - DNA, 39 bp, synthetic construct
  misc_feature 1..39: note = Target Specific Oligonucleotide
  source 1..39: mol_type = other DNA
gcccacaaatatccgtctgctagacgtctcccgtatttt

SEQ ID NO: 1186 - DNA, 36 bp, synthetic construct
  misc_feature 1..36: note = Target Specific Oligonucleotide
  source 1..36: mol_type = other DNA
ccatgttcgcgcggcgatagacgtctcccgtatttt

SEQ ID NO: 1187 - DNA, 42 bp, synthetic construct
  misc_feature 1..42: note = Target Specific Oligonucleotide
  source 1..42: mol_type = other DNA
atgaaaggtcgctagagaagtcctagacgtctcccgtatttt

SEQ ID NO: 1188 - DNA, 40 bp, synthetic construct
  misc_feature 1..40: note = Target Specific Oligonucleotide
  source 1..40: mol_type = other DNA
aatcacaaacccggacttggatagacgtctcccgtatttt

SEQ ID NO: 1189 - DNA, 40 bp, synthetic construct
  misc_feature 1..40: note = Target Specific Oligonucleotide
  source 1..40: mol_type = other DNA
actagcctgtcacgtttgtcttagacgtctcccgtatttt

SEQ ID NO: 1190 - DNA, 41 bp, synthetic construct
  misc_feature 1..41: note = Target Specific Oligonucleotide
  source 1..41: mol_type = other DNA
atctttacaatgcggtcggtcctagacgtctcccgtatttt

SEQ ID NO: 1191 - DNA, 41 bp, synthetic construct
  misc_feature 1..41: note = Target Specific Oligonucleotide
  source 1..41: mol_type = other DNA
tgtcctggtatgatcccaacactagacgtctcccgtatttt

SEQ ID NO: 1192 - DNA, 41 bp, synthetic construct
  misc_feature 1..41: note = Target Specific Oligonucleotide
  source 1..41: mol_type = other DNA
ctgatcatttcgcatcacagtgtagacgtctcccgtatttt

SEQ ID NO: 1193 - DNA, 41 bp, synthetic construct
  misc_feature 1..41: note = Target Specific Oligonucleotide
  source 1..41: mol_type = other DNA
ctttccttacgtgtgtcacacatagacgtctcccgtatttt

SEQ ID NO: 1194 - DNA, 42 bp, synthetic construct
  misc_feature 1..42: note = Target Specific Oligonucleotide
  source 1..42: mol_type = other DNA
tagtttgatcgcctccttaaacctagacgtctcccgtatttt

SEQ ID NO: 1195 - DNA, 42 bp, synthetic construct
  misc_feature 1..42: note = Target Specific Oligonucleotide
  source 1..42: mol_type = other DNA
aaatccctaggatagcacctttgtagacgtctcccgtatttt

SEQ ID NO: 1196 - DNA, 42 bp, synthetic construct
  misc_feature 1..42: note = Target Specific Oligonucleotide
  source 1..42: mol_type = other DNA
cttacacttacgatgagcagatgtagacgtctcccgtatttt

SEQ ID NO: 1197 - DNA, 43 bp, synthetic construct
  misc_feature 1..43: note = Target Specific Oligonucleotide
  source 1..43: mol_type = other DNA
catttgctacctagcatatgagagtagacgtctcccgtatttt

SEQ ID NO: 1198 - DNA, 41 bp, synthetic construct
  misc_feature 1..41: note = Target Specific Oligonucleotide
  source 1..41: mol_type = other DNA
acagatgtcaaacggtcacatttagacgtctcccgtatttt

SEQ ID NO: 1199 - DNA, 43 bp, synthetic construct
  misc_feature 1..43: note = Target Specific Oligonucleotide
  source 1..43: mol_type = other DNA
ttctaagatacgtcactccaattctagacgtctcccgtatttt

SEQ ID NO: 1200 - DNA, 42 bp, synthetic construct
  misc_feature 1..42: note = Target Specific Oligonucleotide
  source 1..42: mol_type = other DNA
acagtccgtcgattctttacaatagactctataaatcagcgt

SEQ ID NO: 1201 - DNA, 41 bp, synthetic construct
  misc_feature 1..41: note = Target Specific Oligonucleotide
  source 1..41: mol_type = other DNA
tctccacgtaaatcccgatcttagactctataaatcagcgt

SEQ ID NO: 1202 - DNA, 40 bp, synthetic construct
  misc_feature 1..40: note = Target Specific Oligonucleotide
  source 1..40: mol_type = other DNA
cacgtgctgaaccaaccacttagactctataaatcagcgt

SEQ ID NO: 1203 - DNA, 39 bp, synthetic construct
  misc_feature 1..39: note = Target Specific Oligonucleotide
  source 1..39: mol_type = other DNA
tcttgccgaagttggccgttagactctataaatcagcgt

SEQ ID NO: 1204 - DNA, 41 bp, synthetic construct
  misc_feature 1..41: note = Target Specific Oligonucleotide
  source 1..41: mol_type = other DNA
agcagcagttggatctacagttagactctataaatcagcgt

SEQ ID NO: 1205 - DNA, 43 bp, synthetic construct
  misc_feature 1..43: note = Target Specific Oligonucleotide
  source 1..43: mol_type = other DNA
gtctagcagtaaacctgtaaacctagactctataaatcagcgt

SEQ ID NO: 1206 - DNA, 42 bp, synthetic construct
  misc_feature 1..42: note = Target Specific Oligonucleotide
  source 1..42: mol_type = other DNA
gtgcattattggacgaacatcatagactctataaatcagcgt

SEQ ID NO: 1207 - DNA, 45 bp, synthetic construct
  misc_feature 1..45: note = Target Specific Oligonucleotide
  source 1..45: mol_type = other DNA
gctgttgttaatggtctataatccatagactctataaatcagcgt

SEQ ID NO: 1208 - DNA, 45 bp, synthetic construct
  misc_feature 1..45: note = Target Specific Oligonucleotide
  source 1..45: mol_type = other DNA
cacacatatcctatgttcatcaatatagactctataaatcagcgt

SEQ ID NO: 1209 - DNA, 43 bp, synthetic construct
  misc_feature 1..43: note = Target Specific Oligonucleotide
  source 1..43: mol_type = other DNA
ttgagtggtcgttttcttacacatagactctataaatcagcgt

SEQ ID NO: 1210 - DNA, 45 bp, synthetic construct
  misc_feature 1..45: note = Target Specific Oligonucleotide
  source 1..45: mol_type = other DNA
cataatcaaaacgaaatgtttggtttagactctataaatcagcgt

SEQ ID NO: 1211 - DNA, 41 bp, synthetic construct
  misc_feature 1..41: note = Target Specific Oligonucleotide
  source 1..41: mol_type = other DNA
tttgtagcatcaacgtcctggtagactctataaatcagcgt

SEQ ID NO: 1212 - DNA, 41 bp, synthetic construct
  misc_feature 1..41: note = Target Specific Oligonucleotide
  source 1..41: mol_type = other DNA
caacacatttgacctcccgtttagactctataaatcagcgt

SEQ ID NO: 1213 - DNA, 43 bp, synthetic construct
  misc_feature 1..43: note = Target Specific Oligonucleotide
  source 1..43: mol_type = other DNA
ctaaccaccgaatagattcctggtagactctataaatcagcgt

SEQ ID NO: 1214 - DNA, 41 bp, synthetic construct
  misc_feature 1..41: note = Target Specific Oligonucleotide
  source 1..41: mol_type = other DNA
gcagatgtttgaccggatgtttagactctataaatcagcgt

SEQ ID NO: 1215 - DNA, 42 bp, synthetic construct
  misc_feature 1..42: note = Target Specific Oligonucleotide
  source 1..42: mol_type = other DNA
tgcttgatgtattcggccatcgtagactctataaatcagcgt

SEQ ID NO: 1216 - DNA, 42 bp, synthetic construct
  misc_feature 1..42: note = Target Specific Oligonucleotide
  source 1..42: mol_type = other DNA
tgagtttacttgcacggaaaggtagactctataaatcagcgt

SEQ ID NO: 1217 - DNA, 42 bp, synthetic construct
  misc_feature 1..42: note = Target Specific Oligonucleotide
  source 1..42: mol_type = other DNA
cactttatcccgcagttcagtttagactctataaatcagcgt

SEQ ID NO: 1218 - DNA, 41 bp, synthetic construct
  misc_feature 1..41: note = Target Specific Oligonucleotide
  source 1..41: mol_type = other DNA
gcaaagcatgtagccattccctagactctataaatcagcgt

SEQ ID NO: 1219 - DNA, 43 bp, synthetic construct
  misc_feature 1..43: note = Target Specific Oligonucleotide
  source 1..43: mol_type = other DNA
aaagacatctcgagctgctaatgtagactctataaatcagcgt

SEQ ID NO: 1220 - DNA, 43 bp, synthetic construct
  misc_feature 1..43: note = Target Specific Oligonucleotide
  source 1..43: mol_type = other DNA
gtcaccacccatagtatgagttttagactctataaatcagcgt

SEQ ID NO: 1221 - DNA, 43 bp, synthetic construct
  misc_feature 1..43: note = Target Specific Oligonucleotide
  source 1..43: mol_type = other DNA
tttctacctaaggctctgatgcatagactctataaatcagcgt

SEQ ID NO: 1222 - DNA, 41 bp, synthetic construct
  misc_feature 1..41: note = Target Specific Oligonucleotide
  source 1..41: mol_type = other DNA
tagagctgcacggaaagattttagactctataaatcagcgt

SEQ ID NO: 1223 - DNA, 43 bp, synthetic construct
  misc_feature 1..43: note = Target Specific Oligonucleotide
  source 1..43: mol_type = other DNA
gtgtagcatatgaatcgacatcatagactctataaatcagcgt

SEQ ID NO: 1224 - DNA, 43 bp, synthetic construct
  misc_feature 1..43: note = Target Specific Oligonucleotide
  source 1..43: mol_type = other DNA
tagccttgtatggcagaatcgtagacctaaattactgtgaatg

SEQ ID NO: 1225 - DNA, 45 bp, synthetic construct
  misc_feature 1..45: note = Target Specific Oligonucleotide
  source 1..45: mol_type = other DNA
tgaattgccctgggtataactcctagacctaaattactgtgaatg

SEQ ID NO: 1226 - DNA, 42 bp, synthetic construct
  misc_feature 1..42: note = Target Specific Oligonucleotide
  source 1..42: mol_type = other DNA
ttcctgttgcaacgtgagggtagacctaaattactgtgaatg

SEQ ID NO: 1227 - DNA, 46 bp, synthetic construct
  misc_feature 1..46: note = Target Specific Oligonucleotide
  source 1..46: mol_type = other DNA
atgaaagacacgatcaaaattgaatagacctaaattactgtgaatg

SEQ ID NO: 1228 - DNA, 43 bp, synthetic construct
  misc_feature 1..43: note = Target Specific Oligonucleotide
  source 1..43: mol_type = other DNA
gtcagcacgaagtgagttcaatagacctaaattactgtgaatg

SEQ ID NO: 1229 - DNA, 44 bp, synthetic construct
  misc_feature 1..44: note = Target Specific Oligonucleotide
  source 1..44: mol_type = other DNA
cagtttgcagcgtagaatctcttagacctaaattactgtgaatg

SEQ ID NO: 1230 - DNA, 45 bp, synthetic construct
  misc_feature 1..45: note = Target Specific Oligonucleotide
  source 1..45: mol_type = other DNA
gtgcagataatacgtgtctttgctagacctaaattactgtgaatg

SEQ ID NO: 1231 - DNA, 45 bp, synthetic construct
  misc_feature 1..45: note = Target Specific Oligonucleotide
  source 1..45: mol_type = other DNA
tccaatgagtatgacaagtccattagacctaaattactgtgaatg

SEQ ID NO: 1232 - DNA, 45 bp, synthetic construct
  misc_feature 1..45: note = Target Specific Oligonucleotide
  source 1..45: mol_type = other DNA
tgtaagaaagctcggtcttcaaatagacctaaattactgtgaatg

SEQ ID NO: 1233 - DNA, 46 bp, synthetic construct
  misc_feature 1..46: note = Target Specific Oligonucleotide
  source 1..46: mol_type = other DNA
ccatgtaagatacacgtaagagaatagacctaaattactgtgaatg

SEQ ID NO: 1234 - DNA, 46 bp, synthetic construct
  misc_feature 1..46: note = Target Specific Oligonucleotide
  source 1..46: mol_type = other DNA
gactcaagagcatttcgtaattgttagacctaaattactgtgaatg

SEQ ID NO: 1235 - DNA, 46 bp, synthetic construct
  misc_feature 1..46: note = Target Specific Oligonucleotide
  source 1..46: mol_type = other DNA
atgtcattagtcacctcaagttcttagacctaaattactgtgaatg

SEQ ID NO: 1236 - DNA, 39 bp, synthetic construct
  misc_feature 1..39: note = Target Specific Oligonucleotide
  source 1..39: mol_type = other DNA
ccgcactcgcacgcagatagacctaaattactgtgaatg

SEQ ID NO: 1237 - DNA, 47 bp, synthetic construct
  misc_feature 1..47: note = Target Specific Oligonucleotide
  source 1..47: mol_type = other DNA
tgttaacagtatcgtgaatatcacttagacctaaattactgtgaatg

SEQ ID NO: 1238 - DNA, 45 bp, synthetic construct
  misc_feature 1..45: note = Target Specific Oligonucleotide
  source 1..45: mol_type = other DNA
actttgccatctataagggaggttagacctaaattactgtgaatg

SEQ ID NO: 1239 - DNA, 48 bp, synthetic construct
  misc_feature 1..48: note = Target Specific Oligonucleotide
  source 1..48: mol_type = other DNA
cttgctatctcgataatttatgaaactagacctaaattactgtgaatg

SEQ ID NO: 1240 - DNA, 48 bp, synthetic construct
  misc_feature 1..48: note = Target Specific Oligonucleotide
  source 1..48: mol_type = other DNA
ttaatgtatcaagagtgttactgaaatagacctaaattactgtgaatg

SEQ ID NO: 1241 - DNA, 46 bp, synthetic construct
  misc_feature 1..46: note = Target Specific Oligonucleotide
  source 1..46: mol_type = other DNA
tcaaatgggataccttaacagatctagacctaaattactgtgaatg

SEQ ID NO: 1242 - DNA, 50 bp, synthetic construct
  misc_feature 1..50: note = Target Specific Oligonucleotide
  source 1..50: mol_type = other DNA
ataaataagcttcgatttatattacagctagacctaaattactgtgaatg

SEQ ID NO: 1243 - DNA, 45 bp, synthetic construct
  misc_feature 1..45: note = Target Specific Oligonucleotide
  source 1..45: mol_type = other DNA
cttgtgtggtaggattaacctggtagacctaaattactgtgaatg

SEQ ID NO: 1244 - DNA, 43 bp, synthetic construct
  misc_feature 1..43: note = Target Specific Oligonucleotide
  source 1..43: mol_type = other DNA
gttggtcaactcgagcatctttagacctaaattactgtgaatg

SEQ ID NO: 1245 - DNA, 44 bp, synthetic construct
  misc_feature 1..44: note = Target Specific Oligonucleotide
  source 1..44: mol_type = other DNA
tttggtttgtaggcctgtagcttagacctaaattactgtgaatg

SEQ ID NO: 1246 - DNA, 45 bp, synthetic construct
  misc_feature 1..45: note = Target Specific Oligonucleotide
  source 1..45: mol_type = other DNA
cattaggcagtaactcttgttcctagacctaaattactgtgaatg

SEQ ID NO: 1247 - DNA, 45 bp, synthetic construct
  misc_feature 1..45: note = Target Specific Oligonucleotide
  source 1..45: mol_type = other DNA
cttctcagatacgcttcttcttatagacctaaattactgtgaatg

SEQ ID NO: 1248 - DNA, 31 bp, synthetic construct
  misc_feature 1..31: note = Decoding Oligonucleotide
  source 1..31: mol_type = other DNA
ggctaatttattaccttctagctataacgat

SEQ ID NO: 1249 - DNA, 31 bp, synthetic construct
  misc_feature 1..31: note = Decoding Oligonucleotide
  source 1..31: mol_type = other DNA
accttaagaatggaattctagctataacgat

SEQ ID NO: 1250 - DNA, 30 bp, synthetic construct
  misc_feature 1..30: note = Decoding Oligonucleotide
  source 1..30: mol_type = other DNA
acttaacttgagtggtctagctataacgat

SEQ ID NO: 1251 - DNA, 29 bp, synthetic construct
  misc_feature 1..29: note = Decoding Oligonucleotide
  source 1..29: mol_type = other DNA
ggctaatttattacctcggtctagatgga

SEQ ID NO: 1252 - DNA, 29 bp, synthetic construct
  misc_feature 1..29: note = Decoding Oligonucleotide
  source 1..29: mol_type = other DNA
accttaagaatggaatcggtctagatgga

SEQ ID NO: 1253 - DNA, 28 bp, synthetic construct
  misc_feature 1..28: note = Decoding Oligonucleotide
  source 1..28: mol_type = other DNA
acttaacttgagtggcggtctagatgga

SEQ ID NO: 1254 - DNA, 32 bp, synthetic construct
  misc_feature 1..32: note = Decoding Oligonucleotide
  source 1..32: mol_type = other DNA
ggctaatttattacctgttaactccgtagtaa

SEQ ID NO: 1255 - DNA, 32 bp, synthetic construct
  misc_feature 1..32: note = Decoding Oligonucleotide
  source 1..32: mol_type = other DNA
accttaagaatggaatgttaactccgtagtaa

SEQ ID NO: 1256 - DNA, 31 bp, synthetic construct
  misc_feature 1..31: note = Decoding Oligonucleotide
  source 1..31: mol_type = other DNA
acttaacttgagtgggttaactccgtagtaa

SEQ ID NO: 1257 - DNA, 31 bp, synthetic construct
  misc_feature 1..31: note = Decoding Oligonucleotide
  source 1..31: mol_type = other DNA
ggctaatttattacctcgctatatctactga

SEQ ID NO: 1258 - DNA, 31 bp, synthetic construct
  misc_feature 1..31: note = Decoding Oligonucleotide
  source 1..31: mol_type = other DNA
accttaagaatggaatcgctatatctactga

SEQ ID NO: 1259 - DNA, 30 bp, synthetic construct
  misc_feature 1..30: note = Decoding Oligonucleotide
  source 1..30: mol_type = other DNA
acttaacttgagtggcgctatatctactga

SEQ ID NO: 1260 - DNA, 30 bp, synthetic construct
  misc_feature 1..30: note = Decoding Oligonucleotide
  source 1..30: mol_type = other DNA
ggctaatttattacctgtttccgtttcgaa

SEQ ID NO: 1261 - DNA, 30 bp, synthetic construct
  misc_feature 1..30: note = Decoding Oligonucleotide
  source 1..30: mol_type = other DNA
accttaagaatggaatgtttccgtttcgaa

SEQ ID NO: 1262 - DNA, 29 bp, synthetic construct
  misc_feature 1..29: note = Decoding Oligonucleotide
  source 1..29: mol_type = other DNA
acttaacttgagtgggtttccgtttcgaa

SEQ ID NO: 1263 - DNA, 30 bp, synthetic construct
  misc_feature 1..30: note = Decoding Oligonucleotide
  source 1..30: mol_type = other DNA
ggctaatttattaccttagcgtttcaaaag

SEQ ID NO: 1264 - DNA, 30 bp, synthetic construct
  misc_feature 1..30: note = Decoding Oligonucleotide
  source 1..30: mol_type = other DNA
accttaagaatggaattagcgtttcaaaag

SEQ ID NO: 1265 - DNA, 29 bp, synthetic construct
  misc_feature 1..29: note = Decoding Oligonucleotide
  source 1..29: mol_type = other DNA
acttaacttgagtggtagcgtttcaaaag

SEQ ID NO: 1266 - DNA, 28 bp, synthetic construct
  misc_feature 1..28: note = Decoding Oligonucleotide
  source 1..28: mol_type = other DNA
ggctaatttattaccttgatccgacgag

SEQ ID NO: 1267 - DNA, 28 bp, synthetic construct
  misc_feature 1..28: note = Decoding Oligonucleotide
  source 1..28: mol_type = other DNA
accttaagaatggaattgatccgacgag

SEQ ID NO: 1268 - DNA, 27 bp, synthetic construct
  misc_feature 1..27: note = Decoding Oligonucleotide
  source 1..27: mol_type = other DNA
acttaacttgagtggtgatccgacgag

SEQ ID NO: 1269 - DNA, 31 bp, synthetic construct
  misc_feature 1..31: note = Decoding Oligonucleotide
  source 1..31: mol_type = other DNA
ggctaatttattacctaatctacatgtctga

SEQ ID NO: 1270 - DNA, 31 bp, synthetic construct
  misc_feature 1..31: note = Decoding Oligonucleotide
  source 1..31: mol_type = other DNA
accttaagaatggaataatctacatgtctga

SEQ ID NO: 1271 - DNA, 30 bp, synthetic construct
  misc_feature 1..30: note = Decoding Oligonucleotide
  source 1..30: mol_type = other DNA
acttaacttgagtggaatctacatgtctga

SEQ ID NO: 1272 - DNA, 30 bp, synthetic construct
  misc_feature 1..30: note = Decoding Oligonucleotide
  source 1..30: mol_type = other DNA
ggctaatttattacctggacgttgaataca

SEQ ID NO: 1273 - DNA, 30 bp, synthetic construct
  misc_feature 1..30: note = Decoding Oligonucleotide
  source 1..30: mol_type = other DNA
accttaagaatggaatggacgttgaataca

SEQ ID NO: 1274 - DNA, 29 bp, synthetic construct
  misc_feature 1..29: note = Decoding Oligonucleotide
  source 1..29: mol_type = other DNA
acttaacttgagtggggacgttgaataca

SEQ ID NO: 1275 - DNA, 31 bp, synthetic construct
  misc_feature 1..31: note = Decoding Oligonucleotide
  source 1..31: mol_type = other DNA
ggctaatttattaccttaaagtgacaattca

SEQ ID NO: 1276 - DNA, 31 bp, synthetic construct
  misc_feature 1..31: note = Decoding Oligonucleotide
  source 1..31: mol_type = other DNA
accttaagaatggaattaaagtgacaattca

SEQ ID NO: 1277 - DNA, 30 bp, synthetic construct
  misc_feature 1..30: note = Decoding Oligonucleotide
  source 1..30: mol_type = other DNA
acttaacttgagtggtaaagtgacaattca

SEQ ID NO: 1278 - DNA, 32 bp, synthetic construct
  misc_feature 1..32: note = Decoding Oligonucleotide
  source 1..32: mol_type = other DNA
ggctaatttattacctgattcccataattagg

SEQ ID NO: 1279 - DNA, 32 bp, synthetic construct
  misc_feature 1..32: note = Decoding Oligonucleotide
  source 1..32: mol_type = other DNA
accttaagaatggaatgattcccataattagg

SEQ ID NO: 1280 - DNA, 31 bp, synthetic construct
  misc_feature 1..31: note = Decoding Oligonucleotide
  source 1..31: mol_type = other DNA
acttaacttgagtgggattcccataattagg

SEQ ID NO: 1281 - DNA, 33 bp, synthetic construct
  misc_feature 1..33: note = Decoding Oligonucleotide
  source 1..33: mol_type = other DNA
ggctaatttattacctcgtcgtataaatctatc

SEQ ID NO: 1282 - DNA, 33 bp, synthetic construct
  misc_feature 1..33: note = Decoding Oligonucleotide
  source 1..33: mol_type = other DNA
accttaagaatggaatcgtcgtataaatctatc

SEQ ID NO: 1283 - DNA, 32 bp, synthetic construct
  misc_feature 1..32: note = Decoding Oligonucleotide
  source 1..32: mol_type = other DNA
acttaacttgagtggcgtcgtataaatctatc

SEQ ID NO: 1284 - DNA, 34 bp, synthetic construct
  misc_feature 1..34: note = Decoding Oligonucleotide
  source 1..34: mol_type = other DNA
ggctaatttattacctgatgtctatcctttataa

SEQ ID NO: 1285 - DNA, 34 bp, synthetic construct
  misc_feature 1..34: note = Decoding Oligonucleotide
  source 1..34: mol_type = other DNA
accttaagaatggaatgatgtctatcctttataa

SEQ ID NO: 1286 - DNA, 33 bp, synthetic construct
  misc_feature 1..33: note = Decoding Oligonucleotide
  source 1..33: mol_type = other DNA
acttaacttgagtgggatgtctatcctttataa

SEQ ID NO: 1287 - DNA, 30 bp, synthetic construct
  misc_feature 1..30: note = Decoding Oligonucleotide
  source 1..30: mol_type = other DNA
ggctaatttattaccttttccacgataacc

SEQ ID NO: 1288 - DNA, 30 bp, synthetic construct
  misc_feature 1..30: note = Decoding Oligonucleotide
  source 1..30: mol_type = other DNA
accttaagaatggaattttccacgataacc

SEQ ID NO: 1289 - DNA, 29 bp, synthetic construct
  misc_feature 1..29: note = Decoding Oligonucleotide
  source 1..29: mol_type = other DNA
acttaacttgagtggtttccacgataacc

SEQ ID NO: 1290 - DNA, 31 bp, synthetic construct
  misc_feature 1..31: note = Decoding Oligonucleotide
  source 1..31: mol_type = other DNA
ggctaatttattaccttagtaccgaataagg

SEQ ID NO: 1291 - DNA, 31 bp, synthetic construct
  misc_feature 1..31: note = Decoding Oligonucleotide
  source 1..31: mol_type = other DNA
accttaagaatggaattagtaccgaataagg

SEQ ID NO: 1292 - DNA, 30 bp, synthetic construct
  misc_feature 1..30: note = Decoding Oligonucleotide
  source 1..30: mol_type = other DNA
acttaacttgagtggtagtaccgaataagg

SEQ ID NO: 1293 - DNA, 32 bp, synthetic construct
  misc_feature 1..32: note = Decoding Oligonucleotide
  source 1..32: mol_type = other DNA
ggctaatttattaccttaaagttgtaaaatcc

SEQ ID NO: 1294 - DNA, 32 bp, synthetic construct
  misc_feature 1..32: note = Decoding Oligonucleotide
  source 1..32: mol_type = other DNA
accttaagaatggaattaaagttgtaaaatcc

SEQ ID NO: 1295 - DNA, 31 bp, synthetic construct
  misc_feature 1..31: note = Decoding Oligonucleotide
  source 1..31: mol_type = other DNA
acttaacttgagtggtaaagttgtaaaatcc

SEQ ID NO: 1296 - DNA, 32 bp, synthetic construct
  misc_feature 1..32: note = Decoding Oligonucleotide
  source 1..32: mol_type = other DNA
ggctaatttattacctggataagtcggtaatc

SEQ ID NO: 1297 - DNA, 32 bp, synthetic construct
  misc_feature 1..32: note = Decoding Oligonucleotide
  source 1..32: mol_type = other DNA
accttaagaatggaatggataagtcggtaatc

SEQ ID NO: 1298 - DNA, 31 bp, synthetic construct
  misc_feature 1..31: note = Decoding Oligonucleotide
  source 1..31: mol_type = other DNA
acttaacttgagtggggataagtcggtaatc

SEQ ID NO: 1299 - DNA, 33 bp, synthetic construct
  misc_feature 1..33: note = Decoding Oligonucleotide
  source 1..33: mol_type = other DNA
ggctaatttattacctggtatttcactctaatt

SEQ ID NO: 1300 - DNA, 33 bp, synthetic construct
  misc_feature 1..33: note = Decoding Oligonucleotide
  source 1..33: mol_type = other DNA
accttaagaatggaatggtatttcactctaatt

SEQ ID NO: 1301 - DNA, 32 bp, synthetic construct
  misc_feature 1..32: note = Decoding Oligonucleotide
  source 1..32: mol_type = other DNA
acttaacttgagtggggtatttcactctaatt

SEQ ID NO: 1302 - DNA, 32 bp, synthetic construct
  misc_feature 1..32: note = Decoding Oligonucleotide
  source 1..32: mol_type = other DNA
ggctaatttattacctagctagataaagtacc

SEQ ID NO: 1303 - DNA, 32 bp, synthetic construct
  misc_feature 1..32: note = Decoding Oligonucleotide
  source 1..32: mol_type = other DNA
accttaagaatggaatagctagataaagtacc

SEQ ID NO: 1304 - DNA, 31 bp, synthetic construct
  misc_feature 1..31: note = Decoding Oligonucleotide
  source 1..31: mol_type = other DNA
acttaacttgagtggagctagataaagtacc

SEQ ID NO: 1305 - DNA, 32 bp, synthetic construct
  misc_feature 1..32: note = Decoding Oligonucleotide
  source 1..32: mol_type = other DNA
ggctaatttattacctccgaaactacgattat

SEQ ID NO: 1306 - DNA, 32 bp, synthetic construct
  misc_feature 1..32: note = Decoding Oligonucleotide
  source 1..32: mol_type = other DNA
accttaagaatggaatccgaaactacgattat

SEQ ID NO: 1307 - DNA, 31 bp, synthetic construct
  misc_feature 1..31: note = Decoding Oligonucleotide
  source 1..31: mol_type = other DNA
acttaacttgagtggccgaaactacgattat

SEQ ID NO: 1308 - DNA, 32 bp, synthetic construct
  misc_feature 1..32: note = Decoding Oligonucleotide
  source 1..32: mol_type = other DNA
ggctaatttattacctcatcgaatttatgtta

SEQ ID NO: 1309 - DNA, 32 bp, synthetic construct
  misc_feature 1..32: note = Decoding Oligonucleotide
  source 1..32: mol_type = other DNA
accttaagaatggaatcatcgaatttatgtta

SEQ ID NO: 1310 - DNA, 31 bp, synthetic construct
  misc_feature 1..31: note = Decoding Oligonucleotide
  source 1..31: mol_type = other DNA
acttaacttgagtggcatcgaatttatgtta

SEQ ID NO: 1311 - DNA, 30 bp, synthetic construct
  misc_feature 1..30: note = Decoding Oligonucleotide
  source 1..30: mol_type = other DNA
ggctaatttattacctccgtaattctaccg

SEQ ID NO: 1312 - DNA, 30 bp, synthetic construct
  misc_feature 1..30: note = Decoding Oligonucleotide
  source 1..30: mol_type = other DNA
accttaagaatggaatccgtaattctaccg

SEQ ID NO: 1313 - DNA, 29 bp, synthetic construct
  misc_feature 1..29: note = Decoding Oligonucleotide
  source 1..29: mol_type = other DNA
acttaacttgagtggccgtaattctaccg

SEQ ID NO: 1314 - DNA, 29 bp, synthetic construct
  misc_feature 1..29: note = Decoding Oligonucleotide
  source 1..29: mol_type = other DNA
ggctaatttattacctgggtaatcgtcac

SEQ ID NO: 1315 - DNA, 29 bp, synthetic construct
  misc_feature 1..29: note = Decoding Oligonucleotide
  source 1..29: mol_type = other DNA
accttaagaatggaatgggtaatcgtcac

SEQ ID NO: 1316 - DNA, 28 bp, synthetic construct
  misc_feature 1..28: note = Decoding Oligonucleotide
  source 1..28: mol_type = other DNA
acttaacttgagtgggggtaatcgtcac

SEQ ID NO: 1317 - DNA, 31 bp, synthetic construct
  misc_feature 1..31: note = Decoding Oligonucleotide
  source 1..31: mol_type = other DNA
ggctaatttattacctagtgttatgagaagc

SEQ ID NO: 1318 - DNA, 31 bp, synthetic construct
  misc_feature 1..31: note = Decoding Oligonucleotide
  source 1..31: mol_type = other DNA
accttaagaatggaatagtgttatgagaagc

SEQ ID NO: 1319 - DNA, 30 bp, synthetic construct
  misc_feature 1..30: note = Decoding Oligonucleotide
  source 1..30: mol_type = other DNA
acttaacttgagtggagtgttatgagaagc

SEQ ID NO: 1320 - DNA, 31 bp, synthetic construct
  misc_feature 1..31: note = Decoding Oligonucleotide
  source 1..31: mol_type = other DNA
ggctaatttattacctctgcaatagaagaga

SEQ ID NO: 1321 - DNA, 31 bp, synthetic construct
  misc_feature 1..31: note = Decoding Oligonucleotide
  source 1..31: mol_type = other DNA
accttaagaatggaatctgcaatagaagaga

SEQ ID NO: 1322 - DNA, 30 bp, synthetic construct
  misc_feature 1..30: note = Decoding Oligonucleotide
  source 1..30: mol_type = other DNA
acttaacttgagtggctgcaatagaagaga

SEQ ID NO: 1323 - DNA, 30 bp, synthetic construct
  misc_feature 1..30: note = Decoding Oligonucleotide
  source 1..30: mol_type = other DNA
ggctaatttattacctgatttttcagcgac

SEQ ID NO: 1324 - DNA, 30 bp, synthetic construct
  misc_feature 1..30: note = Decoding Oligonucleotide
  source 1..30: mol_type = other DNA
accttaagaatggaatgatttttcagcgac

SEQ ID NO: 1325 - DNA, 29 bp, synthetic construct
  misc_feature 1..29: note = Decoding Oligonucleotide
  source 1..29: mol_type = other DNA
acttaacttgagtgggatttttcagcgac

SEQ ID NO: 1326 - DNA, 32 bp, synthetic construct
  misc_feature 1..32: note = Decoding Oligonucleotide
  source 1..32: mol_type = other DNA
ggctaatttattacctcgtaatatgaagatca

SEQ ID NO: 1327 - DNA, 32 bp, synthetic construct
  misc_feature 1..32: note = Decoding Oligonucleotide
  source 1..32: mol_type = other DNA
accttaagaatggaatcgtaatatgaagatca

SEQ ID NO: 1328 - DNA, 31 bp, synthetic construct
  misc_feature 1..31: note = Decoding Oligonucleotide
  source 1..31: mol_type = other DNA
acttaacttgagtggcgtaatatgaagatca

SEQ ID NO: 1329 - DNA, 32 bp, synthetic construct
  misc_feature 1..32: note = Decoding Oligonucleotide
  source 1..32: mol_type = other DNA
ggctaatttattacctgaattggaatattcgt

SEQ ID NO: 1330 - DNA, 32 bp, synthetic construct
  misc_feature 1..32: note = Decoding Oligonucleotide
  source 1..32: mol_type = other DNA
accttaagaatggaatgaattggaatattcgt

SEQ ID NO: 1331 - DNA, 31 bp, synthetic construct
  misc_feature 1..31: note = Decoding Oligonucleotide
  source 1..31: mol_type = other DNA
acttaacttgagtgggaattggaatattcgt

SEQ ID NO: 1332 - DNA, 33 bp, synthetic construct
  misc_feature 1..33: note = Decoding Oligonucleotide
  source 1..33: mol_type = other DNA
ggctaatttattacctggtattaatcttgaaga

SEQ ID NO: 1333 - DNA, 33 bp, synthetic construct
  misc_feature 1..33: note = Decoding Oligonucleotide
  source 1..33: mol_type = other DNA
accttaagaatggaatggtattaatcttgaaga

SEQ ID NO: 1334 - DNA, 32 bp, synthetic construct
  misc_feature 1..32: note = Decoding Oligonucleotide
  source 1..32: mol_type = other DNA
acttaacttgagtggggtattaatcttgaaga

SEQ ID NO: 1335 - DNA, 29 bp, synthetic construct
  misc_feature 1..29: note = Decoding Oligonucleotide
  source 1..29: mol_type = other DNA
ggctaatttattacctacgatgtattgcc

SEQ ID NO: 1336 - DNA, 29 bp, synthetic construct
  misc_feature 1..29: note = Decoding Oligonucleotide
  source 1..29: mol_type = other DNA
accttaagaatggaatacgatgtattgcc

SEQ ID NO: 1337 - DNA, 28 bp, synthetic construct
  misc_feature 1..28: note = Decoding Oligonucleotide
  source 1..28: mol_type = other DNA
acttaacttgagtggacgatgtattgcc

SEQ ID NO: 1338 - DNA, 32 bp, synthetic construct
  misc_feature 1..32: note = Decoding Oligonucleotide
  source 1..32: mol_type = other DNA
ggctaatttattacctcatatacaaacggtac

SEQ ID NO: 1339 - DNA, 32 bp, synthetic construct
  misc_feature 1..32: note = Decoding Oligonucleotide
  source 1..32: mol_type = other DNA
accttaagaatggaatcatatacaaacggtac

SEQ ID NO: 1340 - DNA, 31 bp, synthetic construct
  misc_feature 1..31: note = Decoding Oligonucleotide
  source 1..31: mol_type = other DNA
acttaacttgagtggcatatacaaacggtac

SEQ ID NO: 1341 - DNA, 31 bp, synthetic construct
  misc_feature 1..31: note = Decoding Oligonucleotide
  source 1..31: mol_type = other DNA
ggctaatttattacctttccgatcttaactt

SEQ ID NO: 1342 - DNA, 31 bp, synthetic construct
  misc_feature 1..31: note = Decoding Oligonucleotide
  source 1..31: mol_type = other DNA
accttaagaatggaatttccgatcttaactt

SEQ ID NO: 1343 - DNA, 30 bp, synthetic construct
  misc_feature 1..30: note = Decoding Oligonucleotide
  source 1..30: mol_type = other DNA
acttaacttgagtggttccgatcttaactt

SEQ ID NO: 1344 - DNA, 31 bp, synthetic construct
  misc_feature 1..31: note = Decoding Oligonucleotide
  source 1..31: mol_type = other DNA
ggctaatttattacctgtgttaattcgcatc

SEQ ID NO: 1345 - DNA, 31 bp, synthetic construct
  misc_feature 1..31: note = Decoding Oligonucleotide
  source 1..31: mol_type = other DNA
accttaagaatggaatgtgttaattcgcatc

SEQ ID NO: 1346 - DNA, 30 bp, synthetic construct
  misc_feature 1..30: note = Decoding Oligonucleotide
  source 1..30: mol_type = other DNA
acttaacttgagtgggtgttaattcgcatc

SEQ ID NO: 1347 - DNA, 30 bp, synthetic construct
  misc_feature 1..30: note = Decoding Oligonucleotide
  source 1..30: mol_type = other DNA
ggctaatttattacctcgtttaattgggct

SEQ ID NO: 1348 - DNA, 30 bp, synthetic construct
  misc_feature 1..30: note = Decoding Oligonucleotide
  source 1..30: mol_type = other DNA
accttaagaatggaatcgtttaattgggct

SEQ ID NO: 1349 - DNA, 29 bp, synthetic construct
  misc_feature 1..29: note = Decoding Oligonucleotide
  source 1..29: mol_type = other DNA
acttaacttgagtggcgtttaattgggct

SEQ ID NO: 1350 - DNA, 31 bp, synthetic construct
  misc_feature 1..31: note = Decoding Oligonucleotide
  source 1..31: mol_type = other DNA
ggctaatttattacctcaacacttataacgg

SEQ ID NO: 1351 - DNA, 31 bp, synthetic construct
  misc_feature 1..31: note = Decoding Oligonucleotide
  source 1..31: mol_type = other DNA
accttaagaatggaatcaacacttataacgg

SEQ ID NO: 1352 - DNA, 30 bp, synthetic construct
  misc_feature 1..30: note = Decoding Oligonucleotide
  source 1..30: mol_type = other DNA
acttaacttgagtggcaacacttataacgg

SEQ ID NO: 1353 - DNA, 34 bp, synthetic construct
  misc_feature 1..34: note = Decoding Oligonucleotide
  source 1..34: mol_type = other DNA
ggctaatttattacctggaaataagtattatacc

SEQ ID NO: 1354 - DNA, 34 bp, synthetic construct
  misc_feature 1..34: note = Decoding Oligonucleotide
  source 1..34: mol_type = other DNA
accttaagaatggaatggaaataagtattatacc

SEQ ID NO: 1355 - DNA, 33 bp, synthetic construct
  misc_feature 1..33: note = Decoding Oligonucleotide
  source 1..33: mol_type = other DNA
acttaacttgagtggggaaataagtattatacc

SEQ ID NO: 1356 - DNA, 29 bp, synthetic construct
  misc_feature 1..29: note = Decoding Oligonucleotide
  source 1..29: mol_type = other DNA
ggctaatttattacctcttaacgacggtt

SEQ ID NO: 1357 - DNA, 29 bp, synthetic construct
  misc_feature 1..29: note = Decoding Oligonucleotide
  source 1..29: mol_type = other DNA
accttaagaatggaatcttaacgacggtt

SEQ ID NO: 1358 - DNA, 28 bp, synthetic construct
  misc_feature 1..28: note = Decoding Oligonucleotide
  source 1..28: mol_type = other DNA
acttaacttgagtggcttaacgacggtt

SEQ ID NO: 1359 - DNA, 33 bp, synthetic construct
  misc_feature 1..33: note = Decoding Oligonucleotide
  source 1..33: mol_type = other DNA
ggctaatttattacctgctcgttagaatttatt

SEQ ID NO: 1360 - DNA, 33 bp, synthetic construct
  misc_feature 1..33: note = Decoding Oligonucleotide
  source 1..33: mol_type = other DNA
accttaagaatggaatgctcgttagaatttatt

SEQ ID NO: 1361 - DNA, 32 bp, synthetic construct
  misc_feature 1..32: note = Decoding Oligonucleotide
  source 1..32: mol_type = other DNA
acttaacttgagtgggctcgttagaatttatt

SEQ ID NO: 1362 - DNA, 32 bp, synthetic construct
  misc_feature 1..32: note = Decoding Oligonucleotide
  source 1..32: mol_type = other DNA
ggctaatttattaccttctttatcatcattga

SEQ ID NO: 1363 - DNA, 32 bp, synthetic construct
  misc_feature 1..32: note = Decoding Oligonucleotide
  source 1..32: mol_type = other DNA
accttaagaatggaattctttatcatcattga

SEQ ID NO: 1364 - DNA, 31 bp, synthetic construct
  misc_feature 1..31: note = Decoding Oligonucleotide
  source 1..31: mol_type = other DNA
acttaacttgagtggtctttatcatcattga

SEQ ID NO: 1365 - DNA, 31 bp, synthetic construct
  misc_feature 1..31: note = Decoding Oligonucleotide
  source 1..31: mol_type = other DNA
ggctaatttattacctcgttcgcaatttatc

SEQ ID NO: 1366 - DNA, 31 bp, synthetic construct
  misc_feature 1..31: note = Decoding Oligonucleotide
  source 1..31: mol_type = other DNA
accttaagaatggaatcgttcgcaatttatc

SEQ ID NO: 1367 - DNA, 30 bp, synthetic construct
  misc_feature 1..30: note = Decoding Oligonucleotide
  source 1..30: mol_type = other DNA
acttaacttgagtggcgttcgcaatttatc

SEQ ID NO: 1368 - DNA, 31 bp, synthetic construct
  misc_feature 1..31: note = Decoding Oligonucleotide
  source 1..31: mol_type = other DNA
ggctaatttattacctcgatcttttgttgta

SEQ ID NO: 1369 - DNA, 31 bp, synthetic construct
  misc_feature 1..31: note = Decoding Oligonucleotide
  source 1..31: mol_type = other DNA
accttaagaatggaatcgatcttttgttgta

SEQ ID NO: 1370 - DNA, 30 bp, synthetic construct
  misc_feature 1..30: note = Decoding Oligonucleotide
  source 1..30: mol_type = other DNA
acttaacttgagtggcgatcttttgttgta

SEQ ID NO: 1371 - DNA, 32 bp, synthetic construct
  misc_feature 1..32: note = Decoding Oligonucleotide
  source 1..32: mol_type = other DNA
ggctaatttattacctaccactcaatataaga

SEQ ID NO: 1372 - DNA, 32 bp, synthetic construct
  misc_feature 1..32: note = Decoding Oligonucleotide
  source 1..32: mol_type = other DNA
accttaagaatggaataccactcaatataaga

SEQ ID NO: 1373 - DNA, 31 bp, synthetic construct
  misc_feature 1..31: note = Decoding Oligonucleotide
  source 1..31: mol_type = other DNA
acttaacttgagtggaccactcaatataaga

SEQ ID NO: 1374 - DNA, 30 bp, synthetic construct
  misc_feature 1..30: note = Decoding Oligonucleotide
  source 1..30: mol_type = other DNA
ggctaatttattacctccgtaaattcggtc

SEQ ID NO: 1375 - DNA, 30 bp, synthetic construct
  misc_feature 1..30: note = Decoding Oligonucleotide
  source 1..30: mol_type = other DNA
accttaagaatggaatccgtaaattcggtc

SEQ ID NO: 1376 - DNA, 29 bp, synthetic construct
  misc_feature 1..29: note = Decoding Oligonucleotide
  source 1..29: mol_type = other DNA
acttaacttgagtggccgtaaattcggtc

SEQ ID NO: 1377 - DNA, 30 bp, synthetic construct
  misc_feature 1..30: note = Decoding Oligonucleotide
  source 1..30: mol_type = other DNA
ggctaatttattacctcgtgagatttctga

SEQ ID NO: 1378 - DNA, 30 bp, synthetic construct
  misc_feature 1..30: note = Decoding Oligonucleotide
  source 1..30: mol_type = other DNA
accttaagaatggaatcgtgagatttctga

SEQ ID NO: 1379 - DNA, 29 bp, synthetic construct
  misc_feature 1..29: note = Decoding Oligonucleotide
  source 1..29: mol_type = other DNA
acttaacttgagtggcgtgagatttctga

SEQ ID NO: 1380 - DNA, 31 bp, synthetic construct
  misc_feature 1..31: note = Decoding Oligonucleotide
  source 1..31: mol_type = other DNA
ggctaatttattacctcgaagcatagaatag

SEQ ID NO: 1381 - DNA, 31 bp, synthetic construct
  misc_feature 1..31: note = Decoding Oligonucleotide
  source 1..31: mol_type = other DNA
accttaagaatggaatcgaagcatagaatag

SEQ ID NO: 1382 - DNA, 30 bp, synthetic construct
  misc_feature 1..30: note = Decoding Oligonucleotide
  source 1..30: mol_type = other DNA
acttaacttgagtggcgaagcatagaatag

SEQ ID NO: 1383 - DNA, 30 bp, synthetic construct
  misc_feature 1..30: note = Decoding Oligonucleotide
  source 1..30: mol_type = other DNA
ggctaatttattacctaaaatacgggagac

SEQ ID NO: 1384 - DNA, 30 bp, synthetic construct
  misc_feature 1..30: note = Decoding Oligonucleotide
  source 1..30: mol_type = other DNA
accttaagaatggaataaaatacgggagac

SEQ ID NO: 1385 - DNA, 29 bp, synthetic construct
  misc_feature 1..29: note = Decoding Oligonucleotide
  source 1..29: mol_type = other DNA
acttaacttgagtggaaaatacgggagac

SEQ ID NO: 1386 - DNA, 31 bp, synthetic construct
  misc_feature 1..31: note = Decoding Oligonucleotide
  source 1..31: mol_type = other DNA
ggctaatttattacctcgcatggtataacat

SEQ ID NO: 1387 - DNA, 31 bp, synthetic construct
  misc_feature 1..31: note = Decoding Oligonucleotide
  source 1..31: mol_type = other DNA
accttaagaatggaatcgcatggtataacat

SEQ ID NO: 1388 - DNA, 30 bp, synthetic construct
  misc_feature 1..30: note = Decoding Oligonucleotide
  source 1..30: mol_type = other DNA
acttaacttgagtggcgcatggtataacat

SEQ ID NO: 1389 - DNA, 31 bp, synthetic construct
  misc_feature 1..31: note = Decoding Oligonucleotide
  source 1..31: mol_type = other DNA
ggctaatttattacctacgctgatttataga

SEQ ID NO: 1390 - DNA, 31 bp, synthetic construct
  misc_feature 1..31: note = Decoding Oligonucleotide
  source 1..31: mol_type = other DNA
accttaagaatggaatacgctgatttataga

SEQ ID NO: 1391 - DNA, 30 bp, synthetic construct
  misc_feature 1..30: note = Decoding Oligonucleotide
  source 1..30: mol_type = other DNA
acttaacttgagtggacgctgatttataga

SEQ ID NO: 1392 - DNA, 33 bp, synthetic construct
  misc_feature 1..33: note = Decoding Oligonucleotide
  source 1..33: mol_type = other DNA
ggctaatttattacctcgtagggtaaatagatt

SEQ ID NO: 1393 - DNA, 33 bp, synthetic construct
  misc_feature 1..33: note = Decoding Oligonucleotide
  source 1..33: mol_type = other DNA
accttaagaatggaatcgtagggtaaatagatt

SEQ ID NO: 1394 - DNA, 32 bp, synthetic construct
  misc_feature 1..32: note = Decoding Oligonucleotide
  source 1..32: mol_type = other DNA
acttaacttgagtggcgtagggtaaatagatt

SEQ ID NO: 1395 - DNA, 33 bp, synthetic construct
  misc_feature 1..33: note = Decoding Oligonucleotide
  source 1..33: mol_type = other DNA
ggctaatttattacctcattcacagtaatttag

SEQ ID NO: 1396 - DNA, 33 bp, synthetic construct
  misc_feature 1..33: note = Decoding Oligonucleotide
  source 1..33: mol_type = other DNA
accttaagaatggaatcattcacagtaatttag

SEQ ID NO: 1397 - DNA, 32 bp, synthetic construct
  misc_feature 1..32: note = Decoding Oligonucleotide
  source 1..32: mol_type = other DNA
acttaacttgagtggcattcacagtaatttag

SEQ ID NO: 1398 - DNA, 15 bp, synthetic construct
  misc_feature 1..15: note = Signal Oligonucleotide
  source 1..15: mol_type = other DNA
ccactcaagttaagt

SEQ ID NO: 1399 - DNA, 16 bp, synthetic construct
  misc_feature 1..16: note = Signal Oligonucleotide
  source 1..16: mol_type = other DNA
attccattcttaaggt

SEQ ID NO: 1400 - DNA, 16 bp, synthetic construct
  misc_feature 1..16: note = Signal Oligonucleotide
  source 1..16: mol_type = other DNA
aggtaataaattagcc